European Patent Specification EP 3 697 805 B1, published June 10, 2026. Title: Fermentative production of N-acetylneuraminic acid. Applicant: Jennewein Biotechnologie GmbH. The sequence listing filed with the application follows.

SEQUENCE LISTING (103 sequences)

SEQ ID NO: 1 - DNA, 2851 bp, Artificial Sequence
  Expression fragment
tggccagatgattaattcctaatttttgttgacactctatcattgatagagttattttaccactccctatcagtgatagagaaaagtgaaatgaatagttcgacaaaaatctagaaataattttgtttaactttaagaaggagatatacaaatgtactatttaaaaaacacaaacttttggatgttcggtttattctttttcttttacttttttatcatgggagcctacttcccgtttttcccgatttggctacatgacatcaaccatatcagcaaaagtgatacgggtattatttttgccgctatttctctgttctcgctattattccaaccgctgtttggtctgctttctgacaaactcgggctgcgcaaatacctgctgtggattattaccggcatgttagtgatgtttgcgccgttctttatttttatcttcgggccactgttacaatacaacattttagtaggatcgattgttggtggtatttatctaggcttttgttttaacgccggtgcgccagcagtagaggcatttattgagaaagtcagccgtcgcagtaatttcgaatttggtcgcgcgcggatgtttggctgtgttggctgggcgctgtgtgcctcgattgtcggcatcatgttcaccatcaataatcagtttgttttctggctgggctctggctgtgcactcatcctcgccgttttactctttttcgccaaaacggatgcgccctcttctgccacggttgccaatgcggtaggtgccaaccattcggcatttagccttaagctggcactggaactgttcagacagccaaaactgtggtttttgtcactgtatgttattggcgtttcctgcacctacgatgtttttgaccaacagtttgctaatttctttacttcgttctttgctaccggtgaacagggtacgcgggtatttggctacgtaacgacaatgggcgaattacttaacgcctcgattatgttctttgcgccactgatcattaatcgcatcggtgggaaaaacgccctgctgctggctggcactattatgtctgtacgtattattggctcatcgttcgccacctcagcgctggaagtggttattctgaaaacgctgcatatgtttgaagtaccgttcctgctggtgggctgctttaaatatattaccagccagtttgaagtgcgtttttcagcgacgatttatctggtctgtttctgcttctttaagcaactggcgatgatttttatgtctgtactggcgggcaatatgtatgaaagcatcggtttccagggcgcttatctggtgctgggtctggtggcgctgggcttcaccttaatttccgtgttcacgcttagcggccccggcccgctttccctgctgcgtcgtcaggtgaatgaagtcgctgggagctaagcggccgcgtcgacacgcaaaaaggccatccgtcaggatggccttctgcttaatttgatgcctggcagtttatggcgggcgtcctgcccgccaccctccgggccgttgcttcgcaacgttcaaatccgctcccggcggatttgtcctactcaggagagcgttcaccgacaaacaacagataaaacgaaaggcccagtctttcgactgagcctttcgttttatttgatgcctggcagttccctactctcgcatggggagaccccacactaccatcatgtatgaatatcctccttagttcctattccgaagttcctattctctagaaagtataggaacttcggcgcgtcctacctgtgacacgcgtgccgcagtctcacgcccggagcgtagcgaccgagtgagctagctatttgtttatttttctaaatacattcaaatatgtatccgctcatgagacaataaccctgataaatgcttcaataatattgaaaaaggaagagtatgagggaagcggtgatcgccgaagtatcgactcaactatcagaggtagttggcgtcatcgagcgccatctcgaaccgacgttgctggccgtacatttgtacggctccgcagtggatggcggcctgaagccacacagtgatattgatttgctggttacggtgaccgtaaggcttgatgaaacaacgcggcgagctttgatcaacgaccttttggaaacttcggcttcccctggagagagcgagattctccgcgctgtagaagtcaccattgttgtgcacgacgacatcattccgtggcgttatccagctaagcgcgaactgcaatttggagaatggcagcgcaatgacattcttgcaggtatcttcgagccagccacgatcgacattgatctggctatcttgctgacaaaagcaagagaacatagcgttgccttggtaggtccagcggcggaggaactctttgatccggttcctgaacaggatctatttgaggcgctaaatgaaaccttaacgctatggaactcgccgcccgactgggctggcgatgagcgaaatgtagtgcttacgttgtcccgcatttggtacagcgcagtaaccggcaaaatcgcgccgaaggatgtcgctgccgactgggcaatggagcgcctgccggcccagtatcagcccgtcatacttgaagctagacaggcttatcttggacaagaagaagatcgcttggcctcgcgcgcagatcagttggaagaatttgtccactacgtgaaaggcgagatcaccaaggtagtcggcaaataatgtctaacaattcgttcaagccgaggggccgcaagatccggccacgatgacccggtcgtcgggtaccggcagggcggggcgtaaggcgcgccatttaaatgaagttcctattccgaagttcctattctctagaaagtataggaactt

SEQ ID NO: 2 - DNA, 5226 bp, Artificial Sequence
  E. coli W csc gene cluster comprising the genes for sucrose permease (cscB), fructokinase (cscK), sucrose hydrolase (cscA) and a transcriptional repressor (cscR)
acaggttggctgataagtccccggtctggcagccgcgactgtaccagaacatgaatgaggcgtttggattaggcgattattagcagggctaagcattttactattattattttccggttgagggatatagagctatcgacaacaaccggaaaaagtttacgtctatattgctgaaggtacaggcgtttccataactatttgctcgcgttttttactcaagaagaaaatgccaaatagcaacatcaggcagacaatacccgaaattgcgaagaaaactgtctggtagcctgcgtggtcaaagagtatcccagtcggcgttgaaagcagcacaatcccaagcgaactggcaatttgaaaaccaatcagaaagatcgtcgacgacaggcgcttatcaaagtttgccacgctgtatttgaagacggatatgacacaaagtggaacctcaatggcatgtaacaacttcactaatgaaataatccaggggttaacgaacagcgcgcaggaaaggatacgcaacgccataatcacaactccgataagtaatgcattttttggccctacccgattcacaaagaaaggaataatcgccatgcacagcgcttcgagtaccacctggaatgagttgagataaccatacaggcgcgttcctacatcgtgtgattcgaataaacctgaataaaagacaggaaaaagttgttgatcaaaaatgttatagaaagaccacgtccccacaataaatatgacgaaaacccagaagtttcgatccttgaaaactgcgataaaatcctctttttttacccctcccgcatctgccgctacgcactggtgatccttatctttaaaacgcatgttgatcatcataaatacagcgccaaatagcgagaccaaccagaagttgatatggggactgatactaaaaaatatgccggcaaagaacgcgccaatagcatagccaaaagatccccaggcgcgcgctgttccatattcgaaatgaaaatttcgcgccattttttcggtgaagctatcaagcaaaccgcatcccgccagataccccaagccaaaaaatagcgcccccagaattagacctacagaaaaattgctttgcagtaacggttcataaacgtaaatcataaacggtccggtcaagaccaggatgaaactcatacaccagatgagcggtttcttcagaccgagtttatcctgaacgatgccgtagaacatcataaatagaatgctggtaaactggttgaccgaataaagtgtacctaattccgtccctgtcaaccctagatgtcctttcagccaaatagcgtataacgaccaccacagcgaccaggaaataaaaaagagaaatgagtaactggatgcaaaacgatagtacgcatttctgaatggaatattcagtgccataattacctgcctgtcgttaaaaaattcacgtcctatttagagataagagcgacttcgccgtttacttctcactattccagttcttgtcgacatggcagcgctgtcattgcccctttcgccgttactgcaagcgctccgcaacgttgagcgagatcgataattcgtcgcatttctctctcatctgtagataatcccgtagaggacagacctgtgagtaacccggcaacgaacgcatctcccgcccccgtgctatcgacacaattcacagacattccagcaaaatggtgaacttgtcctcgataacagaccaccaccccttctgcacctttagtcaccaacagcatggcgatctcatactcttttgccagggcgcatatatcctgatcgttctgtgtttttccactgataagtcgccattcttcttccgagagcttgacgacatccgccagttgtagcgcctgccgcaaacacaagcggagcaaatgctcgtcttgccatagatcttcacgaatattaggatcgaagctgacaaaacctccggcatgccggatcgccgtcatcgcagtaaatgcgctggtacgcgaaggctcggcagacaacgcaattgaacagagatgtaaccattcgccatgtcgccagcagggcaagtctgtcgtctctaaaaaaagatcggcactggggcggaccataaacgtaaatgaacgttccccttgatcgttcagatcgacaagcaccgtggatgtccggtgccattcatcttgcttcagatacgtgatatcgactccctcagttagcagcgttctttgcattaacgcaccaaaaggatcatcccccacccgacctataaacccacttgttccgcctaatctggcgattcccaccgcaacgttagctggcgcgccgccaggacaaggcagtaggcgcccgtctgattctggcaagagatctacgaccgcatcccctaaaacccatactttggctgacatttttttcccttaaattcatctgagttacgcatagtgataaacctctttttcgcaaaatcgtcatggatttactaaaacatgcatattcgatcacaaaacgtcatagttaacgttaacatttgtgatattcatcgcatttatgaaagtaagggactttatttttataaaagttaacgttaacaattcaccaaatttgcttaaccaggatgattaaaatgacgcaatctcgattgcatgcggcgcaaaacgccctagcaaaacttcatgagcaccggggtaacactttctatccccattttcacctcgcgcctcctgccgggtggatgaacgatccaaacggcctgatctggtttaacgatcgttatcacgcgttttatcaacatcatccgatgagcgaacactgggggccaatgcactggggacatgccaccagcgacgatatgatccactggcagcatgagcctattgcgctagcgccaggagacgataatgacaaagacgggtgtttttcaggtagtgctgtcgatgacaatggtgtcctctcacttatctacaccggacacgtctggctcgatggtgcaggtaatgacgatgcaattcgcgaagtacaatgtctggctaccagtcgggatggtattcatttcgagaaacagggtgtgatcctcactccaccagaaggaatcatgcacttccgcgatcctaaagtgtggcgtgaagccgacacatggtggatggtagtcggggcgaaagatccaggcaacacggggcagatcctgctttatcgcggcagttcgttgcgtgaatggaccttcgatcgcgtactggcccacgctgatgcgggtgaaagctatatgtgggaatgtccggactttttcagccttggcgatcagcattatctgatgttttccccgcagggaatgaatgccgagggatacagttaccgaaatcgctttcaaagtggcgtaatacccggaatgtggtcgccaggacgactttttgcacaatccgggcattttactgaacttgataacgggcatgacttttatgcaccacaaagctttttagcgaaggatggtcggcgtattgttatcggctggatggatatgtgggaatcgccaatgccctcaaaacgtgaaggatgggcaggctgcatgacgctggcgcgcgagctatcagagagcaatggcaaacttctacaacgcccggtacacgaagctgagtcgttacgccagcagcatcaatctgtctctccccgcacaatcagcaataaatatgttttgcaggaaaacgcgcaagcagttgagattcagttgcagtgggcgctgaagaacagtgatgccgaacattacggattacagctcggcactggaatgcggctgtatattgataaccaatctgagcgacttgttttgtggcggtattacccacacgagaatttagacggctaccgtagtattcccctcccgcagcgtgacacgctcgccctaaggatatttatcgatacatcatccgtggaagtatttattaacgacggggaagcggtgatgagtagtcgaatctatccgcagccagaagaacgggaactgtcgctttatgcctcccacggagtggctgtgctgcaacatggagcactctggctactgggttaacataatatcaggtggaacaacggatcaacagcgggcaagggatccgcgtcactcttcccccttcacgaccttcaataatatgcaatgcagcttcccgcccgataatgtcatgtggaagctgaattgtggtcagcggcggtaaaaacagatgcccgacgccaaccagattatcaaagcccattacggcgacatcctgcgggattcgtacccccttcgccagaagaacctgataagccacaaaggctgcgcgatcgttaccacatatcagaacatcaaaatctggtttgcccggtttgaagtgggcattgagtaaacttgcgagatcggtgtagtgatcatcacctgttgccatgtgaaattgtttcacctcagccagatctcgtccagcatcacgccaggcctgctcaaatccctgccgacgataccctgttgccaacgcactttccggtagccagaagcataacggttgacgatagcccgccgcgagcaaatgctgtgttgattcatattgtgcagtgtaatcatcagggatataactgggtaacgctgggtcatccgccacacagttcgccaatacaatattttcaccatacagagactcaggcagcgtgatatgtcgcagccccattgtagtatagataatgccatccggacggtgggcaagcagctgacgtgccgcgcgggcagcgtcatcttcagaaaaaatattgattaaaaaactattccagccgaactcgctggcggtttgctcaatggcaagcagaatatcaacagagaaaggagtggtagccgtgtcctgcgccagcacggcgagagtcgacggcttacgtccttgagcgcgcatcttacgggcggaaagatcaggaacataattcagggtctggattgcctgcaatacgcggtcacgcgttgcaggacgcacagattctgcattatgcatcacccgggagactgtcatcatcgacactcccgccaggcgtgcgacatcctttaatgaagccatacccaagccgtttgccgtaaaacgggcactgtagcagaaacagacgtcactggcgagatccaacgccctatcacctgacacagcaatacaataaaaaataacaataattcccggacaattgtccccaattccgcctctgttctcgcattgtagaccggggacttatcagccaacctgt

SEQ ID NO: 3 - DNA, 3123 bp, Artificial Sequence
  Expression cassette
ctgtctcttatacacatctccggccagatgattaattcctaatttttgttgacactctatcattgatagagttattttaccactccctatcagtgatagagaaaagtgaaatgaatagttcgacaaaaatctagaaataattttgtttaactttaagaaggagatatacaaatgatcgctcaccgtcgtcaggaactggctcaacagtattatcaggctctgcaccaagatgtgctgccgttctgggaaaagtattcgctggatcgtcaaggcggtggctattttacctgcctggaccgcaagggtcaggtttttgatacggacaagttcatttggctgcaaaaccgtcaagtgtggcaatttgcggttttctacaatcgcctggaaccgaaaccgcagtggctggaaatcgctcgtcatggtgcggattttctggcacgtcacggtcgtgatcaggacggtaactggtatttcgccctggatcaggaaggcaaaccgctgcgccaaccgtacaatgtgttttccgactgtttcgcggcgatggcgtttagccagtatgcactggcttctggtgctcaagaagcgaaggccattgcactgcaagcgtataacaatgttctgcgtcgccagcataacccgaaaggtcaatatgaaaagagttacccgggtacccgtccgctgaaatccctggcagtgccgatgatcctggctaatctgacgctggaaatggaatggctgctgccgccgaccacggtcgaagaagtgctggcccagaccgttcgtgaagtcatgacggattttctggacccggaaattggcctgatgcgcgaagcagttaccccgacgggtgaatttgtcgattcattcgaaggccgcctgctgaacccgggtcatggcattgaagcgatgtggtttatgatggatattgcccagcgttcgggtgaccgccagctgcaagaacaggctattgcggtggttctgaataccctggaatatgcatgggatgaagaatttggtggcatcttttacttcctggaccgtcaaggtcacccgccgcagcaactggaatgggatcagaaactgtggtgggtccatctggaaaccctggtggccctggcaaaaggtcaccaggcgacgggccaagaaaagtgctggcagtggtttgaacgcgtgcatgattatgcatggagccactttgctgacccggaatatggtgaatggttcggctacctgaaccgtcgcggtgaagtgctgctgaatctgaaaggtggcaaatggaagggctgcttccacgttccgcgtgcgctgtggctgtgtgccgaaaccctgcaactgccggtctcttaataatcgaaggagatacaacatgagcttacccgatggattttatataaggcgaatggaagagggggatttggaacaggtcactgagacgctaaaggttttgaccaccgtgggcactattacccccgaatccttcagcaaactcataaaatactggaatgaagccacagtatggaatgataacgaagataaaaaaataatgcaatataaccccatggtgattgtggacaagcgcaccgagacggttgccgctacggggaatatcatcatcgaaagaaagatcattcatgaactggggctatgtggccacatcgaggacattgcagtaaactccaagtatcagggccaaggtttgggcaagctcttgattgatcaattggtaactatcggctttgactacggttgttataagattattttagattgcgatgagaaaaatgtcaaattctatgaaaaatgtgggtttagcaacgcaggcgtggaaatgcaaattagaaaatagaataactagcataaacccccttggggcctctaaacgggtcttgaggggttttttgctgaaaccaatttgcctggcggcagtagcgcggtggtcccacctgaccccatgccgaactcagaagtgaaacgccgtagcgccgatggtagtgtggggtctccccatgcgagagtagggaactgccaggcatcaaataaaacgaaaggctcagtcgaaagactgggcctttcgggatccaggccggcctgttaagacggccagtgaattcgagctcggtacctaccgttcgtataatgtatgctatacgaagttatcgagctctagagaatgatcccctcattaggccacacgttcaagtgcagcgcacaccgtggaaacggatgaaggcacgaacccagttgacataagcctgttcggttcgtaaactgtaatgcaagtagcgtatgcgctcacgcaactggtccagaaccttgaccgaacgcagcggtggtaacggcgcagtggcggttttcatggcttgttatgactgtttttttgtacagtctatgcctcgggcatccaagcagcaagcgcgttacgccgtgggtcgatgtttgatgttatggagcagcaacgatgttacgcagcagcaacgatgttacgcagcagggcagtcgccctaaaacaaagttaggtggctcaagtatgggcatcattcgcacatgtaggctcggccctgaccaagtcaaatccatgcgggctgctcttgatcttttcggtcgtgagttcggagacgtagccacctactcccaacatcagccggactccgattacctcgggaacttgctccgtagtaagacattcatcgcgcttgctgccttcgaccaagaagcggttgttggcgctctcgcggcttacgttctgcccaggtttgagcagccgcgtagtgagatctatatctatgatctcgcagtctccggcgagcaccggaggcagggcattgccaccgcgctcatcaatctcctcaagcatgaggccaacgcgcttggtgcttatgtgatctacgtgcaagcagattacggtgacgatcccgcagtggctctctatacaaagttgggcatacgggaagaagtgatgcactttgatatcgacccaagtaccgccacctaacaattcgttcaagccgagatcgtagaatttcgacgacctgcagccaagcataacttcgtataatgtatgctatacgaacggtaggatcctctagagtcgacctgcaggcatgagatgtgtataagagacag

SEQ ID NO: 4 - DNA, 2965 bp, Artificial Sequence
  Expression cassette
ctgtctcttatacacatctccggccagatgattaattcctaatttttgttgacactctatcattgatagagttattttaccactccctatcagtgatagagaaaagtgaaatgaatagttcgacaaaaatctagaaataattttgtttaactttaagaaggagatatacaaatgaaagaaatcaaaatccagaacatcatcatcagcgaagaaaaagcgccgctggttgtgccggaaatcggcattaaccataatggtagtctggaactggcaaaaatcatggtggatgcggcctttagcgccggtgcaaaaatcattaaacatcagacccacattgtggaagatgaaatgtctaaagcagcgaaaaaagttatcccgggcaacgcgaaaatcagtatctacgaaatcatgcagaaatgcgcgctggattacaaagatgaactggccctgaaagaatataccgaaaaactgggtctggtgtacctgtctaccccgtttagtcgtgcgggtgcaaaccgtctggaagatatgggtgttagtgcgttcaaaatcggcagcggtgaatgtaacaattatccgctgatcaaacatattgccgcatttaaaaaaccgatgattgttagcaccggcatgaatagcatcgaatctattaaaccgacggtgaaaatcctgctggataacgaaattccgtttgttctgatgcataccacgaatctgtacccgaccccgcacaacctggtgcgtctgaatgccatgctggaactgaaaaaagaattctcttgcatggttggtctgagtgatcacaccacggataatctggcatgcctgggtgcagtggttctgggtgcgtgtgtgctggaacgtcatttcaccgatagcatgcaccgctctggtccggatattgtttgtagtatggatacgaaagcactgaaagaactgatcattcagagcgaacagatggcgatcattcgcggcaacaatgaatctaaaaaagcggccaaacaggaacaggtgaccatcgattttgcattcgcgagtgtggttagcatcaaagatatcaaaaaaggcgaagtgctgagcatggataatatttgggttaaacgtccgggtctgggcggtatctctgcagcggaatttgaaaacattctgggcaaaaaagcactgcgcgatattgaaaatgatgcgcagctgtcttatgaagatttcgcctaataaatcgatactagcataaccccttggggcctctaaacgcgtcgacacgcaaaaaggccatccgtcaggatggccttctgcttaatttgatgcctggcagtttatggcgggcgtcctgcccgccaccctccgggccgttgcttcgcaacgttcaaatccgctcccggcggatttgtcctactcaggagagcgttcaccgacaaacaacagataaaacgaaaggcccagtctttcgactgagcctttcgttttatttgatgcctggcagttccctactctcgcatggggagaccccacactaccatccggtatcgataagcttgatggcgaaagggggatgtgctgcaaggcgattaagttgggtaacgccagggttttcccagtcacgacgttgtaaaacgacggccagtgaattcgagctcggtacctaccgttcgtataatgtatgctatacgaagttatcgagctctagagaatgatcccctccctcacgctgccgcaagcactcagggcgcaagggctgctaaaggaagcggaacacgtagaaagccagtccgcagaaacggtgctgaccccggatgaatgtcagctactgggctatctggacaagggaaaacgcaagcgcaaagagaaagcaggtagcttgcagtgggcttacatggcgatagctagactgggcggttttatggacagcaagcgaaccggaattgccagctggggcgccctctggtaaggttgggaagccctgcaaagtaaactggatggctttcttgccgccaaggatctgatggcgcaggggatcaagatctgatcaagagacaggatgaggatcgtttcgcatgattgaacaagatggattgcacgcaggttctccggccgcttgggtggagaggctattcggctatgactgggcacaacagacaatcggctgctctgatgccgccgtgttccggctgtcagcgcaggggcgcccggttctttttgtcaagaccgacctgtccggtgccctgaatgaactgcaggacgaggcagcgcggctatcgtggctggccacgacgggcgttccttgcgcagctgtgctcgacgttgtcactgaagcgggaagggactggctgctattgggcgaagtgccggggcaggatctcctgtcatctcaccttgctcctgccgagaaagtatccatcatggctgatgcaatgcggcggctgcatacgcttgatccggctacctgcccattcgaccaccaagcgaaacatcgcatcgagcgagcacgtactcggatggaagccggtcttgtcgatcaggatgatctggacgaagagcatcaggggctcgcgccagccgaactgttcgccaggctcaaggcgcgcatgcccgacggcgaggatctcgtcgtgacccatggcgatgcctgcttgccgaatatcatggtggaaaatggccgcttttctggattcatcgactgtggccggctgggtgtggcggaccgctatcaggacatagcgttggctacccgtgatattgctgaagagcttggcggcgaatgggctgaccgcttcctcgtgctttacggtatcgccgctcccgattcgcagcgcatcgccttctatcgccttcttgacgagttcttctgagcgggactctgggaatttcgacgacctgcagccaagcataacttcgtataatgtatgctatacgaacggtaggatcctctagagtcgacctgcaggcatgagatgtgtataagagacag

SEQ ID NO: 5 - DNA, 3904 bp, Artificial Sequence
  Expression cassette
ctgtctcttatacacatctccggccagatgattaattcctaatttttgttgacactctatcattgatagagttattttaccactccctatcagtgatagagaaaagtgaaatgaatagttcgacaaaaatctagaaataattttgtttaactttaagaaggagatatacaaatgatcgctcaccgtcgtcaggaactggctcaacagtattatcaggctctgcaccaagatgtgctgccgttctgggaaaagtattcgctggatcgtcaaggcggtggctattttacctgcctggaccgcaagggtcaggtttttgatacggacaagttcatttggctgcaaaaccgtcaagtgtggcaatttgcggttttctacaatcgcctggaaccgaaaccgcagtggctggaaatcgctcgtcatggtgcggattttctggcacgtcacggtcgtgatcaggacggtaactggtatttcgccctggatcaggaaggcaaaccgctgcgccaaccgtacaatgtgttttccgactgtttcgcggcgatggcgtttagccagtatgcactggcttctggtgctcaagaagcgaaggccattgcactgcaagcgtataacaatgttctgcgtcgccagcataacccgaaaggtcaatatgaaaagagttacccgggtacccgtccgctgaaatccctggcagtgccgatgatcctggctaatctgacgctggaaatggaatggctgctgccgccgaccacggtcgaagaagtgctggcccagaccgttcgtgaagtcatgacggattttctggacccggaaattggcctgatgcgcgaagcagttaccccgacgggtgaatttgtcgattcattcgaaggccgcctgctgaacccgggtcatggcattgaagcgatgtggtttatgatggatattgcccagcgttcgggtgaccgccagctgcaagaacaggctattgcggtggttctgaataccctggaatatgcatgggatgaagaatttggtggcatcttttacttcctggaccgtcaaggtcacccgccgcagcaactggaatgggatcagaaactgtggtgggtccatctggaaaccctggtggccctggcaaaaggtcaccaggcgacgggccaagaaaagtgctggcagtggtttgaacgcgtgcatgattatgcatggagccactttgctgacccggaatatggtgaatggttcggctacctgaaccgtcgcggtgaagtgctgctgaatctgaaaggtggcaaatggaagggctgcttccacgttccgcgtgcgctgtggctgtgtgccgaaaccctgcaactgccggtctcttaatttcgtcgacacacaggaaacatattaaaaattaaaacctgcaggagtttaaacgcggccgcgatatcgttgtaaaacgacggccagtgcaagaatcataaaaaatttatttgctttcaggaaaatttttctgtataatagattcataaatttgagagaggagtttttgtgagcggataacaattccccatcttagtatattagttaagtataaatacacaaggagatatacatatgaaagaaatcaaaatccagaacatcatcatcagcgaagaaaaagcgccgctggttgtgccggaaatcggcattaaccataatggtagtctggaactggcaaaaatcatggtggatgcggcctttagcgccggtgcaaaaatcattaaacatcagacccacattgtggaagatgaaatgtctaaagcagcgaaaaaagttatcccgggcaacgcgaaaatcagtatctacgaaatcatgcagaaatgcgcgctggattacaaagatgaactggccctgaaagaatataccgaaaaactgggtctggtgtacctgtctaccccgtttagtcgtgcgggtgcaaaccgtctggaagatatgggtgttagtgcgttcaaaatcggcagcggtgaatgtaacaattatccgctgatcaaacatattgccgcatttaaaaaaccgatgattgttagcaccggcatgaatagcatcgaatctattaaaccgacggtgaaaatcctgctggataacgaaattccgtttgttctgatgcataccacgaatctgtacccgaccccgcacaacctggtgcgtctgaatgccatgctggaactgaaaaaagaattctcttgcatggttggtctgagtgatcacaccacggataatctggcatgcctgggtgcagtggttctgggtgcgtgtgtgctggaacgtcatttcaccgatagcatgcaccgctctggtccggatattgtttgtagtatggatacgaaagcactgaaagaactgatcattcagagcgaacagatggcgatcattcgcggcaacaatgaatctaaaaaagcggccaaacaggaacaggtgaccatcgattttgcattcgcgagtgtggttagcatcaaagatatcaaaaaaggcgaagtgctgagcatggataatatttgggttaaacgtccgggtctgggcggtatctctgcagcggaatttgaaaacattctgggcaaaaaagcactgcgcgatattgaaaatgatgcgcagctgtcttatgaagatttcgcctaaaataactagcataaccccttggggcctctaaacgggtcttgaggggttttttgctgaaaccaatttgcctggcggcagtagcgcggtggtcccacctgaccccatgccgaactcagaagtgaaacgccgtagcgccgatggtagtgtggggtctccccatgcgagagtagggaactgccaggcatcaaataaaacgaaaggctcagtcgaaagactgggcctttcgggatccaggccggcctgttaacgaattaatcttccgcggcggtatcgataagcttgatatcgaattccgaagttcctattctctagaaagtataggaacttcaggtctgaagaggagtttacgtccagccaagctagcttggctgcaggtcgtcgaaattctaccgggtaggggaggcgcttttcccaaggcagtctggagcatgcgctttagcagccccgctgggcacttggcgctacacaagtggcctctggcctcgcacacattccacatccaccggtaggcgccaaccggctccgttctttggtggccccttcgcgccaccttctactcctcccctagtcaggaagttcccccccgccccgcagctcgcgtcgtgcaggacgtgacaaatggaagtagcacgtctcactagtctcgtgcagatggacagcaccgctgagcaatggaagcgggtaggcctttggggcagcggccaatagcagctttgctccttcgctttctgggctcaggggcgggctcagggggcggggcgggcgcccgaaggtcctccggaggcccggcattctgcacgcttcaaaagcgcacgtctgccgcgctgttctcctcttcctcatctccgggcctttcgacctgcagcctgttgacaattaatcatcggcatagtatatcggcatagtataatacgacaaggtgaggaactaaaccatgggtcaaagtagcgatgaagccaacgctcccgttgcagggcagtttgcgcttcccctgagtgccacctttggcttaggggatcgcgtacgcaagaaatctggtgccgcttggcagggtcaagtcgtcggttggtattgcacaaaactcactcctgaaggctatgcggtcgagtccgaatcccacccaggctcagtgcaaatttatcctgtggctgcacttgaacgtgtggcctaatgaggggatcaattctctagagctcgctgatcagaagttcctattctctagaaagtataggaacttcgatggcgcctcatccctgaagccaaagatgtgtataagagacag

SEQ ID NO: 6 - DNA, 3793 bp, Artificial Sequence
  expression cassette
ctgtctcttatacacatctccggccagatgattaattcctaatttttgttgacactctatcattgatagagttattttaccactccctatcagtgatagagaaaagtgaaatgaatagttcgacaaaaatctagaaataattttgtttggcgtcgagaaggagatagaaaatgtgcggtatcgttggtgctatcgcacagcgtgatgtagcgaaaatcctcctggaaggtctgcgtcgtctcgaataccgtggttacgactctgccggtctggcagtagtggatgcagaaggtcacatgactcgtctgcgtcgtctgggtaaagtgcagatgctcgcgcaggcggcggaagaacacccactccacggtggtacgggtatcgcacacactcgttgggcaacccacggtgaaccgtctgaggtcaacgcacacccgcatgttagcgagcacatcgtagtcgttcacaacggtatcatcgagaaccacgaaccactccgtgaggaactcaaagcccgtggttacaccttcgtaagcgaaaccgacacggaagttatcgcccacctcgttaactgggaactcaaacagggtggtactctgcgtgaagcagttctgcgtgccattccacagctgcgtggtgcatacggtaccgtgatcatggactctcgtcatccggataccctgctcgccgcacgttctggttctccactcgttatcggtctgggtatgggtgagaacttcatcgcctctgatcagctggccctgctcccagttacccgtcgcttcatcttcctggaagagggtgacatcgccgaaatcacccgtcgttccgttaacatcttcgacaaaacgggtgcggaagttaaacgtcaggacatcgagtctaacctgcagtatgacgctggtgacaaaggcatctaccgtcactacatgcagaaagagatctacgaacagccgaacgcgatcaaaaacaccctgaccggtcgtatctctcacggtcaggttgacctgtctgagctgggtccaaacgcggacgaactcctgtccaaagtcgagcacatccagatcctggcttgtggtacctcttacaactccggtatggtttctcgttactggttcgaatctctggcaggtatcccatgcgacgttgaaatcgcctccgaattccgttatcgtaaatctgcggtacgtcgtaactccctcatgatcaccctgtctcagtctggtgaaaccgctgatactctggcaggtctgcgtctcagcaaagaactgggttacctgggttctctggccatctgcaacgttccgggttctagcctggttcgtgagtctgtgctggctctgatgaccaacgcgggtacggagatcggtgttgcctctaccaaagcgttcactacccagctcactgtcctgctgatgctggttgccaaactgtctcgtctcaaaggcctcgacgctagcatcgaacacgacatcgtacacggtctgcaggccctcccatctcgtatcgagcagatgctgccgcaggacaaacgtatcgaagcactggcagaagacttcagcgacaaacaccacgcgctgtttctgggtcgtggtgaccagtacccaattgcgctggaaggtgccctgaaactgaaagagatcagctacatccatgcagaggcatacgcagcgggtgagctgaaacatggtccactggccctgatcgacgcagatatgccggttattgtggttgctccgaacaacggcctgctggagaaactgaaatccaacatcgaggaagtacgtgcgcgtggtggtcagctgtacgtgtttgctgaccaggacgcgggtttcgtttccagcgacaacatgcacatcatcgaaatgccgcatgttgaagaggtaatcgcgccaatcttctacaccgtaccgctgcagctgctggcgtaccatgtagccctgatcaaaggtacggacgttgaccagccgcgtaacctggcgaaatccgtgaccgtggaataacgaaggagatagaaccatgagcttacccgatggattttatataaggcgaatggaagagggggatttggaacaggtcactgagacgctaaaggttttgaccaccgtgggcactattacccccgaatccttcagcaaactcataaaatactggaatgaagccacagtatggaatgataacgaagataaaaaaataatgcaatataaccccatggtgattgtggacaagcgcaccgagacggttgccgctacggggaatatcatcatcgaaagaaagatcattcatgaactggggctatgtggccacatcgaggacattgcagtaaactccaagtatcagggccaaggtttgggcaagctcttgattgatcaattggtaactatcggctttgactacggttgttataagattattttagattgcgatgagaaaaatgtcaaattctatgaaaaatgtgggtttagcaacgcaggcgtggaaatgcaaattagaaaatagcatccgtatcggaaacactagcataaccccttggggcctctaaacgggtcttgaggggttttttgctgaaaccaatttgcctggcggcagtagcgcggtggtcccacctgaccccatgccgaactcagaagtgaaacgccgtagcgccgatggtagtgtggggtctccccatgcgagagtagggaactgccaggcatcaaataaaacgaaaggctcagtcgaaagactgggcctttcgcttccacaactttgtataataaagttgtccccacggccagtgaattcgagctcggtacctaccgttcgtataatgtatgctatacgaagttatcgagctctagagaatgatcccctcattaggccacacgttcaagtgcagcgcacaccgtggaaacggatgaaggcacgaacccagttgacataagcctgttcggttcgtaaactgtaatgcaagtagcgtatgcgctcacgcaactggtccagaaccttgaccgaacgcagcggtggtaacggcgcagtggcggttttcatggcttgttatgactgtttttttgtacagtctatgcctcgggcatccaagcagcaagcgcgttacgccgtgggtcgatgtttgatgttatggagcagcaacgatgttacgcagcagcaacgatgttacgcagcagggcagtcgccctaaaacaaagttaggtggctcaagtatgggcatcattcgcacatgtaggctcggccctgaccaagtcaaatccatgcgggctgctcttgatcttttcggtcgtgagttcggagacgtagccacctactcccaacatcagccggactccgattacctcgggaacttgctccgtagtaagacattcatcgcgcttgctgccttcgaccaagaagcggttgttggcgctctcgcggcttacgttctgcccaggtttgagcagccgcgtagtgagatctatatctatgatctcgcagtctccggcgagcaccggaggcagggcattgccaccgcgctcatcaatctcctcaagcatgaggccaacgcgcttggtgcttatgtgatctacgtgcaagcagattacggtgacgatcccgcagtggctctctatacaaagttgggcatacgggaagaagtgatgcactttgatatcgacccaagtaccgccacctaacaattcgttcaagccgagatcgtagaatttcgacgacctgcagccaagcataacttcgtataatgtatgctatacgaacggtaggatcctctagagtcgacctgcaggcatgagatgtgtataagagacag

SEQ ID NO: 7 - DNA, 3847 bp, Artificial Sequence
  Expression cassette
ctgtctcttatacacatctccggccagatgattaattcctaatttttgttgacactctatcattgatagagttattttaccactccctatcagtgatagagaaaagtgaaatgaatagttcgacaaaaatctagaaataattttgtttggcgtcgagaaggagatagaaccatgtccaacaatggctcgtcaccgctggtgctttggtataaccaactcggcatgaatgatgtagacagggttgggggcaaaaatgcctccctgggtgaaatgattactaacctttccggaatgggtgtttccgttccgaatggtttcgccacaaccgccgacgcgtttaaccagtttctggaccaaagcggcgtaaaccagcgcatttatgaactgctggataaaacggatattgacgatgttactcagcttgcgaaagcgggcgcgcaaatccgccagtggattatcgacactcccttccagcctgagctggaaaacgccatcagcgaagcctatgcacagctttctgccgatgacgaaaacgcctcttttgcggtgcgctcctccgccaccgcagaagatatgccggacgcttcttttgccggtcagcaggaaaccttcctcaacgttcagggttttgacgccgttctcgtggcagtgaaacatgtatttgcttctctgtttaacgatcgcgccatctcttatcgtgtgcaccagggttacgatcaccgtggtgtggcgctctccgccggtgttcaacggatggtgcgctctgacctcgcatcatctggcgtgatgttctccattgataccgaatccggctttgaccaggtggtgtttatcacttccgcatggggccttggtgagatggtcgtgcagggtgcggttaacccggatgagttttacgtgcataaaccgacactggcggcgaatcgcccggctatcgtgcgccgcaccatggggtcgaaaaaaatccgcatggtttacgcgccgacccaggagcacggcaagcaggttaaaatcgaagacgtaccgcaggaacagcgtgacatcttctcgctgaccaacgaagaagtgcaggaactggcaaaacaggccgtacaaattgagaaacactacggtcgcccgatggatattgagtgggcgaaagatggccacaccggtaaactgttcattgtgcaggcgcgtccggaaaccgtgcgctcacgcggtcaggtcatggagcgttatacgctgcattcacagggtaagattatcgccgaaggccgtgctatcggtcatcgcatcggtgcgggtccggtgaaagtcatccatgatatcagcgaaatgaaccgcatcgaacctggtgacgtgctggtcactgacatgaccgacccggactgggaaccgatcatgaagaaagcatctgccatcgtcaccaaccgtggcggtcgtacctgtcacgcggcgatcatcgctcgtgaactgggcattccggcggtagtgggctgtggtgatgcaacagaacggatgaaagacggtgagaacgtcactgtttcttgtgccgaaggtgataccggttacgtctatgcggagttgctggaatttagcgtgaaaagctccagcgtagaaacgatgccggatctgccgttgaaagtgatgatgaacgtcggtaacccggaccgagctttcgacttcgcctgtctgccgaacgaaggcgtgggacttgcgcgtctggaatttatcatcaaccgtatgattggcgtccacccacgcgcactgcttgagtttgacgatcaggaaccgcagttgcaaaacgaaatccgcgagatgatgaaaggttttgattctccgcgtgaattttacgttggtcgtctgactgaagggatcgcgacgctgggtgccgcgttttatccgaagcgcgtcattgtccgtctctctgattttaaatcgaacgaatatgccaacctggtcggtggtgagcgttacgagccagatgaagagaacccgatgctcggcttccgtggcgcgggacgctatatttccgacagcttccgcgactgtttcgcgctggagtgcgaagcagtgaaacgtgtgcgcaacgacatggggctgaccaacgttgagatcatgatcccgttcgtgcgaaccgtagatcaggcgaaagcggtggttgaggaactggcgcgtcaggggctgaaacgtggtgagaacgggctgaaaatcatcatgatgtgtgaaatcccgtccaacgccttgctggccgagcagttcctcgaatatttcgacggcttctcaattggctcaaacgacatgacgcagctggcgctcggtctggatcgtgactccggcgtggtgtctgaactgttcgatgagcgcaacgatgcggtgaaagcactgctgtcgatggcgattcgtgccgcgaagaaacagggcaaatatgtcgggatttgcggtcagggtccgtccgaccacgaagactttgccgcatggttgatggaagaggggatcgatagcctgtctctgaacccggacaccgtggtgcaaacctggttaagcctggctgaactgaagaaataacatccgtatcggaaacactagcataaccccttggggcctctaaacgggtcttgaggggttttttgctgaaaccaatttgcctggcggcagtagcgcggtggtcccacctgaccccatgccgaactcagaagtgaaacgccgtagcgccgatggtagtgtggggtctccccatgcgagagtagggaactgccaggcatcaaataaaacgaaaggctcagtcgaaagactgggcctttcgcttccacaactttgtataataaagttgtccccacggccagtgaattcgagctcggtacctaccgttcgtataatgtatgctatacgaagttatcgagctctagagaatgatcccctcattaggccacacgttcaagtgcagcgcacaccgtggaaacggatgaaggcacgaacccagttgacataagcctgttcggttcgtaaactgtaatgcaagtagcgtatgcgctcacgcaactggtccagaaccttgaccgaacgcagcggtggtaacggcgcagtggcggttttcatggcttgttatgactgtttttttgtacagtctatgcctcgggcatccaagcagcaagcgcgttacgccgtgggtcgatgtttgatgttatggagcagcaacgatgttacgcagcagcaacgatgttacgcagcagggcagtcgccctaaaacaaagttaggtggctcaagtatgggcatcattcgcacatgtaggctcggccctgaccaagtcaaatccatgcgggctgctcttgatcttttcggtcgtgagttcggagacgtagccacctactcccaacatcagccggactccgattacctcgggaacttgctccgtagtaagacattcatcgcgcttgctgccttcgaccaagaagcggttgttggcgctctcgcggcttacgttctgcccaggtttgagcagccgcgtagtgagatctatatctatgatctcgcagtctccggcgagcaccggaggcagggcattgccaccgcgctcatcaatctcctcaagcatgaggccaacgcgcttggtgcttatgtgatctacgtgcaagcagattacggtgacgatcccgcagtggctctctatacaaagttgggcatacgggaagaagtgatgcactttgatatcgacccaagtaccgccacctaacaattcgttcaagccgagatcgtagaatttcgacgacctgcagccaagcataacttcgtataatgtatgctatacgaacggtaggatcctctagagtcgacctgcaggcatgagatgtgtataagagacag

SEQ ID NO: 8 - DNA, 5554 bp, Artificial Sequence
  Plasmid
catcgatttattatgacaacttgacggctacatcattcactttttcttcacaaccggcacggaactcgctcgggctggccccggtgcattttttaaatacccgcgagaaatagagttgatcgtcaaaaccaacattgcgaccgacggtggcgataggcatccgggtggtgctcaaaagcagcttcgcctggctgatacgttggtcctcgcgccagcttaagacgctaatccctaactgctggcggaaaagatgtgacagacgcgacggcgacaagcaaacatgctgtgcgacgctggcgatatcaaaattgctgtctgccaggtgatcgctgatgtactgacaagcctcgcgtacccgattatccatcggtggatggagcgactcgttaatcgcttccatgcgccgcagtaacaattgctcaagcagatttatcgccagcagctccgaatagcgcccttccccttgcccggcgttaatgatttgcccaaacaggtcgctgaaatgcggctggtgcgcttcatccgggcgaaagaaccccgtattggcaaatattgacggccagttaagccattcatgccagtaggcgcgcggacgaaagtaaacccactggtgataccattcgcgagcctccggatgacgaccgtagtgatgaatctctcctggcgggaacagcaaaatatcacccggtcggcaaacaaattctcgtccctgatttttcaccaccccctgaccgcgaatggtgagattgagaatataacctttcattcccagcggtcggtcgataaaaaaatcgagataaccgttggcctcaatcggcgttaaacccgccaccagatgggcattaaacgagtatcccggcagcaggggatcattttgcgcttcagccatacttttcatactcccgccattcagagaagaaaccaattgtccatattgcatcagacattgccgtcactgcgtcttttactggctcttctcgctaaccaaaccggtaaccccgcttattaaaagcattctgtaacaaagcgggaccaaagccatgacaaaaacgcgtaacaaaagtgtctataatcacggcagaaaagtccacattgattatttgcacggcgtcacactttgctatgccatagcatttttatccataagattagcggatcctacctgacgctttttatcgcaactctctactgtttctccatacccgtttttttgggaattcgagctctaaggaggttataaaaaatgtctaatctgctgacggtccaccaaaacctgccggctctgccggtcgatgctacctctgatgaagttcgcaaaaacctgatggatatgtttcgtgatcgccaggcattcagcgaacatacctggaaaatgctgctgtccgtgtgccgttcatgggcggcctggtgtaaactgaacaatcgcaaatggtttccggcggaaccggaagatgtccgtgactatctgctgtacctgcaggcccgcggtctggcagttaaaacgatccagcaacatctgggccaactgaatatgctgcaccgtcgctccggtctgccgcgtccgagcgattctaatgcggtgtcactggttatgcgtcgcattcgtaaagaaaacgtggatgcaggcgaacgcgctaaacaggcactggcttttgaacgtaccgatttcgaccaagttcgctcgctgatggaaaacagcgatcgttgccaggacatccgcaatctggcgttcctgggtattgcctataacaccctgctgcgcattgcagaaatcgctcgtattcgcgtgaaagatatcagccgtacggacggcggtcgcatgctgattcacatcggccgtaccaaaacgctggtctctaccgcaggcgtggaaaaagctctgagtctgggtgtgacgaaactggttgaacgctggattagtgtctccggcgtggcggatgacccgaacaattacctgttttgtcgtgttcgcaaaaatggtgtcgcagctccgtcagccacctcgcagctgagcacgcgtgcactggaaggcatcttcgaagctacccatcgcctgatttatggcgccaaagatgactcgggtcaacgttacctggcgtggtctggtcacagtgcacgtgttggtgccgcacgtgatatggcccgtgccggtgtttccatcccggaaattatgcaggcaggcggttggaccaacgttaatatcgtcatgaactatattcgcaatctggactcggaaacgggtgctatggttcgcctgctggaagacggtgactaatgagtgccggagttcatcgaaaaaatggacgaggcactggctgaaattggttttgtatttggggagcaatggcgatgacgcatcctcacgataatatccgggtaggcgcaatcactttcgtctactccgttacaaagcgaggctgggtatttcccggcctttctgttatccgaaatccactgaaagcacagcggctggctgaggagataaataataaacgaggggctgtatgcacaaagcatcttctgttgagttaagaacgagtatcgagatggcacatagccttgctcaaattggaatcaggtttgtgccaataccagtagaaacagacgaagaatccatgggtatggacagttttccctttgatatgtaacggtgaacagttgttctacttttgtttgttagtcttgatgcttcactgatagatacaagagccataagaacctcagatccttccgtatttagccagtatgttctctagtgtggttcgttgtttttgcgtgagccatgagaacgaaccattgagatcatacttactttgcatgtcactcaaaaattttgcctcaaaactggtgagctgaatttttgcagttaaagcatcgtgtagtgtttttcttagtccgttacgtaggtaggaatctgatgtaatggttgttggtattttgtcaccattcatttttatctggttgttctcaagttcggttacgagatccatttgtctatctagttcaacttggaaaatcaacgtatcagtcgggcggcctcgcttatcaaccaccaatttcatattgctgtaagtgtttaaatctttacttattggtttcaaaacccattggttaagccttttaaactcatggtagttattttcaagcattaacatgaacttaaattcatcaaggctaatctctatatttgccttgtgagttttcttttgtgttagttcttttaataaccactcataaatcctcatagagtatttgttttcaaaagacttaacatgttccagattatattttatgaatttttttaactggaaaagataaggcaatatctcttcactaaaaactaattctaatttttcgcttgagaacttggcatagtttgtccactggaaaatctcaaagcctttaaccaaaggattcctgatttccacagttctcgtcatcagctctctggttgctttagctaatacaccataagcattttccctactgatgttcatcatctgagcgtattggttataagtgaacgataccgtccgttctttccttgtagggttttcaatcgtggggttgagtagtgccacacagcataaaattagcttggtttcatgctccgttaagtcatagcgactaatcgctagttcatttgctttgaaaacaactaattcagacatacatctcaattggtctaggtgattttaatcactataccaattgagatgggctagtcaatgataattactagtccttttcctttgagttgtgggtatctgtaaattctgctagacctttgctggaaaacttgtaaattctgctagaccctctgtaaattccgctagacctttgtgtgttttttttgtttatattcaagtggttataatttatagaataaagaaagaataaaaaaagataaaaagaatagatcccagccctgtgtataactcactactttagtcagttccgcagtattacaaaaggatgtcgcaaacgctgtttgctcctctacaaaacagaccttaaaaccctaaaggcttaagtagcaccctcgcaagctcggttgcggccgcaatcgggcaaatcgctgaatattccttttgtctccgaccatcaggcacctgagtcgctgtctttttcgtgacattcagttcgctgcgctcacggctctggcagtgaatgggggtaaatggcactacaggcgccttttatggattcatgcaaggaaactacccataatacaagaaaagcccgtcacgggcttctcagggcgttttatggcgggtctgctatgtggtgctatctgactttttgctgttcagcagttcctgccctctgattttccagtctgaccacttcggattatcccgtgacaggtcattcagactggctaatgcacccagtaaggcagcggtatcatcaacggggtctgacgctcagtggaacgaaaactcacgttaagggattttggtcatgagattatcaaaaaggatcttcacctagatccttttaaattaaaaatgaagttttaaatcaatctaaagtatatatgagtaaacttggtctgacagttaccaatgcttaatcagtgaggcacctatctcagcgatctgtctatttcgttcatccatagttgcctgactccccgtcgtgtagataactacgatacgggagggcttaccatctggccccagtgctgcaatgataccgcgagacccacgctcaccggctccagatttatcagcaataaaccagccagccggaagggccgagcgcagaagtggtcctgcaactttatccgcctccatccagtctattaattgttgccgggaagctagagtaagtagttcgccagttaatagtttgcgcaacgttgttgccattgctacaggcatcgtggtgtcacgctcgtcgtttggtatggcttcattcagctccggttcccaacgatcaaggcgagttacatgatcccccatgttgtgcaaaaaagcggttagctccttcggtcctccgatcgttgtcagaagtaagttggccgcagtgttatcactcatggttatggcagcactgcataattctcttactgtcatgccatccgtaagatgcttttctgtgactggtgagtactcaaccaagtcattctgagaatagtgtatgcggcgaccgagttgctcttgcccggcgtcaatacgggataataccgcgccacatagcagaactttaaaagtgctcatcattggaaaacgttcttcggggcgaaaactctcaaggatcttaccgctgttgagatccagttcgatgtaacccactcgtgcacccaactgatcttcagcatcttttactttcaccagcgtttctgggtgagcaaaaacaggaaggcaaaatgccgcaaaaaagggaataagggcgacacggaaatgttgaatactcatactcttcctttttcaatattattgaagcatttatcagggttattgtctcatgagcggatacatatttgaatgtatttagaaaaataaacaaataggggttccgcgcacatttccccgaaaagtgccacctg

SEQ ID NO: 9 - DNA, 3436 bp, Artificial Sequence
  Expression cassette
ctgtctcttatacacatctccggccagatgattaattcctaatttttgttgacactctatcattgatagagttattttaccactccctatcagtgatagagaaaagtgaaatgaatagttcgacaaaaatctagaaataattttgtttaactttaagaaggagatatacaaatgaagaccgtgctggacaccctgaaaggtcgcctggttgtgagctgccaagcgctggaaaatgagccgctgcatagcccgtttattatgagccgtatggcgctggcggcgcgtcagggtggtgcggcggcgatccgtgcgaacagcgtggttgatatcgaggcgattaaggaacaagttaccctgccggtgatcggcatcattaagcgtgagtacccggatagcgaagttttcattaccgcgaccatgaaagaggtggacgaactgatgaccgtgagcccggcgatcattgcgctggatgcgaccgaccgtgcgcgtccgggtggcgagagcctggcgatgctggttacccgtatccgtacccgttatccgagcgtgctgctgatggcggatattgcgaccgttgacgaagcggtgaccgcgcaggcgctgggtttcgattgcgttggcaccaccctgtacggttataccgcgcagaccgtgggtcatgcgctgccggacgatgactgccaatttctgaaagcggttctggcggcggttaccgtgccggtggttgcggaaggcaacgtggacaccccggaacgtgcggcgcgttgcctggcgctgggtgcgcacatggtggttgtgggtggcgcgattacccgtccgcaacagattaccgaacgcttcatggcggcgattgatgcgcagagcaccgaccgtgcgtaatttcgtcgacacacaggaaacatattaaaaattaaaacctgcaggagtttaaacgcggccgcgatatcgttgtaaaacgacggccagtgcaagaatcataaaaaatttatttgctttcaggaaaatttttctgtataatagattcataaatttgagagaggagtttttgtgagcggataacaattccccatcttagtatattagttaagtataaatacacaaggagatatacatatgaaagaaatcaaaatccagaacatcatcatcagcgaagaaaaagcgccgctggttgtgccggaaatcggcattaaccataatggtagtctggaactggcaaaaatcatggtggatgcggcctttagcgccggtgcaaaaatcattaaacatcagacccacattgtggaagatgaaatgtctaaagcagcgaaaaaagttatcccgggcaacgcgaaaatcagtatctacgaaatcatgcagaaatgcgcgctggattacaaagatgaactggccctgaaagaatataccgaaaaactgggtctggtgtacctgtctaccccgtttagtcgtgcgggtgcaaaccgtctggaagatatgggtgttagtgcgttcaaaatcggcagcggtgaatgtaacaattatccgctgatcaaacatattgccgcatttaaaaaaccgatgattgttagcaccggcatgaatagcatcgaatctattaaaccgacggtgaaaatcctgctggataacgaaattccgtttgttctgatgcataccacgaatctgtacccgaccccgcacaacctggtgcgtctgaatgccatgctggaactgaaaaaagaattctcttgcatggttggtctgagtgatcacaccacggataatctggcatgcctgggtgcagtggttctgggtgcgtgtgtgctggaacgtcatttcaccgatagcatgcaccgctctggtccggatattgtttgtagtatggatacgaaagcactgaaagaactgatcattcagagcgaacagatggcgatcattcgcggcaacaatgaatctaaaaaagcggccaaacaggaacaggtgaccatcgattttgcattcgcgagtgtggttagcatcaaagatatcaaaaaaggcgaagtgctgagcatggataatatttgggttaaacgtccgggtctgggcggtatctctgcagcggaatttgaaaacattctgggcaaaaaagcactgcgcgatattgaaaatgatgcgcagctgtcttatgaagatttcgcctaaaataactagcataaccccttggggcctctaaacgggtcttgaggggttttttgctgaaaccaatttgcctggcggcagtagcgcggtggtcccacctgaccccatgccgaactcagaagtgaaacgccgtagcgccgatggtagtgtggggtctccccatgcgagagtagggaactgccaggcatcaaataaaacgaaaggctcagtcgaaagactgggcctttcgggatccaggccggcctgttaacgaattaatcttccgcggcggtatcgataagcttgatatcgaattccgaagttcctattctctagaaagtataggaacttcaggtctgaagaggagtttacgtccagccaagctagcttggctgcaggtcgtcgaaattctaccgggtaggggaggcgcttttcccaaggcagtctggagcatgcgctttagcagccccgctgggcacttggcgctacacaagtggcctctggcctcgcacacattccacatccaccggtaggcgccaaccggctccgttctttggtggccccttcgcgccaccttctactcctcccctagtcaggaagttcccccccgccccgcagctcgcgtcgtgcaggacgtgacaaatggaagtagcacgtctcactagtctcgtgcagatggacagcaccgctgagcaatggaagcgggtaggcctttggggcagcggccaatagcagctttgctccttcgctttctgggctcaggggcgggctcagggggcggggcgggcgcccgaaggtcctccggaggcccggcattctgcacgcttcaaaagcgcacgtctgccgcgctgttctcctcttcctcatctccgggcctttcgacctgcagcctgttgacaattaatcatcggcatagtatatcggcatagtataatacgacaaggtgaggaactaaaccatgggtcaaagtagcgatgaagccaacgctcccgttgcagggcagtttgcgcttcccctgagtgccacctttggcttaggggatcgcgtacgcaagaaatctggtgccgcttggcagggtcaagtcgtcggttggtattgcacaaaactcactcctgaaggctatgcggtcgagtccgaatcccacccaggctcagtgcaaatttatcctgtggctgcacttgaacgtgtggcctaatgaggggatcaattctctagagctcgctgatcagaagttcctattctctagaaagtataggaacttcgatggcgcctcatccctgaagccaaagatgtgtataagagacag

SEQ ID NO: 10 - DNA, 1830 bp, Escherichia coli
atgtgtggaattgttggcgcgatcgcgcaacgtgatgtagcagaaatccttcttgaaggtttacgtcgtctggaataccgcggatatgactctgccggtctggccgttgttgatgcagaaggtcatatgacccgcctgcgtcgcctcggtaaagtccagatgctggcacaggcagcggaagaacatcctctgcatggcggcactggtattgctcacactcgctgggcgacccacggtgaaccttcagaagtgaatgcgcatccgcatgtttctgaacacattgtggtggtgcataacggcatcatcgaaaaccatgaaccgctgcgtgaagagctaaaagcgcgtggctataccttcgtttctgaaaccgacaccgaagtgattgcccatctggtgaactgggagctgaaacaaggcgggactctgcgtgaggccgttctgcgtgctatcccgcagctgcgtggtgcgtacggtacagtgatcatggactcccgtcacccggataccctgctggcggcacgttctggtagtccgctggtgattggcctggggatgggcgaaaactttatcgcttctgaccagctggcgctgttgccggtgacccgtcgctttatcttccttgaagagggcgatattgcggaaatcactcgccgttcggtaaacatcttcgataaaactggcgcggaagtaaaacgtcaggatatcgaatccaatctgcaatatgacgcgggcgataaaggcatttaccgtcactacatgcagaaagagatctacgaacagccgaacgcgatcaaaaacacccttaccggacgcatcagccacggtcaggttgatttaagcgagctgggaccgaacgccgacgaactgctgtcgaaggttgagcatattcagatcctcgcctgtggtacttcttataactccggtatggtttcccgctactggtttgaatcgctagcaggtattccgtgcgacgtcgaaatcgcctctgaattccgctatcgcaaatctgccgtgcgtcgtaacagcctgatgatcaccttgtcacagtctggcgaaaccgcggataccctggctggcctgcgtctgtcgaaagagctgggttaccttggttcactggcaatctgtaacgttccgggttcttctctggtgcgcgaatccgatctggcgctaatgaccaacgcgggtacagaaatcggcgtggcatccactaaagcattcaccactcagttaactgtgctgttgatgctggtggcgaagctgtctcgcctgaaaggtctggatgcctccattgaacatgacatcgtgcatggtctgcaggcgctgccgagccgtattgagcagatgctgtctcaggacaaacgcattgaagcgctggcagaagatttctctgacaaacatcacgcgctgttcctgggccgtggcgatcagtacccaatcgcgctggaaggcgcattgaagttgaaagagatctcttacattcacgctgaagcctacgctgctggcgaactgaaacacggtccgctggcgctaattgatgccgatatgccggttattgttgttgcaccgaacaacgaattgctggaaaaactgaaatccaacattgaagaagttcgcgcgcgtggcggtcagttgtatgtcttcgccgatcaggatgcgggttttgtaagtagcgataacatgcacatcatcgagatgccgcatgtggaagaggtgattgcaccgatcttctacaccgttccgctgcagctgctggcttaccatgtcgcgctgatcaaaggcaccgacgttgaccagccgcgtaacctggcaaaatcggttacggttgagtaa

SEQ ID NO: 11 - protein, 609 aa, Escherichia coli
MCGIVGAIAQRDVAEILLEGLRRLEYRGYDSAGLAVVDAEGHMTRLRRLGKVQMLAQAAEEHPLHGGTGIAHTRWATHGEPSEVNAHPHVSEHIVVVHNGIIENHEPLREELKARGYTFVSETDTEVIAHLVNWELKQGGTLREAVLRAIPQLRGAYGTVIMDSRHPDTLLAARSGSPLVIGLGMGENFIASDQLALLPVTRRFIFLEEGDIAEITRRSVNIFDKTGAEVKRQDIESNLQYDAGDKGIYRHYMQKEIYEQPNAIKNTLTGRISHGQVDLSELGPNADELLSKVEHIQILACGTSYNSGMVSRYWFESLAGIPCDVEIASEFRYRKSAVRRNSLMITLSQSGETADTLAGLRLSKELGYLGSLAICNVPGSSLVRESDLALMTNAGTEIGVASTKAFTTQLTVLLMLVAKLSRLKGLDASIEHDIVHGLQALPSRIEQMLSQDKRIEALAEDFSDKHHALFLGRGDQYPIALEGALKLKEISYIHAEAYAAGELKHGPLALIDADMPVIVVAPNNELLEKLKSNIEEVRARGGQLYVFADQDAGFVSSDNMHIIEMPHVEEVIAPIFYTVPLQLLAYHVALIKGTDVDQPRNLAKSVTVE

SEQ ID NO: 12 - DNA, 1830 bp, Escherichia coli
atgtgcggtatcgttggtgctatcgcacagcgtgatgtagcgaaaatcctcctggaaggtctgcgtcgtctcgaataccgtggttacgactctgccggtctggcagtagtggatgcagaaggtcacatgactcgtctgcgtcgtctgggtaaagtgcagatgctcgcgcaggcggcggaagaacacccactccacggtggtacgggtatcgcacacactcgttgggcaacccacggtgaaccgtctgaggtcaacgcacacccgcatgttagcgagcacatcgtagtcgttcacaacggtatcatcgagaaccacgaaccactccgtgaggaactcaaagcccgtggttacaccttcgtaagcgaaaccgacacggaagttatcgcccacctcgttaactgggaactcaaacagggtggtactctgcgtgaagcagttctgcgtgccattccacagctgcgtggtgcatacggtaccgtgatcatggactctcgtcatccggataccctgctcgccgcacgttctggttctccactcgttatcggtctgggtatgggtgagaacttcatcgcctctgatcagctggccctgctcccagttacccgtcgcttcatcttcctggaagagggtgacatcgccgaaatcacccgtcgttccgttaacatcttcgacaaaacgggtgcggaagttaaacgtcaggacatcgagtctaacctgcagtatgacgctggtgacaaaggcatctaccgtcactacatgcagaaagagatctacgaacagccgaacgcgatcaaaaacaccctgaccggtcgtatctctcacggtcaggttgacctgtctgagctgggtccaaacgcggacgaactcctgtccaaagtcgagcacatccagatcctggcttgtggtacctcttacaactccggtatggtttctcgttactggttcgaatctctggcaggtatcccatgcgacgttgaaatcgcctccgaattccgttatcgtaaatctgcggtacgtcgtaactccctcatgatcaccctgtctcagtctggtgaaaccgctgatactctggcaggtctgcgtctcagcaaagaactgggttacctgggttctctggccatctgcaacgttccgggttctagcctggttcgtgagtctgtgctggctctgatgaccaacgcgggtacggagatcggtgttgcctctaccaaagcgttcactacccagctcactgtcctgctgatgctggttgccaaactgtctcgtctcaaaggcctcgacgctagcatcgaacacgacatcgtacacggtctgcaggccctcccatctcgtatcgagcagatgctgccgcaggacaaacgtatcgaagcactggcagaagacttcagcgacaaacaccacgcgctgtttctgggtcgtggtgaccagtacccaattgcgctggaaggtgccctgaaactgaaagagatcagctacatccatgcagaggcatacgcagcgggtgagctgaaacatggtccactggccctgatcgacgcagatatgccggttattgtggttgctccgaacaacggcctgctggagaaactgaaatccaacatcgaggaagtacgtgcgcgtggtggtcagctgtacgtgtttgctgaccaggacgcgggtttcgtttccagcgacaacatgcacatcatcgaaatgccgcatgttgaagaggtaatcgcgccaatcttctacaccgtaccgctgcagctgctggcgtaccatgtagccctgatcaaaggtacggacgttgaccagccgcgtaacctggcgaaatccgtgaccgtggaataa

SEQ ID NO: 13 - protein, 609 aa, Escherichia coli
MCGIVGAIAQRDVAKILLEGLRRLEYRGYDSAGLAVVDAEGHMTRLRRLGKVQMLAQAAEEHPLHGGTGIAHTRWATHGEPSEVNAHPHVSEHIVVVHNGIIENHEPLREELKARGYTFVSETDTEVIAHLVNWELKQGGTLREAVLRAIPQLRGAYGTVIMDSRHPDTLLAARSGSPLVIGLGMGENFIASDQLALLPVTRRFIFLEEGDIAEITRRSVNIFDKTGAEVKRQDIESNLQYDAGDKGIYRHYMQKEIYEQPNAIKNTLTGRISHGQVDLSELGPNADELLSKVEHIQILACGTSYNSGMVSRYWFESLAGIPCDVEIASEFRYRKSAVRRNSLMITLSQSGETADTLAGLRLSKELGYLGSLAICNVPGSSLVRESVLALMTNAGTEIGVASTKAFTTQLTVLLMLVAKLSRLKGLDASIEHDIVHGLQALPSRIEQMLPQDKRIEALAEDFSDKHHALFLGRGDQYPIALEGALKLKEISYIHAEAYAAGELKHGPLALIDADMPVIVVAPNNGLLEKLKSNIEEVRARGGQLYVFADQDAGFVSSDNMHIIEMPHVEEVIAPIFYTVPLQLLAYHVALIKGTDVDQPRNLAKSVTVE

SEQ ID NO: 14 - DNA, 480 bp, Saccharomyces cerevisiae
atgagcttacccgatggattttatataaggcgaatggaagagggggatttggaacaggtcactgagacgctaaaggttttgaccaccgtgggcactattacccccgaatccttcagcaaactcataaaatactggaatgaagccacagtatggaatgataacgaagataaaaaaataatgcaatataaccccatggtgattgtggacaagcgcaccgagacggttgccgctacggggaatatcatcatcgaaagaaagatcattcatgaactggggctatgtggccacatcgaggacattgcagtaaactccaagtatcagggccaaggtttgggcaagctcttgattgatcaattggtaactatcggctttgactacggttgttataagattattttagattgcgatgagaaaaatgtcaaattctatgaaaaatgtgggtttagcaacgcaggcgtggaaatgcaaattagaaaatag

SEQ ID NO: 15 - protein, 159 aa, Saccharomyces cerevisiae
MSLPDGFYIRRMEEGDLEQVTETLKVLTTVGTITPESFSKLIKYWNEATVWNDNEDKKIMQYNPMVIVDKRTETVAATGNIIIERKIIHELGLCGHIEDIAVNSKYQGQGLGKLLIDQLVTIGFDYGCYKIILDCDEKNVKFYEKCGFSNAGVEMQIRK

SEQ ID NO: 16 - DNA, 567 bp, Escherichia coli
atgtacgagcgttatgcaggtttaatttttgatatggatggcacaatcctggatacggagcctacgcaccgtaaagcgtggcgcgaagtattagggcactacggtcttcagtacgatattcaggcgatgattgcgcttaatggatcgcccacctggcgtattgctcaggcaattattgagctgaatcaggccgatctcgacccgcatgcgttagcgcgtgaaaaaacagaagcagtaagaagtatgctgctggatagcgtcgaaccgcttcctcttgttgatgtggtgaaaagttggcatggtcgtcgcccaatggctgtaggaacggggagtgaaagcgccatcgctgaggcattgctggcgcacctgggattacgccattattttgacgccgtcgtcgctgccgatcacgtcaaacaccataaacccgcgccagacacatttttgttgtgcgcgcagcgtatgggcgtgcaaccgacgcagtgtgtggtctttgaagatgccgatttcggtattcaggcggcccgtgcagcaggcatggacgccgtggatgttcgcttgctgtga

SEQ ID NO: 17 - protein, 188 aa, Escherichia coli
MYERYAGLIFDMDGTILDTEPTHRKAWREVLGHYGLQYDIQAMIALNGSPTWRIAQAIIELNQADLDPHALAREKTEAVRSMLLDSVEPLPLVDVVKSWHGRRPMAVGTGSESAIAEALLAHLGLRHYFDAVVAADHVKHHKPAPDTFLLCAQRMGVQPTQCVVFEDADFGIQAARAAGMDAVDVRLL

SEQ ID NO: 18 - DNA, 600 bp, Escherichia coli
atgctctatatctttgatttaggtaatgtgattgtcgatatcgactttaaccgtgtgctgggagcctggagcgatttaacgcgtattccgctggcatcgcttaagaagagttttcatatgggggaggcgtttcatcagcatgagcgtggggaaattagcgacgaagcgttcgcagaggcgctgtgtcatgagatggctctaccgctaagctacgagcagttctctcacggctggcaggcggtgtttgttgcgctgcgcccggaagtgatcgccatcatgcataaactgcgtgagcaggggcatcgcgtggtggtgctttccaataccaaccgcctgcataccaccttctggccggaagaatacccggaaattcgtgatgctgctgaccatatctatctgtcgcaagatctggggatgcgcaaacctgaagcacgaatttaccagcatgttttgcaggcggaaggtttttcacccagcgatacggtctttttcgacgataacgccgataatatagaaggagccaatcagctgggcattaccagtattctggtgaaagataaaaccaccatcccggactatttcgcgaaggtgttatgctaa

SEQ ID NO: 19 - protein, 199 aa, Escherichia coli
MLYIFDLGNVIVDIDFNRVLGAWSDLTRIPLASLKKSFHMGEAFHQHERGEISDEAFAEALCHEMALPLSYEQFSHGWQAVFVALRPEVIAIMHKLREQGHRVVVLSNTNRLHTTFWPEEYPEIRDAADHIYLSQDLGMRKPEARIYQHVLQAEGFSPSDTVFFDDNADNIEGANQLGITSILVKDKTTIPDYFAKVLC

SEQ ID NO: 20 - DNA, 1266 bp, Bacteroides ovatus
atggatagtaagaataacattggtcattcagcagacatctctttaactgctgaattacccataccaatctataatggaaatacgattatggatttcaaaaaactggcaagtctgtacaaggatgagctcctggacaacgtccttcctttctggcttgaacattcacaagaccatgagtatggtggttacttcacctgtctggaccgtgaaggaaaagtattcgatacggataagtttatttggctgcaaagtcgtgaggtatggatgttctccatgctttacaacaaagtggagaaacgtcaggaatggctagactgtgccattcagggtggcgaatttctaaaaaaatatggacatgacggcaattataactggtatttttccctcgaccgttcgggtagaccattggtagaaccgtacaatatattctcgtatacattcgctaccatggctttcggacagttgagccttacaaccggtaatcaggaatatgcggacattgccaagaaaactttcgatataatcctttccaaagtggataatccgaaagggagatggaataagcttcatccgggtacccgtaatctgaagaactttgccttgccaatgatcctctgtaacttggcactggagatagagcatttattggatgaaacgtatctgcgggaaacaatggatacttgtatccatgaagtgatggaagttttctatcgtcctgaactcggaggtatcattgttgaaaacgtggacatagacggtaatttggtcgattgttttgaaggccgtcaggtgaccccgggacatgccattgaagcgatgtggtttatcatggatctaggcaagcgtctgaatcgtccggaattgatagagaaagccaaagagactactctcacgatgcttaattatggctgggacaagcaatatggaggtatctactattttatggatcgtaacggttgtcctccccaacaattggagtgggaccagaaactctggtgggtccatatcgaaacgcttatttccctgctgaaaggctatcaattgacgggagacaaaaaatgcttggaatggtttgaaaaggtacatgactacacttgggagcatttcaaggataaagaatatcctgaatggtatggctacttgaaccgaagaggcgaagtattgctaccactcaaaggaggaaaatggaaaggatgcttccatgtgccaagaggactgtatcagtgctggaaaacattagaagaaataaaaaatatagtatcctaa

SEQ ID NO: 21 - protein, 421 aa, Bacteroides ovatus
MDSKNNIGHSADISLTAELPIPIYNGNTIMDFKKLASLYKDELLDNVLPFWLEHSQDHEYGGYFTCLDREGKVFDTDKFIWLQSREVWMFSMLYNKVEKRQEWLDCAIQGGEFLKKYGHDGNYNWYFSLDRSGRPLVEPYNIFSYTFATMAFGQLSLTTGNQEYADIAKKTFDIILSKVDNPKGRWNKLHPGTRNLKNFALPMILCNLALEIEHLLDETYLRETMDTCIHEVMEVFYRPELGGIIVENVDIDGNLVDCFEGRQVTPGHAIEAMWFIMDLGKRLNRPELIEKAKETTLTMLNYGWDKQYGGIYYFMDRNGCPPQQLEWDQKLWWVHIETLISLLKGYQLTGDKKCLEWFEKVHDYTWEHFKDKEYPEWYGYLNRRGEVLLPLKGGKWKGCFHVPRGLYQCWKTLEEIKNIVS

SEQ ID NO: 22 - DNA, 1176 bp, Synechocystis PCC6803
atgattgcccatcgccgtcaggagttagcccagcaatattaccaggctttacaccaggacgtattgcccttttgggaaaaatattccctcgatcgccaggggggcggttactttacctgcttagaccgtaaaggccaggtttttgacacagataaattcatttggttacaaaaccgtcaggtatggcagtttgccgttttctacaaccgtttggaaccaaaaccccaatggttagaaattgcccgccatggtgctgattttttagctcgccacggccgagatcaagacggtaattggtattttgctttggatcaggaaggcaaacccctgcgtcaaccctataacgttttttccgattgcttcgccgccatggcctttagtcaatatgccttagccagtggggcgcaggaagctaaagccattgccctgcaggcctacaataacgtcctacgccgtcagcacaatcccaaaggtcaatacgagaagtcctatccaggtactagacccctcaaatccctggcggtgccgatgattttagccaacctcaccctggagatggaatggttattaccgcctactaccgtggaagaggtgttggcccaaaccgtcagagaagtgatgacggatttcctcgacccagaaataggattaatgcgggaagcggtgacccccacaggagaatttgttgatagttttgaagggcggttgctcaacccaggacacggcattgaagccatgtggttcatgatggacattgcccaacgctccggcgatcgccagttacaggagcaagccattgcagtggtgttgaacaccctggaatatgcctgggatgaagaatttggtggcatattttatttccttgatcgccagggccaccctccccaacaactggaatgggaccaaaagctctggtgggtacatttggaaaccctggttgccctagccaagggccaccaagccactggccaagaaaaatgttggcaatggtttgagcgggtccatgattacgcctggagtcatttcgccgatcctgagtatggggaatggtttggctacctgaatcgccggggagaggtgttactcaacctaaaaggggggaaatggaaagggtgcttccacgtgccccgagctctgtggctctgtgcggaaactctccaacttccggttagttaa

SEQ ID NO: 23 - protein, 391 aa, Synechocystis PCC6803
MIAHRRQELAQQYYQALHQDVLPFWEKYSLDRQGGGYFTCLDRKGQVFDTDKFIWLQNRQVWQFAVFYNRLEPKPQWLEIARHGADFLARHGRDQDGNWYFALDQEGKPLRQPYNVFSDCFAAMAFSQYALASGAQEAKAIALQAYNNVLRRQHNPKGQYEKSYPGTRPLKSLAVPMILANLTLEMEWLLPPTTVEEVLAQTVREVMTDFLDPEIGLMREAVTPTGEFVDSFEGRLLNPGHGIEAMWFMMDIAQRSGDRQLQEQAIAVVLNTLEYAWDEEFGGIFYFLDRQGHPPQQLEWDQKLWWVHLETLVALAKGHQATGQEKCWQWFERVHDYAWSHFADPEYGEWFGYLNRRGEVLLNLKGGKWKGCFHVPRALWLCAETLQLPVS

SEQ ID NO: 24 - DNA, 708 bp, Enterobacter cloacae
atgaaaactgtactggataccctgaagggaagactggtcgtctcctgtcaggcgcttgagaacgaaccgttgcatagcccgtttattatgtcgcggatggcgctggcggcgcgtcagggaggggctgcggccatccgtgccaacagcgtggtggatattgaggcgatcaaagagcaggttacgctgccggttattggcatcatcaagcgggagtaccccgacagcgaggtgtttatcaccgcaacgatgaaagaggtggatgaactgatgaccgtctccccggcgatcattgcgcttgatgcgaccgacagggcgcggcctggcggggaatctctggcaatgctggttacgcgcattcgtacccgttatccctcggtgctgcttatggctgatatagccactgttgatgaggccgtcacggcgcaggcgctggggtttgattgtgtcgggaccacgctttacggctacaccgcgcagaccgtcggccacgccttacccgatgatgactgtcagtttctgaaagcggtactggcagccgtcacggtaccggtggtggccgaaggtaacgtggacaccccggaacgcgccgccagatgtctggcgttgggggcgcatatggtggtggtgggcggggcaatcacccgcccgcagcagattacggaacgctttatggcggcaattgacgcgcaaagcaccgatcgagcatga

SEQ ID NO: 25 - protein, 235 aa, Enterobacter cloacae
MKTVLDTLKGRLVVSCQALENEPLHSPFIMSRMALAARQGGAAAIRANSVVDIEAIKEQVTLPVIGIIKREYPDSEVFITATMKEVDELMTVSPAIIALDATDRARPGGESLAMLVTRIRTRYPSVLLMADIATVDEAVTAQALGFDCVGTTLYGYTAQTVGHALPDDDCQFLKAVLAAVTVPVVAEGNVDTPERAARCLALGAHMVVVGGAITRPQQITERFMAAIDAQSTDRA

SEQ ID NO: 26 - DNA, 2652 bp, Escherichia coli
atgaacgaacaatattccgcattgcgtagtaatgtcagtatgctcggcaaagtgctgggagaaaccatcaaggatgcgttgggagaacacattcttgaacgcgtagaaactatccgtaagttgtcgaaatcttcacgcgctggcaatgatgctaaccgccaggagttgctcaccaccttacaaaatttgtcgaacgacgagctgctgcccgttgcgcgtgcgtttagtcagttcctgaacctggccaacaccgccgagcaataccacagcatttcgccgaaaggcgaagctgccagcaacccggaagtgatcgcccgcaccctgcgtaaactgaaaaaccagccggaactgagcgaagacaccatcaaaaaagcagtggaatcgctgtcgctggaactggtcctcacggctcacccaaccgaaattacccgtcgtacactgatccacaaaatggtggaagtgaacgcctgtttaaaacagctcgataacaaagatatcgctgactacgaacacaaccagctgatgcgtcgcctgcgccagttgatcgcccagtcatggcataccgatgaaatccgtaagctgcgtccaagcccggtagatgaagccaaatggggctttgccgtagtggaaaacagcctgtggcaaggcgtaccaaattacctgcgcgaactgaacgaacaactggaagagaacctcggctacaaactgcccgtcgaatttgttccggtccgttttacttcgtggatgggcggcgaccgcgacggcaacccgaacgtcactgccgatatcacccgccacgtcctgctactcagccgctggaaagccaccgatttgttcctgaaagatattcaggtgctggtttctgaactgtcgatggttgaagcgacccctgaactgctggcgctggttggcgaagaaggtgccgcagaaccgtatcgctatctgatgaaaaacctgcgttctcgcctgatggcgacacaggcatggctggaagcgcgcctgaaaggcgaagaactgccaaaaccagaaggcctgctgacacaaaacgaagaactgtgggaaccgctctacgcttgctaccagtcacttcaggcgtgtggcatgggtattatcgccaacggcgatctgctcgacaccctgcgccgcgtgaaatgtttcggcgtaccgctggtccgtattgatatccgtcaggagagcacgcgtcataccgaagcgctgggcgagctgacccgctacctcggtatcggcgactacgaaagctggtcagaggccgacaaacaggcgttcctgatccgcgaactgaactccaaacgtccgcttctgccgcgcaactggcaaccaagcgccgaaacgcgcgaagtgctcgatacctgccaggtgattgccgaagcaccgcaaggctccattgccgcctacgtgatctcgatggcgaaaacgccgtccgacgtactggctgtccacctgctgctgaaagaagcgggtatcgggtttgcgatgccggttgctccgctgtttgaaaccctcgatgatctgaacaacgccaacgatgtcatgacccagctgctcaatattgactggtatcgtggcctgattcagggcaaacagatggtgatgattggctattccgactcagcaaaagatgcgggagtgatggcagcttcctgggcgcaatatcaggcacaggatgcattaatcaaaacctgcgaaaaagcgggtattgagctgacgttgttccacggtcgcggcggttccattggtcgcggcggcgcacctgctcatgcggcgctgctgtcacaaccgccaggaagcctgaaaggcggcctgcgcgtaaccgaacagggcgagatgatccgctttaaatatggtctgccagaaatcaccgtcagcagcctgtcgctttataccggggcgattctggaagccaacctgctgccaccgccggagccgaaagagagctggcgtcgcattatggatgaactgtcagtcatctcctgcgatgtctaccgcggctacgtacgtgaaaacaaagattttgtgccttacttccgctccgctacgccggaacaagaactgggcaaactgccgttgggttcacgtccggcgaaacgtcgcccaaccggcggcgtcgagtcactacgcgccattccgtggatcttcgcctggacgcaaaaccgtctgatgctccccgcctggctgggtgcaggtacggcgctgcaaaaagtggtcgaagacggcaaacagagcgagctggaggctatgtgccgcgattggccattcttctcgacgcgtctcggcatgctggagatggtcttcgccaaagcagacctgtggctggcggaatactatgaccaacgcctggtagacaaagcactgtggccgttaggtaaagagttacgcaacctgcaagaagaagacatcaaagtggtgctggcgattgccaacgattcccatctgatggccgatctgccgtggattgcagagtctattcagctacggaatatttacaccgacccgctgaacgtattgcaggccgagttgctgcaccgctcccgccaggcagaaaaagaaggccaggaaccggatcctcgcgtcgaacaagcgttaatggtcactattgccgggattgcggcaggtatgcgtaataccggctaa

SEQ ID NO: 27 - protein, 883 aa, Escherichia coli
MNEQYSALRSNVSMLGKVLGETIKDALGEHILERVETIRKLSKSSRAGNDANRQELLTTLQNLSNDELLPVARAFSQFLNLANTAEQYHSISPKGEAASNPEVIARTLRKLKNQPELSEDTIKKAVESLSLELVLTAHPTEITRRTLIHKMVEVNACLKQLDNKDIADYEHNQLMRRLRQLIAQSWHTDEIRKLRPSPVDEAKWGFAVVENSLWQGVPNYLRELNEQLEENLGYKLPVEFVPVRFTSWMGGDRDGNPNVTADITRHVLLLSRWKATDLFLKDIQVLVSELSMVEATPELLALVGEEGAAEPYRYLMKNLRSRLMATQAWLEARLKGEELPKPEGLLTQNEELWEPLYACYQSLQACGMGIIANGDLLDTLRRVKCFGVPLVRIDIRQESTRHTEALGELTRYLGIGDYESWSEADKQAFLIRELNSKRPLLPRNWQPSAETREVLDTCQVIAEAPQGSIAAYVISMAKTPSDVLAVHLLLKEAGIGFAMPVAPLFETLDDLNNANDVMTQLLNIDWYRGLIQGKQMVMIGYSDSAKDAGVMAASWAQYQAQDALIKTCEKAGIELTLFHGRGGSIGRGGAPAHAALLSQPPGSLKGGLRVTEQGEMIRFKYGLPEITVSSLSLYTGAILEANLLPPPEPKESWRRIMDELSVISCDVYRGYVRENKDFVPYFRSATPEQELGKLPLGSRPAKRRPTGGVESLRAIPWIFAWTQNRLMLPAWLGAGTALQKVVEDGKQSELEAMCRDWPFFSTRLGMLEMVFAKADLWLAEYYDQRLVDKALWPLGKELRNLQEEDIKVVLAIANDSHLMADLPWIAESIQLRNIYTDPLNVLQAELLHRSRQAEKEGQEPDPRVEQALMVTIAGIAAGMRNTG

SEQ ID NO: 28 - DNA, 1041 bp, Campylobacter jejuni
atgaaagaaataaaaatacaaaatataatcataagtgaagaaaaagcacccttagtcgtgcctgaaataggcattaatcataatggcagtttagaactagctaaaattatggtagatgcagcctttagcgcaggtgctaagattataaagcatcaaacccacatcgttgaagatgagatgagtaaggccgctaaaaaagtaattcctggtaatgcaaaaataagcatttatgagattatgcaaaaatgtgctttagattataaagatgagctagcacttaaagaatacacagaaaaattaggtcttgtttatcttagcacacctttttctcgtgcaggtgcaaaccgcttagaagatatgggagttagtgcttttaagattggttcaggtgagtgtaataattatccgcttattaaacacatagcagcctttaaaaagcctatgatagttagcacaggaatgaatagtattgaaagtataaaaccaactgtaaaaatcttattagacaatgaaattccctttgttttaatgcactcgaccaatctttacccaaccccgcataatcttgtaagattaaacgctatgcttgaattaaaaaaagaattttcttgcatggtaggcttaagcgaccacacaacagataatcttgcgtgtttaggtgcggttgcacttggtgcttgtgtgcttgaaagacattttactgatagtatgcatagaagtggccctgatatagtttgttctatggatacaaaggctttaaaagagctaattatccaaagtgagcaaatggctataatgaaaggaaataatgaaagcaaaaaagcagctaagcaagaacaagttacaattgattttgcctttgcaagcgtagttagcattaaagatattaaaaaaggcgaagttttatctatggacaatatctgggttaaaagacctggacttggtggaattagtgcggctgaatttgaaaatattttaggcaaaaaagcattaagagatatagaaaatgatactcagttaagctatgaggattttgcgtga

SEQ ID NO: 29 - protein, 346 aa, Campylobacter jejuni
MKEIKIQNIIISEEKAPLVVPEIGINHNGSLELAKIMVDAAFSAGAKIIKHQTHIVEDEMSKAAKKVIPGNAKISIYEIMQKCALDYKDELALKEYTEKLGLVYLSTPFSRAGANRLEDMGVSAFKIGSGECNNYPLIKHIAAFKKPMIVSTGMNSIESIKPTVKILLDNEIPFVLMHSTNLYPTPHNLVRLNAMLELKKEFSCMVGLSDHTTDNLACLGAVALGACVLERHFTDSMHRSGPDIVCSMDTKALKELIIQSEQMAIMKGNNESKKAAKQEQVTIDFAFASVVSIKDIKKGEVLSMDNIWVKRPGLGGISAAEFENILGKKALRDIENDTQLSYEDFA

SEQ ID NO: 30 - DNA, 876 bp, Escherichia coli
atgaccacactggcgattgatatcggcggtactaaacttgccgccgcgctgattggcgctgacgggcagatccgcgatcgtcgtgaacttcctacgccagccagccagacaccagaagccttgcgtgatgccttatccgcattagtctctccgttgcaagctcatgcgcagcgggttgccatcgcttcgaccgggataatccgtgacggcagcttgctggcgcttaatccgcataatcttggtggattgctacactttccgttagtcaaaacgctggaacaacttaccaatttgccgaccattgccattaacgacgcgcaggccgcagcatgggcggagtttcaggcgctggatggcgatataaccgatatggtctttatcaccgtttccaccggcgttggcggcggtgtagtgagcggctgcaaactgcttaccggccctggcggtctggcggggcatatcgggcatacgcttgccgatccacacggcccagtctgcggctgtggacgcacaggttgcgtggaagcgattgcttctggtcgcggcattgcagcggcagcgcagggggagttggctggcgcggatgcgaaaactattttcacgcgcgccgggcagggtgacgagcaggcgcagcagctgattcaccgctccgcacgtacgcttgcaaggctgatcgctgatattaaagccacaactgattgccagtgcgtggtggtcggtggcagcgttggtctggcagaagggtatctggcgctggtggaaacgtatctggcgcaggagccagcggcatttcatgttgatttactggcggcgcattaccgccatgatgcaggtttacttggggctgcgctgttggcccagggagaaaaattatga

SEQ ID NO: 31 - protein, 291 aa, Escherichia coli
MTTLAIDIGGTKLAAALIGADGQIRDRRELPTPASQTPEALRDALSALVSPLQAHAQRVAIASTGIIRDGSLLALNPHNLGGLLHFPLVKTLEQLTNLPTIAINDAQAAAWAEFQALDGDITDMVFITVSTGVGGGVVSGCKLLTGPGGLAGHIGHTLADPHGPVCGCGRTGCVEAIASGRGIAAAAQGELAGADAKTIFTRAGQGDEQAQQLIHRSARTLARLIADIKATTDCQCVVVGGSVGLAEGYLALVETYLAQEPAAFHVDLLAAHYRHDAGLLGAALLAQGEKL

SEQ ID NO: 32 - DNA, 690 bp, Escherichia coli
atgtcgttacttgcacaactggatcaaaaaatcgctgctaacggtggcctgattgtctcctgccagccggttccggacagcccgctcgataaacccgaaatcgtcgccgccatggcattagcggcagaacaggcgggcgcggttgccattcgcattgaaggtgtggcaaatctgcaagccacgcgtgcggtggtgagcgtgccgattattggaattgtgaaacgcgatctggaggattctccggtacgcatcacggcctatattgaagatgttgatgcgctggcgcaggcgggcgcggacattatcgccattgacggcaccgaccgcccgcgtccggtgcctgttgaaacgctgctggcacgtattcaccatcacggtttactggcgatgaccgactgctcaacgccggaagacggcctggcatgccaaaagctgggagccgaaattattggcactacgctttctggctataccacgcctgaaacgccagaagagccggatctggcgctggtgaaaacgttgagcgacgccggatgtcgggtgattgccgaagggcgttacaacacgcctgctcaggcggcggatgcgatgcgccacggcgcgtgggcggtgacggtcggttctgcaatcacgcgtcttgagcacatttgtcagtggtacaacacagcgatgaaaaaggcggtgctatga

SEQ ID NO: 33 - protein, 229 aa, Escherichia coli
MSLLAQLDQKIAANGGLIVSCQPVPDSPLDKPEIVAAMALAAEQAGAVAIRIEGVANLQATRAVVSVPIIGIVKRDLEDSPVRITAYIEDVDALAQAGADIIAIDGTDRPRPVPVETLLARIHHHGLLAMTDCSTPEDGLACQKLGAEIIGTTLSGYTTPETPEEPDLALVKTLSDAGCRVIAEGRYNTPAQAADAMRHGAWAVTVGSAITRLEHICQWYNTAMKKAVL

SEQ ID NO: 34 - DNA, 894 bp, Escherichia coli
atggcaacgaatttacgtggcgtaatggctgcactcctgactccttttgaccaacaacaagcactggataaagcgagtctgcgtcgcctggttcagttcaatattcagcagggcatcgacggtttatacgtgggtggttcgaccggcgaggcctttgtacaaagcctttccgagcgtgaacaggtactggaaatcgtcgccgaagaggcgaaaggtaagattaaactcatcgcccacgtcggttgcgtcagcaccgccgaaagccaacaacttgcggcatcggctaaacgttatggcttcgatgccgtctccgccgtcacgccgttctactatcctttcagctttgaagaacactgcgatcactatcgggcaattattgattcggcggatggtttgccgatggtggtgtacaacattccagccctgagtggggtaaaactgaccctggatcagatcaacacacttgttacattgcctggcgtaggtgcgctgaaacagacctctggcgatctctatcagatggagcagatccgtcgtgaacatcctgatcttgtgctctataacggttacgacgaaatcttcgcctctggtctgctggcgggcgctgatggtggtatcggcagtacctacaacatcatgggctggcgctatcaggggatcgttaaggcgctgaaagaaggcgatatccagaccgcgcagaaactgcaaactgaatgcaataaagtcattgatttactgatcaaaacgggcgtattccgcggcctgaaaactgtcctccattatatggatgtcgtttctgtgccgctgtgccgcaaaccgtttggaccggtagatgaaaaatatctgccagaactgaaggcgctggcccagcagttgatgcaagagcgcgggtga

SEQ ID NO: 35 - protein, 297 aa, Escherichia coli
MATNLRGVMAALLTPFDQQQALDKASLRRLVQFNIQQGIDGLYVGGSTGEAFVQSLSEREQVLEIVAEEAKGKIKLIAHVGCVSTAESQQLAASAKRYGFDAVSAVTPFYYPFSFEEHCDHYRAIIDSADGLPMVVYNIPALSGVKLTLDQINTLVTLPGVGALKQTSGDLYQMEQIRREHPDLVLYNGYDEIFASGLLAGADGGIGSTYNIMGWRYQGIVKALKEGDIQTAQKLQTECNKVIDLLIKTGVFRGLKTVLHYMDVVSVPLCRKPFGPVDEKYLPELKALAQQLMQERG

SEQ ID NO: 36 - DNA, 1491 bp, Escherichia coli
atgagtactacaacccagaatatcccgtggtatcgccatctcaaccgtgcacaatggcgcgcattttccgctgcctggttgggatatctgcttgacggttttgatttcgttttaatcgccctggtactcaccgaagtacaaggtgaattcgggctgacgacggtgcaggcggcaagtctgatctctgcagcctttatctctcgctggttcggcggcctgatgctcggcgctatgggtgaccgctacgggcgtcgtctggcaatggtcaccagcatcgttctcttctcggccgggacgctggcctgcggctttgcgccaggctacatcaccatgtttatcgctcgtctggtcatcggcatggggatggcgggtgaatacggttccagcgccacctatgtcattgaaagctggccaaaacatctgcgtaacaaagccagtggttttttgatttcaggcttctctgtgggggccgtcgttgccgctcaggtctatagcctggtggttccggtctggggctggcgtgcgctgttctttatcggcattttgccaatcatctttgctctctggctgcgtaaaaacatcccggaagcggaagactggaaagagaaacacgcaggtaaagcaccagtacgcacaatggtggatattctctaccgtggtgaacatcgcattgccaatatcgtaatgacactggcggcggctactgcgctgtggttctgcttcgccggtaacctgcaaaatgccgcgatcgtcgctgttcttgggctgttatgcgccgcaatctttatcagctttatggtgcagagtgcaggcaaacgctggccaacgggcgtaatgctgatggtggtcgtgttgtttgctttcctctactcatggccgattcaggcgctgctgccaacgtatctgaaaaccgatctggcttataacccgcatactgtagccaatgtgctgttctttagtggctttggcgcggcggtgggatgctgcgtaggtggcttcctcggtgactggctgggaacccgcaaagcgtacgtttgtagcctgctggcctcgcagctgctgattattccggtatttgcgattggcggcgcaaacgtctgggtgctcggtctgttactgttcttccagcaaatgcttggacaagggatcgccgggatcttaccaaaactgattggcggttatttcgataccgaccagcgtgcagcgggcctgggctttacctacaacgttggcgcattgggcggtgcactggccccaatcatcggcgcgttgatcgctcaacgtctggatctgggtactgcgctggcatcgctctcgttcagtctgacgttcgtggtgatcctgctgattgggctggatatgccttctcgcgttcagcgttggttgcgcccggaagcgttgcgtactcatgacgctatcgacggtaaaccattcagcggtgccgtgccgtttggcagcgccaaaaacgatttagtcaaaaccaaaagttaa

SEQ ID NO: 37 - protein, 496 aa, Escherichia coli
MSTTTQNIPWYRHLNRAQWRAFSAAWLGYLLDGFDFVLIALVLTEVQGEFGLTTVQAASLISAAFISRWFGGLMLGAMGDRYGRRLAMVTSIVLFSAGTLACGFAPGYITMFIARLVIGMGMAGEYGSSATYVIESWPKHLRNKASGFLISGFSVGAVVAAQVYSLVVPVWGWRALFFIGILPIIFALWLRKNIPEAEDWKEKHAGKAPVRTMVDILYRGEHRIANIVMTLAAATALWFCFAGNLQNAAIVAVLGLLCAAIFISFMVQSAGKRWPTGVMLMVVVLFAFLYSWPIQALLPTYLKTDLAYNPHTVANVLFFSGFGAAVGCCVGGFLGDWLGTRKAYVCSLLASQLLIIPVFAIGGANVWVLGLLLFFQQMLGQGIAGILPKLIGGYFDTDQRAAGLGFTYNVGALGGALAPIIGALIAQRLDLGTALASLSFSLTFVVILLIGLDMPSRVQRWLRPEALRTHDAIDGKPFSGAVPFGSAKNDLVKTKS

SEQ ID NO: 38 - DNA, 1149 bp, Escherichia coli
atgtatgcattaacccagggccggatctttaccggccacgaatttcttgatgaccacgcggttgttatcgctgatggcctgattaaaagcgtctgtccggtagcggaactgccgccagagatcgaacaacgttcactgaacggggccattctctcccccggttttatcgatgtgcagttaaacggctgcggcggcgtacagtttaacgacaccgctgaagcggtcagcgtggaaacgctggaaatcatgcagaaagccaatgagaaatcaggctgtactaactatctgccgacgcttatcaccaccagcgatgagctgatgaaacagggcgtgcgcgttatgcgcgagtacctggcaaaacatccgaatcaggcgttaggtctgcatctggaaggtccgtggctgaatctggtaaaaaaaggcacccataatccgaattttgtgcgtaagcctgatgccgcgctggtcgatttcctgtgtgaaaacgccgacgtcattaccaaagtgaccctggcaccggaaatggttcctgcggaagtcatcagcaaactggcaaatgccgggattgtggtttctgccggtcactccaacgcgacgttgaaagaagcaaaagccggtttccgcgcggggattacctttgccacccatctgtacaacgcgatgccgtatattaccggtcgtgaacctggcctggcgggcgcgatcctcgacgaagctgacatttattgcggtattattgctgatggcctgcatgttgattacgccaacattcgcaacgctaaacgtctgaaaggcgacaaactgtgtctggttactgacgccaccgcgccagcaggtgccaacattgaacagttcatttttgcgggtaaaacaatatactaccgtaacggactttgtgtggatgagaacggtacgttaagcggttcatccttaaccatgattgaaggcgtgcgtaatctggtcgaacattgcggtatcgcactggatgaagtgctacgtatggcgacgctctatccggcgcgtgcgattggcgttgagaaacgtctcggcacactcgccgcaggtaaagtagccaacctgactgcattcacacctgattttaaaatcaccaagaccatcgttaacggtaacgaggtcgtaactcaataa

SEQ ID NO: 39 - protein, 382 aa, Escherichia coli
MYALTQGRIFTGHEFLDDHAVVIADGLIKSVCPVAELPPEIEQRSLNGAILSPGFIDVQLNGCGGVQFNDTAEAVSVETLEIMQKANEKSGCTNYLPTLITTSDELMKQGVRVMREYLAKHPNQALGLHLEGPWLNLVKKGTHNPNFVRKPDAALVDFLCENADVITKVTLAPEMVPAEVISKLANAGIVVSAGHSNATLKEAKAGFRAGITFATHLYNAMPYITGREPGLAGAILDEADIYCGIIADGLHVDYANIRNAKRLKGDKLCLVTDATAPAGANIEQFIFAGKTIYYRNGLCVDENGTLSGSSLTMIEGVRNLVEHCGIALDEVLRMATLYPARAIGVEKRLGTLAAGKVANLTAFTPDFKITKTIVNGNEVVTQ

SEQ ID NO: 40 - DNA, 801 bp, Escherichia coli
atgagactgatccccctgactaccgctgaacaggtcggcaaatgggctgctcgccatatcgtcaatcgtatcaatgcgttcaaaccgactgccgatcgtccgtttgtactgggcctgccgactggcggcacgccgatgaccacctataaagcgttagtcgaaatgcataaagcaggccaggtcagctttaagcacgttgtcaccttcaacatggacgaatatgtcggtctgccgaaagagcatccggaaagctactacagctttatgcaccgtaatttcttcgatcacgttgatattccagcagaaaacatcaaccttctcaacggcaacgccccggatatcgacgccgagtgccgccagtatgaagaaaaaatccgttcttacggaaaaattcatctgtttatgggcggtgtaggtaacgacggtcatattgcatttaacgaaccggcgtcttctctggcttctcgtactcgtatcaaaaccctgactcatgacactcgcgtcgcaaactctcgtttctttgataacgatgttaatcaggtgccaaaatatgccctgactgtcggtgttggtacactgctggatgccgaagaagtgatgattctggtgctgggtagccagaaagcactggcgctgcaggccgccgttgaaggttgcgtgaaccatatgtggaccatcagctgtctgcaactgcatccgaaagcgatcatggtgtgcgatgaaccttccaccatggagctgaaagttaagactttaagatatttcaatgaattagaagcagaaaatatcaaaggtctgtaa

SEQ ID NO: 41 - protein, 266 aa, Escherichia coli [sequence omitted]

SEQ ID NO: 42 - DNA, 1947 bp, Escherichia coli
atgaatattttaggttttttccagcgactcggtagggcgttacagctccctatcgcggtgctgccggtggcggcactgttgctgcgattcggtcagccagatttacttaacgttgcgtttattgcccaggcgggcggtgcgatttttgataacctcgcattaatcttcgccatcggtgtggcatccagctggtcgaaagacagcgctggtgcggcggcgctggcgggtgcggtaggttactttgtgttaaccaaagcgatggtgaccatcaacccagaaattaacatgggtgtactggcgggtatcattaccggtctggttggtggcgcagcctataaccgttggtccgatattaaactgccggacttcctgagcttcttcggcggcaaacgctttgtgccgattgccaccggattcttctgcctggtgctggcggccatttttggttacgtctggccgccggtacagcacgctatccatgcaggcggcgagtggatcgtttctgcgggcgcgctgggttccggtatctttggtttcatcaaccgtctgctgatcccaaccggtctgcatcaggtactgaacaccatcgcctggttccagattggtgaattcaccaacgcggcgggtacggttttccacggtgacattaaccgcttctatgccggtgacggcaccgcggggatgttcatgtccggcttcttcccgatcatgatgttcggtctgccgggtgcggcgctggcgatgtacttcgcagcaccgaaagagcgtcgtccgatggttggcggtatgctgctttctgttgctgttactgcgttcctgaccggtgtgactgagccgctggaattcctgttcatgttccttgctccgctgctgtacctcctgcacgcactgctgaccggtatcagcctgtttgtggcaacgctgctgggtatccacgcgggcttctctttctctgcgggggctatcgactacgcgttgatgtataacctgccggccgccagccagaacgtctggatgctgctggtgatgggcgttatcttcttcgctatctacttcgtggtgttcagtttggttatccgcatgttcaacctgaaaacgccgggtcgtgaagataaagaagacgagatcgttactgaagaagccaacagcaacactgaagaaggtctgactcaactggcaaccaactatattgctgcggttggcggcactgacaacctgaaagcgattgacgcctgtatcacccgtctgcgccttacagtggctgactctgcccgcgttaacgatacgatgtgtaaacgtctgggtgcttctggggtagtgaaactgaacaaacagactattcaggtgattgttggcgcgaaagcagaatccatcggcgatgcgatgaagaaagtcgttgcccgtggtccggtagccgctgcgtcagctgaagcaactccggcaactgccgcgcctgtagcaaaaccgcaggctgtaccaaacgcggtatctatcgcggagctggtatcgccgattaccggtgatgtcgtggcactggatcaggttcctgacgaagcattcgccagcaaagcggtgggtgacggtgtggcggtgaaaccgacagataaaatcgtcgtatcaccagccgcagggacaatcgtgaaaatcttcaacaccaaccacgcgttctgcctggaaaccgaaaaaggcgcggagatcgtcgtccatatgggtatcgacaccgtagcgctggaaggtaaaggctttaaacgtctggtggaagagggtgcgcaggtaagcgcagggcaaccgattctggaaatggatctggattacctgaacgctaacgcccgctcgatgattagcccggtggtttgcagcaatatcgacgatttcagtggcttgatcattaaagctcagggccatattgtggcgggtcaaacaccgctgtatgaaatcaaaaagtaa

SEQ ID NO: 43 - protein, 648 aa, Escherichia coli
MNILGFFQRLGRALQLPIAVLPVAALLLRFGQPDLLNVAFIAQAGGAIFDNLALIFAIGVASSWSKDSAGAAALAGAVGYFVLTKAMVTINPEINMGVLAGIITGLVGGAAYNRWSDIKLPDFLSFFGGKRFVPIATGFFCLVLAAIFGYVWPPVQHAIHAGGEWIVSAGALGSGIFGFINRLLIPTGLHQVLNTIAWFQIGEFTNAAGTVFHGDINRFYAGDGTAGMFMSGFFPIMMFGLPGAALAMYFAAPKERRPMVGGMLLSVAVTAFLTGVTEPLEFLFMFLAPLLYLLHALLTGISLFVATLLGIHAGFSFSAGAIDYALMYNLPAASQNVWMLLVMGVIFFAIYFVVFSLVIRMFNLKTPGREDKEDEIVTEEANSNTEEGLTQLATNYIAAVGGTDNLKAIDACITRLRLTVADSARVNDTMCKRLGASGVVKLNKQTIQVIVGAKAESIGDAMKKVVARGPVAAASAEATPATAAPVAKPQAVPNAVSIAELVSPITGDVVALDQVPDEAFASKAVGDGVAVKPTDKIVVSPAAGTIVKIFNTNHAFCLETEKGAEIVVHMGIDTVALEGKGFKRLVEEGAQVSAGQPILEMDLDYLNANARSMISPVVCSNIDDFSGLIIKAQGHIVAGQTPLYEIKK

SEQ ID NO: 44 - DNA, 972 bp, Escherichia coli
atgaccattgctattgttataggcacacatggttgggctgcagagcagttgcttaaaacggcagaaatgctgttaggcgagcaggaaaacgtcggctggatcgatttcgttccaggtgaaaatgccgaaacgctgattgaaaagtacaacgctcagttggcaaaactcgacaccactaaaggcgtgctgtttctcgttgatacatggggaggcagcccgttcaatgctgccagccgcattgtcgtcgacaaagagcattatgaagtcattgcaggcgttaacattccaatgctcgtggaaacgttaatggcccgtgatgatgacccaagctttgatgaactggtggcactggcagtagaaacaggccgtgaaggcgtgaaagcactgaaagccaaaccggttgaaaaagccgcgccagcacccgctgccgcagcaccaaaagcggctccaactccggcaaaaccaatggggccaaacgactacatggttattggccttgcgcgtatcgacgaccgtctgattcacggtcaggtcgccacccgctggaccaaagaaaccaatgtctcccgtattattgttgttagtgatgaagtggctgcggataccgttcgtaagacactgctcacccaggttgcacctccgggcgtaacagcacacgtagttgatgttgccaaaatgattcgcgtctacaacaacccgaaatatgctggcgaacgcgtaatgctgttatttaccaacccaacagatgtagagcgtctcgttgaaggcggcgtgaaaatcacctctgttaacgtcggtggtatggcattccgtcagggtaaaacccaggtgaataacgcggtttcggttgatgaaaaagatatcgaggcgttcaagaaactgaatgcgcgcggtattgagctggaagtccgtaaggtttccaccgatccgaaactgaaaatgatggatctgatcagcaaaatcgataagtaa

SEQ ID NO: 45 - protein, 323 aa, Escherichia coli
MTIAIVIGTHGWAAEQLLKTAEMLLGEQENVGWIDFVPGENAETLIEKYNAQLAKLDTTKGVLFLVDTWGGSPFNAASRIVVDKEHYEVIAGVNIPMLVETLMARDDDPSFDELVALAVETGREGVKALKAKPVEKAAPAPAAAAPKAAPTPAKPMGPNDYMVIGLARIDDRLIHGQVATRWTKETNVSRIIVVSDEVAADTVRKTLLTQVAPPGVTAHVVDVAKMIRVYNNPKYAGERVMLLFTNPTDVERLVEGGVKITSVNVGGMAFRQGKTQVNNAVSVDEKDIEAFKKLNARGIELEVRKVSTDPKLKMMDLISKIDK

SEQ ID NO: 46 - DNA, 801 bp, Escherichia coli
atggagattaccactcttcaaattgtgctggtatttatcgtagcctgtatcgcaggtatgggatcaatcctcgatgaatttcagtttcaccgtccgctaatcgcgtgtaccctggtgggtatcgttcttggggatatgaaaaccggtattattatcggtggtacgctggaaatgatcgcgctgggctggatgaacatcggtgctgcagttgcgcctgacgccgctctggcttctatcatttctaccattctggttatcgcaggtcatcagagcattggtgcaggtatcgcactggcaatccctctggccgctgcgggccaggtactgaccatcatcgttcgtactattaccgttgctttccagcacgctgcggataaggctgctgataacggcaacctgacagcgatttcctggatccacgtttcttctctgttcctgcaagcaatgcgtgtggctattccggccgtcatcgttgcgctgtctgttggtaccagcgaagtacagaacatgctgaatgcgattccggaagtggtgaccaatggtctgaatatcgccggtggcatgatcgtggtggttggttatgcgatggttatcaacatgatgcgtgctggctacctgatgccgttcttctacctcggcttcgtaaccgcagcattcaccaactttaacctggttgctctgggtgtgattggtactgttatggcagtgctctacatccaacttagcccgaaatacaaccgcgtagccggtgcgcctgctcaggcagctggtaacaacgatctcgataacgaactggactaa

SEQ ID NO: 47 - protein, 266 aa, Escherichia coli
MEITTLQIVLVFIVACIAGMGSILDEFQFHRPLIACTLVGIVLGDMKTGIIIGGTLEMIALGWMNIGAAVAPDAALASIISTILVIAGHQSIGAGIALAIPLAAAGQVLTIIVRTITVAFQHAADKAADNGNLTAISWIHVSSLFLQAMRVAIPAVIVALSVGTSEVQNMLNAIPEVVTNGLNIAGGMIVVVGYAMVINMMRAGYLMPFFYLGFVTAAFTNFNLVALGVIGTVMAVLYIQLSPKYNRVAGAPAQAAGNNDLDNELD

SEQ ID NO: 48 - DNA, 852 bp, Escherichia coli
atggttgatacaactcaaactaccaccgagaaaaaactcactcaaagtgatattcgtggcgtcttcctgcgttctaacctcttccagggttcatggaacttcgaacgtatgcaggcactgggtttctgcttctctatggtaccggcaattcgtcgcctctaccctgagaacaacgaagctcgtaaacaagctattcgccgtcacctggagttctttaacacccagccgttcgtggctgcgccgattctcggcgtaaccctggcgctggaagaacagcgtgctaatggcgcagagatcgacgacggtgctatcaacggtatcaaagtcggtttgatggggccactggctggtgtaggcgacccgatcttctggggaaccgtacgtccggtatttgcagcactgggtgccggtatcgcgatgagcggcagcctgttaggtccgctgctgttcttcatcctgtttaacctggtgcgtctggcaacccgttactacggcgtagcgtatggttactccaaaggtatcgatatcgttaaagatatgggtggtggcttcctgcaaaaactgacggaaggggcgtctatcctcggcctgtttgtcatgggggcattggttaacaagtggacacatgtcaacatcccgctggttgtctctcgcattactgaccagacgggcaaagaacacgttactactgtccagactattctggaccagttaatgccaggcctggtaccactgctgctgacctttgcttgtatgtggctactgcgcaaaaaagttaacccgctgtggatcatcgttggcttcttcgtcatcggtatcgctggttacgcttgcggcctgctgggactgtaa

SEQ ID NO: 49 - protein, 283 aa, Escherichia coli
MVDTTQTTTEKKLTQSDIRGVFLRSNLFQGSWNFERMQALGFCFSMVPAIRRLYPENNEARKQAIRRHLEFFNTQPFVAAPILGVTLALEEQRANGAEIDDGAINGIKVGLMGPLAGVGDPIFWGTVRPVFAALGAGIAMSGSLLGPLLFFILFNLVRLATRYYGVAYGYSKGIDIVKDMGGGFLQKLTEGASILGLFVMGALVNKWTHVNIPLVVSRITDQTGKEHVTTVQTILDQLMPGLVPLLLTFACMWLLRKKVNPLWIIVGFFVIGIAGYACGLLGL

SEQ ID NO: 50 - DNA, 1434 bp, Escherichia coli
atgtttaagaatgcatttgctaacctgcaaaaggtcggtaaatcgctgatgctgccggtatccgtactgcctatcgcaggtattctgctgggcgtcggttccgcgaatttcagctggctgcccgccgttgtatcgcatgttatggcagaagcaggcggttccgtctttgcaaacatgccactgatttttgcgatcggtgtcgccctcggctttaccaataacgatggcgtatccgcgctggccgcagttgttgcctatggcatcatggttaaaaccatggccgtggttgcgccactggtactgcatttacctgctgaagaaatcgcctctaaacacctggcggatactggcgtactcggagggattatctccggtgcgatcgcagcgtacatgtttaaccgtttctaccgtattaagctgcctgagtatcttggcttctttgccggtaaacgctttgtgccgatcatttctggcctggctgccatctttactggcgttgtgctgtccttcatttggccgccgattggttctgcaatccagaccttctctcagtgggctgcttaccagaacccggtagttgcgtttggcatttacggtttcatcgaacgttgcctggtaccgtttggtctgcaccacatctggaacgtacctttccagatgcagattggtgaatacaccaacgcagcaggtcaggttttccacggcgacattccgcgttatatggcgggtgacccgactgcgggtaaactgtctggtggcttcctgttcaaaatgtacggtctgccagctgccgcaattgctatctggcactctgctaaaccagaaaaccgcgcgaaagtgggcggtattatgatctccgcggcgctgacctcgttcctgaccggtatcaccgagccgatcgagttctccttcatgttcgttgcgccgatcctgtacatcatccacgcgattctggcaggcctggcattcccaatctgtattcttctggggatgcgtgacggtacgtcgttctcgcacggtctgatcgacttcatcgttctgtctggtaacagcagcaaactgtggctgttcccgatcgtcggtatcggttatgcgattgtttactacaccatcttccgcgtgctgattaaagcactggatctgaaaacgccgggtcgtgaagacgcgactgaagatgcaaaagcgacaggtaccagcgaaatggcaccggctctggttgctgcatttggtggtaaagaaaacattactaacctcgacgcatgtattacccgtctgcgcgtcagcgttgctgatgtgtctaaagtggatcaggccggcctgaagaaactgggcgcagcgggcgtagtggttgctggttctggtgttcaggcgattttcggtactaaatccgataacctgaaaaccgagatggatgagtacatccgtaaccactaa

SEQ ID NO: 51 - protein, 477 aa, Escherichia coli
MFKNAFANLQKVGKSLMLPVSVLPIAGILLGVGSANFSWLPAVVSHVMAEAGGSVFANMPLIFAIGVALGFTNNDGVSALAAVVAYGIMVKTMAVVAPLVLHLPAEEIASKHLADTGVLGGIISGAIAAYMFNRFYRIKLPEYLGFFAGKRFVPIISGLAAIFTGVVLSFIWPPIGSAIQTFSQWAAYQNPVVAFGIYGFIERCLVPFGLHHIWNVPFQMQIGEYTNAAGQVFHGDIPRYMAGDPTAGKLSGGFLFKMYGLPAAAIAIWHSAKPENRAKVGGIMISAALTSFLTGITEPIEFSFMFVAPILYIIHAILAGLAFPICILLGMRDGTSFSHGLIDFIVLSGNSSKLWLFPIVGIGYAIVYYTIFRVLIKALDLKTPGREDATEDAKATGTSEMAPALVAAFGGKENITNLDACITRLRVSVADVSKVDQAGLKKLGAAGVVVAGSGVQAIFGTKSDNLKTEMDEYIRNH

SEQ ID NO: 52 - DNA, 510 bp, Escherichia coli
atgggtttgttcgataaactgaaatctctggtttccgacgacaagaaggataccggaactattgagatcattgctccgctctctggcgagatcgtcaatatcgaagacgtgccggatgtcgtttttgcggaaaaaatcgttggtgatggtattgctatcaaaccaacgggtaacaaaatggtcgcgccagtagacggcaccattggtaaaatctttgaaaccaaccacgcattctctatcgaatctgatagcggcgttgaactgttcgtccacttcggtatcgacaccgttgaactgaaaggcgaaggcttcaagcgtattgctgaagaaggtcagcgcgtgaaagttggcgatactgtcattgaatttgatctgccgctgctggaagagaaagccaagtctaccctgactccggttgttatctccaacatggacgaaatcaaagaactgatcaaactgtccggtagcgtaaccgtgggtgaaaccccggttatccgcatcaagaagtaa

SEQ ID NO: 53 - protein, 169 aa, Escherichia coli [sequence omitted]

SEQ ID NO: 54 - DNA, 1248 bp, Escherichia coli
atggcactgaatattccattcagaaatgcgtactatcgttttgcatccagttactcatttctcttttttatttcctggtcgctgtggtggtcgttatacgctatttggctgaaaggacatctaggattaacagggacggaattaggtacactttattcggtcaaccagtttaccagcattctatttatgatgttctacggcatcgttcaggataaactcggtctgaagaaaccgctcatctggtgtatgagtttcattctggtcttgaccggaccgtttatgatttacgtttatgaaccgttactgcaaagcaatttttctgtaggtctaattctgggggcgctcttttttggcctggggtatctggcgggatgcggtttgcttgacagcttcaccgaaaaaatggcgcgaaattttcatttcgaatatggaacagcgcgcgcctggggatcttttggctatgctattggcgcgttctttgccggtatattttttagtatcagtccccatatcaacttctggttggtctcgctatttggcgctgtatttatgatgatcaacatgcgttttaaagataaggatcaccagtgcatagcggcggatgcgggaggggtaaaaaaagaggattttatcgcagttttcaaggatcgaaacttctgggttttcgtcatatttattgtggggacgtggtctttctataacatttttgatcaacaactctttcctgtcttttatgcaggtttattcgaatcacacgatgtaggaacgcgcctgtatggttatctcaactcattccaggtggtactcgaagcgctgtgcatggcgattattcctttctttgtgaatcgggtagggccaaaaaatgcattacttatcggtgttgtgattatggcgttgcgtatcctttcctgcgcgttgttcgttaacccctggattatttcattagtgaagctgttacatgccattgaggttccactttgtgtcatatccgtcttcaaatacagcgtggcaaactttgataagcgcctgtcgtcgacgatctttctgattggttttcaaattgccagttcgcttgggattgtgctgctttcaacgccgactgggatactctttgaccacgcaggctaccagacagttttcttcgcaatttcgggtattgtctgcctgatgttgctatttggcattttcttcctgagtaaaaaacgcgagcaaatagttatggaaacgcctgtaccttcagcaatatag

SEQ ID NO: 55 - protein, 415 aa, Escherichia coli
MALNIPFRNAYYRFASSYSFLFFISWSLWWSLYAIWLKGHLGLTGTELGTLYSVNQFTSILFMMFYGIVQDKLGLKKPLIWCMSFILVLTGPFMIYVYEPLLQSNFSVGLILGALFFGLGYLAGCGLLDSFTEKMARNFHFEYGTARAWGSFGYAIGAFFAGIFFSISPHINFWLVSLFGAVFMMINMRFKDKDHQCIAADAGGVKKEDFIAVFKDRNFWVFVIFIVGTWSFYNIFDQQLFPVFYAGLFESHDVGTRLYGYLNSFQVVLEALCMAIIPFFVNRVGPKNALLIGVVIMALRILSCALFVNPWIISLVKLLHAIEVPLCVISVFKYSVANFDKRLSSTIFLIGFQIASSLGIVLLSTPTGILFDHAGYQTVFFAISGIVCLMLLFGIFFLSKKREQIVMETPVPSAI

SEQ ID NO: 56 - DNA, 924 bp, Escherichia coli
atgtcagccaaagtatgggttttaggggatgcggtcgtagatctcttgccagaatcagacgggcggctactgccttgtcctggcggcgcgccagctaacgttgcggtgggaatcgccagattaggcggaacaagtgggtttataggtcgggtcggtgatgatccttttggtgcgttaatgcaaagaacgctgctaactgagggtgtcgatatcacgtatctgaagcaagatgaatggcaccggacatccacggtgcttgtcgatctgaacgatcaaggagaacgttcatttacgtttatggtccgccccagtgccgatctttttttagagacgacagacttgccctgctggcgacatggcgaatggttacatctctgttcaattgcgttgtctgccgagccttcgcgtaccagcgcatttactgcgatgacggcgatccggcatgccggaggttttgtcagcttcgatcccaatattcgtgaagatctatggcaagacgagcatttgctccgcttgtgtttgcggcaggcgctacaactggcggatgtcgtcaagctctcggaagaagaatggcgacttatcagtggaaaaacacagaacgatcgggatatatgcgccctggcaaaagagtatgagatcgccatgctgttggtgactaaaggtgcagaaggggtggtggtctgttatcgaggacaagtccaccattttgctggaatgtctgtgaattgtgtcgatagcactggggcgggagatgcgttcgttgccgggttactcacaggtctgtcctctacgggattatctacagatgagagagaaatgcgacgaattatcgatctcgctcaacgttgcggagcgcttgcagtaacagcgaaaggggcaatgacagcgctgccatgtcgacaagaactggaaagtgagaagtaa

SEQ ID NO: 57 - protein, 307 aa, Escherichia coli
MSAKVWVLGDAVVDLLPESDGRLLPCPGGAPANVAVGIARLGGTSGFIGRVGDDPFGALMQRTLLTEGVDITYLKQDEWHRTSTVLVDLNDQGERSFTFMVRPSADLFLETTDLPCWRHGEWLHLCSIALSAEPSRTSAFTAMTAIRHAGGFVSFDPNIREDLWQDEHLLRLCLRQALQLADVVKLSEEEWRLISGKTQNDRDICALAKEYEIAMLLVTKGAEGVVVCYRGQVHHFAGMSVNCVDSTGAGDAFVAGLLTGLSSTGLSTDEREMRRIIDLAQRCGALAVTAKGAMTALPCRQELESEK

SEQ ID NO: 58 - DNA, 1434 bp, Escherichia coli
atgacgcaatctcgattgcatgcggcgcaaaacgccctagcaaaacttcatgagcaccggggtaacactttctatccccattttcacctcgcgcctcctgccgggtggatgaacgatccaaacggcctgatctggtttaacgatcgttatcacgcgttttatcaacatcatccgatgagcgaacactgggggccaatgcactggggacatgccaccagcgacgatatgatccactggcagcatgagcctattgcgctagcgccaggagacgataatgacaaagacgggtgtttttcaggtagtgctgtcgatgacaatggtgtcctctcacttatctacaccggacacgtctggctcgatggtgcaggtaatgacgatgcaattcgcgaagtacaatgtctggctaccagtcgggatggtattcatttcgagaaacagggtgtgatcctcactccaccagaaggaatcatgcacttccgcgatcctaaagtgtggcgtgaagccgacacatggtggatggtagtcggggcgaaagatccaggcaacacggggcagatcctgctttatcgcggcagttcattgcgtgaatggaccttcgatcgcgtactggcccacgctgatgcgggtgaaagctatatgtgggaatgtccggactttttcagccttggcgatcagcattatctgatgttttccccgcagggaatgaatgccgagggatacagttaccgaaatcgctttcaaagtggcgtaatacccggaatgtggtcgccaggacgactttttgcacaatccgggcattttactgaacttgataacgggcatgacttttatgcaccacaaagctttttagcgaaggatggtcggcgtattgttatcggatggatggatatgtgggaatcgccaatgccctcaaaacgtgaaggctgggcaggctgcatgacgctggcgcgcgagctatcagagagcaatggcaaacttctacaacgcccggttcacgaagctgagtcgttacgccagcagcatcaatctgtctctccccgcacaatcagcaataaatatgttttgcaggaaaacgcgcaagcagttgagattcagttgcagtgggcgctgaagaacagtgatgccgaacattacggattacagctcggcactggaatgcggctgtatattgataaccaatctgagcgacttgttttgtggcggtattacccacacgagaatttagacggctaccgtagtattcccctcccgcagcgtgacacgctcgccctaaggatatttatcgatacatcatccgtggaagtatttattaacgacggggaagcggtgatgagtagtcgaatctatccgcagccagaagaacgggaactgtcgctttatgcctcccacggagtggctgtgctgcaacatggagcactctggctactgggttaa

SEQ ID NO: 59 - protein, 480 aa, Escherichia coli
MIKMTQSRLHAAQNALAKLHEHRGNTFYPHFHLAPPAGWMNDPNGLIWFNDRYHAFYQHHPMSEHWGPMHWGHATSDDMIHWQHEPIALAPGDDNDKDGCFSGSAVDDNGVLSLIYTGHVWLDGAGNDDAIREVQCLATSRDGIHFEKQGVILTPPEGIMHFRDPKVWREADTWWMVVGAKDPGNTGQILLYRGSSLREWTFDRVLAHADAGESYMWECPDFFSLGDQHYLMFSPQGMNAEGYSYRNRFQSGVIPGMWSPGRLFAQSGHFTELDNGHDFYAPQSFLAKDGRRIVIGWMDMWESPMPSKREGWAGCMTLARELSESNGKLLQRPVHEAESLRQQHQSVSPRTISNKYVLQENAQAVEIQLQWALKNSDAEHYGLQLGTGMRLYIDNQSERLVLWRYYPHENLDGYRSIPLPQRDTLALRIFIDTSSVEVFINDGEAVMSSRIYPQPEERELSLYASHGVAVLQHGALWLLG

SEQ ID NO: 60 - DNA, 954 bp, Escherichia coli
atgatgacagtctcccgggtgatgcataatgcagaatctgtgcgtcctgcaacgcgtgaccgcgtattgcaggcaatccagaccctgaattatgttcctgatctttccgcccgtaagatgcgcgctcaaggacgtaagccgtcgactctcgccgtgctggcgcaggacacggctaccactcctttctctgttgatattctgcttgccattgagcaaaccgccagcgagttcggctggaatagttttttaatcaatattttttctgaagatgacgctgcccgtgctgcacgtcagctgcttgcccaccgtccggatggcattatctatactacaatggggctgcgacatatcacgctgcctgagtctctgtatggtgaaaatattgtattggcgaactgtgtggcggatgacccagcgttacccagttatatccctgatgattacactgcacaatatgaatcaacacagcatttgctcgcggcgggctatcgtcaaccgttatgcttctggctaccggaaagtgcgttggcaacagggtatcgtcggcagggatttgagcaggcctggcgtgatgctggacgagatctggctgaggtgaaacaatttcacatggcaacaggtgatgatcactacaccgatctcgcaagtttactcaatgcccacttcaaatcgggcaaaccagattttgatgttctgatatgtggtaacgatcgcgcagcttttgtggcttatcaggttcttttggcgaagggggtacgtatcccgcaggatgtcgccgtaatgggctttgataatctggttggcgtcgggcatctgtttttaccgccgctgaccacaattcagcttccacatgacattatcgggcgggaagctgcattgcatattattgaaggtcgtgaagggggaagagtgacccggatcccttgcccgctgttgatccgttgttccacctga

SEQ ID NO: 61 - protein, 317 aa, Escherichia coli
MMTVSRVMHNAESVRPATRDRVLQAIQTLNYVPDLSARKMRAQGRKPSTLAVLAQDTATTPFSVDILLAIEQTASEFGWNSFLINIFSEDDAARAARQLLAHRPDGIIYTTMGLRHITLPESLYGENIVLANCVADDPALPSYIPDDYTAQYESTQHLLAAGYRQPLCFWLPESALATGYRRQGFEQAWRDAGRDLAEVKQFHMATGDDHYTDLASLLNAHFKSGKPDFDVLICGNDRAAFVAYQVLLAKGVRIPQDVAVMGFDNLVGVGHLFLPPLTTIQLPHDIIGREAALHIIEGREGGRVTRIPCPLLIRCST

SEQ ID NO: 62 - DNA, 1254 bp, Escherichia coli
atgtactatttaaaaaacacaaacttttggatgttcggtttattctttttcttttacttttttatcatgggagcctacttcccgtttttcccgatttggctacatgacatcaaccatatcagcaaaagtgatacgggtattatttttgccgctatttctctgttctcgctattattccaaccgctgtttggtctgctttctgacaaactcgggctgcgcaaatacctgctgtggattattaccggcatgttagtgatgtttgcgccgttctttatttttatcttcgggccactgttacaatacaacattttagtaggatcgattgttggtggtatttatctaggcttttgttttaacgccggtgcgccagcagtagaggcatttattgagaaagtcagccgtcgcagtaatttcgaatttggtcgcgcgcggatgtttggctgtgttggctgggcgctgtgtgcctcgattgtcggcatcatgttcaccatcaataatcagtttgttttctggctgggctctggctgtgcactcatcctcgccgttttactctttttcgccaaaacggatgcgccctcttctgccacggttgccaatgcggtaggtgccaaccattcggcatttagccttaagctggcactggaactgttcagacagccaaaactgtggtttttgtcactgtatgttattggcgtttcctgcacctacgatgtttttgaccaacagtttgctaatttctttacttcgttctttgctaccggtgaacagggtacgcgggtatttggctacgtaacgacaatgggcgaattacttaacgcctcgattatgttctttgcgccactgatcattaatcgcatcggtgggaaaaacgccctgctgctggctggcactattatgtctgtacgtattattggctcatcgttcgccacctcagcgctggaagtggttattctgaaaacgctgcatatgtttgaagtaccgttcctgctggtgggctgctttaaatatattaccagccagtttgaagtgcgtttttcagcgacgatttatctggtctgtttctgcttctttaagcaactggcgatgatttttatgtctgtactggcgggcaatatgtatgaaagcatcggtttccagggcgcttatctggtgctgggtctggtggcgctgggcttcaccttaatttccgtgttcacgcttagcggccccggcccgctttccctgctgcgtcgtcaggtgaatgaagtcgcttaa

SEQ ID NO: 63 - protein, 417 aa, Escherichia coli [sequence omitted]

SEQ ID NO: 64 - DNA, 3075 bp, Escherichia coli
atgaccatgattacggattcactggccgtcgttttacaacgtcgtgactgggaaaaccctggcgttacccaacttaatcgccttgcagcacatccccctttcgccagctggcgtaatagcgaagaggcccgcaccgatcgcccttcccaacagttgcgcagcctgaatggcgaatggcgctttgcctggtttccggcaccagaagcggtgccggaaagctggctggagtgcgatcttcctgaggccgatactgtcgtcgtcccctcaaactggcagatgcacggttacgatgcgcccatctacaccaacgtgacctatcccattacggtcaatccgccgtttgttcccacggagaatccgacgggttgttactcgctcacatttaatgttgatgaaagctggctacaggaaggccagacgcgaattatttttgatggcgttaactcggcgtttcatctgtggtgcaacgggcgctgggtcggttacggccaggacagtcgtttgccgtctgaatttgacctgagcgcatttttacgcgccggagaaaaccgcctcgcggtgatggtgctgcgctggagtgacggcagttatctggaagatcaggatatgtggcggatgagcggcattttccgtgacgtctcgttgctgcataaaccgactacacaaatcagcgatttccatgttgccactcgctttaatgatgatttcagccgcgctgtactggaggctgaagttcagatgtgcggcgagttgcgtgactacctacgggtaacagtttctttatggcagggtgaaacgcaggtcgccagcggcaccgcgcctttcggcggtgaaattatcgatgagcgtggtggttatgccgatcgcgtcacactacgtctgaacgtcgaaaacccgaaactgtggagcgccgaaatcccgaatctctatcgtgcggtggttgaactgcacaccgccgacggcacgctgattgaagcagaagcctgcgatgtcggtttccgcgaggtgcggattgaaaatggtctgctgctgctgaacggcaagccgttgctgattcgaggcgttaaccgtcacgagcatcatcctctgcatggtcaggtcatggatgagcagacgatggtgcaggatatcctgctgatgaagcagaacaactttaacgccgtgcgctgttcgcattatccgaaccatccgctgtggtacacgctgtgcgaccgctacggcctgtatgtggtggatgaagccaatattgaaacccacggcatggtgccaatgaatcgtctgaccgatgatccgcgctggctaccggcgatgagcgaacgcgtaacgcgaatggtgcagcgcgatcgtaatcacccgagtgtgatcatctggtcgctggggaatgaatcaggccacggcgctaatcacgacgcgctgtatcgctggatcaaatctgtcgatccttcccgcccggtgcagtatgaaggcggcggagccgacaccacggccaccgatattatttgcccgatgtacgcgcgcgtggatgaagaccagcccttcccggctgtgccgaaatggtccatcaaaaaatggctttcgctacctggagagacgcgcccgctgatcctttgcgaatacgcccacgcgatgggtaacagtcttggcggtttcgctaaatactggcaggcgtttcgtcagtatccccgtttacagggcggcttcgtctgggactgggtggatcagtcgctgattaaatatgatgaaaacggcaacccgtggtcggcttacggcggtgattttggcgatacgccgaacgatcgccagttctgtatgaacggtctggtctttgccgaccgcacgccgcatccagcgctgacggaagcaaaacaccagcagcagtttttccagttccgtttatccgggcaaaccatcgaagtgaccagcgaatacctgttccgtcatagcgataacgagctcctgcactggatggtggcgctggatggtaagccgctggcaagcggtgaagtgcctctggatgtcgctccacaaggtaaacagttgattgaactgcctgaactaccgcagccggagagcgccgggcaactctggctcacagtacgcgtagtgcaaccgaacgcgaccgcatggtcagaagccgggcacatcagcgcctggcagcagtggcgtctggcggaaaacctcagtgtgacgctccccgccgcgtcccacgccatcccgcatctgaccaccagcgaaatggatttttgcatcgagctgggtaataagcgttggcaatttaaccgccagtcaggctttctttcacagatgtggattggcgataaaaaacaactgctgacgccgctgcgcgatcagttcacccgtgcaccgctggataacgacattggcgtaagtgaagcgacccgcattgaccctaacgcctgggtcgaacgctggaaggcggcgggccattaccaggccgaagcagcgttgttgcagtgcacggcagatacacttgctgatgcggtgctgattacgaccgctcacgcgtggcagcatcaggggaaaaccttatttatcagccggaaaacctaccggattgatggtagtggtcaaatggcgattaccgttgatgttgaagtggcgagcgatacaccgcatccggcgcggattggcctgaactgccagctggcgcaggtagcagagcgggtaaactggctcggattagggccgcaagaaaactatcccgaccgccttactgccgcctgttttgaccgctgggatctgccattgtcagacatgtataccccgtacgtcttcccgagcgaaaacggtctgcgctgcgggacgcgcgaattgaattatggcccacaccagtggcgcggcgacttccagttcaacatcagccgctacagtcaacagcaactgatggaaaccagccatcgccatctgctgcacgcggaagaaggcacatggctgaatatcgacggtttccatatggggattggtggcgacgactcctggagcccgtcagtatcggcggaattccagctgagcgccggtcgctaccattaccagttggtctggtgtcaaaaataa

SEQ ID NO: 65 - protein, 1024 aa, Escherichia coli
MTMITDSLAVVLQRRDWENPGVTQLNRLAAHPPFASWRNSEEARTDRPSQQLRSLNGEWRFAWFPAPEAVPESWLECDLPEADTVVVPSNWQMHGYDAPIYTNVTYPITVNPPFVPTENPTGCYSLTFNVDESWLQEGQTRIIFDGVNSAFHLWCNGRWVGYGQDSRLPSEFDLSAFLRAGENRLAVMVLRWSDGSYLEDQDMWRMSGIFRDVSLLHKPTTQISDFHVATRFNDDFSRAVLEAEVQMCGELRDYLRVTVSLWQGETQVASGTAPFGGEIIDERGGYADRVTLRLNVENPKLWSAEIPNLYRAVVELHTADGTLIEAEACDVGFREVRIENGLLLLNGKPLLIRGVNRHEHHPLHGQVMDEQTMVQDILLMKQNNFNAVRCSHYPNHPLWYTLCDRYGLYVVDEANIETHGMVPMNRLTDDPRWLPAMSERVTRMVQRDRNHPSVIIWSLGNESGHGANHDALYRWIKSVDPSRPVQYEGGGADTTATDIICPMYARVDEDQPFPAVPKWSIKKWLSLPGETRPLILCEYAHAMGNSLGGFAKYWQAFRQYPRLQGGFVWDWVDQSLIKYDENGNPWSAYGGDFGDTPNDRQFCMNGLVFADRTPHPALTEAKHQQQFFQFRLSGQTIEVTSEYLFRHSDNELLHWMVALDGKPLASGEVPLDVAPQGKQLIELPELPQPESAGQLWLTVRVVQPNATAWSEAGHISAWQQWRLAENLSVTLPAASHAIPHLTTSEMDFCIELGNKRWQFNRQSGFLSQMWIGDKKQLLTPLRDQFTRAPLDNDIGVSEATRIDPNAWVERWKAAGHYQAEAALLQCTADTLADAVLITTAHAWQHQGKTLFISRKTYRIDGSGQMAITVDVEVASDTPHPARIGLNCQLAQVAERVNWLGLGPQENYPDRLTAACFDRWDLPLSDMYTPYVFPSENGLRCGTRELNYGPHQWRGDFQFNISRYSQQQLMETSHRHLLHAEEGTWLNIDGFHMGIGGDDSWSPSVSAEFQLSAGRYHYQLVWCQK

SEQ ID NO: 66 - DNA, 1119 bp, Staphylococcus epidermidis
atgactaaactccatatcttttacttttctttaatgtactttcttattggcatgatacacacttttgtcggttcatttaatcaattcttaaaaatagaacttaatatgaatcaatcagatgtatcaaatctaattagtattcagttcataacatttatgattggagtattttattctaccttcttagttaataaagacataaagaattttttaaaaataatacatttatttattctattaattactactacttttattatatttgaacattacttaataatatatctgattgtagctatattaggtttttgcgctggatttattgaatcatctatcgcatcatatatttttaatagtaagtttgagtccgctaaaacttttggatatatagaatcattttttgcagtagggtcatttttgctccctgtaattgtgaaagtgtttgaataccattcagatacaaaacacgctattatctttatacttataataaatataatcttatttttaattatctattcattagagtttgaagtaagtagcagcgatagaaataaaatacccatactgtcttttaataaaaagtcaatgctagttatgattatttttacatggtgtttcttttatattagtatagaaacaaatttttcaaatttactaccatatatcaacttagtttctgaaaaatatagctatattactgtaagtatattttgggttggaataattataggaaggtttttatatacgctaatattgacgttaattagattcaggctagaatcattactattaacatatacagtgacatctttttttctatatattattttaatatatttgaatactcaagatgaagtcaaattaataattttgtttttacttactctattcttagcacctatgttccctttaggtgttagtatcattaatcaacatagtagtaataagaacttactaactagtatttttattgctgtagctggatgtggtggtgcagttggtgcagtaattataaaatcagctttatacattcatattcccgtacatttatctattttattaatattaatgacttgcttatttttaagtactgtgattttaaaaataaagctttaa

SEQ ID NO: 67 - protein, 372 aa, Staphylococcus epidermidis
MTKLHIFYFSLMYFLIGMIHTFVGSFNQFLKIELNMNQSDVSNLISIQFITFMIGVFYSTFLVNKDIKNFLKIIHLFILLITTTFIIFEHYLIIYLIVAILGFCAGFIESSIASYIFNSKFESAKTFGYIESFFAVGSFLLPVIVKVFEYHSDTKHAIIFILIINIILFLIIYSLEFEVSSSDRNKIPILSFNKKSMLVMIIFTWCFFYISIETNFSNLLPYINLVSEKYSYITVSIFWVGIIIGRFLYTLILTLIRFRLESLLLTYTVTSFFLYIILIYLNTQDEVKLIILFLLTLFLAPMFPLGVSIINQHSSNKNLLTSIFIAVAGCGGAVGAVIIKSALYIHIPVHLSILLILMTCLFLSTVILKIKL

SEQ ID NO: 68 - DNA, 1350 bp, Lactobacillus brevis
atgcaagcaactgaaaccaagcacggctggacccaattagcggacggctacctcagcaaaacgccattatttcaatttattttagtttcattgatttttccactgtggggaactgcggcaagtttaaatgatattttgattacgcagttcaagacagtctttcaacttaacgatgccgcgacggcctttgttcaaagtgccttctatggtgggtatttcttaattgccattccggcatccctgattattaagaagaacagttataaatttgccatcatgaccgggttgatcttttatatcatcgggtgtgggctgtttttcccggcctcacatctcgcaacttacagtatgttcctggtggccatctttgccattgccattggtctgagcttcttggaaacatcatgtgatacgtatagttcaatgctgggaccgaagcaacacgccacgatgcgcttgaacttttcccagacattaattccgttaggcgacatcatgggaattgttttagggaagtacttaatttttggttctgtaggtaatttatctgaaaagatgagccatatgcacggcgcagcacgcattgcttacggcgaacagatgttacaattgacgttacggccttacaaatatatcttaatcgtgttactcgtgatgctgattatctttgccgtaacgcctatgccacgggctaaggcgacgaaggaaattggtggggaacaacaagaagaacgtcctagtcttggggaaactctgaagtatctatcacacaacaagcactatattaaaggggtagtaacccagttcttttatgcgggtctgcaaacaaccgtctggtcctttacgattcgtttggtattaaacttgaaccatcaaattaccgacagcggtgcatcaacctttatgatttatagttatgtggcgtggttcgttggtaagctggttgccaatacctttatgagtcgcttctcaattacgaaggtgctgacgtggtactccttattggggacattagcattagttgtgacctttacggttccgaatatgattgcggtctacgcagccatcttaacgagtttcttctttggtccagaatggccaacaatttatgcgcacacgttggatgccgttacggagaagaaatacactgaaacggctggggcaattatcgtgatggccctgatcggtggtgcagtcattccagccattcaaggcctggtttctgatgcgaccggttcaatgcagttctcattcgttgtaccaatgctctgctacgctttaattacagggtactttttcttcgaacatcgttttgagaaagctcaccctaacgaagttcaagaacattaa

SEQ ID NO: 69 - protein, 449 aa, Lactobacillus brevis
MQATETKHGWTQLADGYLSKTPLFQFILVSLIFPLWGTAASLNDILITQFKTVFQLNDAATAFVQSAFYGGYFLIAIPASLIIKKNSYKFAIMTGLIFYIIGCGLFFPASHLATYSMFLVAIFAIAIGLSFLETSCDTYSSMLGPKQHATMRLNFSQTLIPLGDIMGIVLGKYLIFGSVGNLSEKMSHMHGAARIAYGEQMLQLTLRPYKYILIVLLVMLIIFAVTPMPRAKATKEIGGEQQEERPSLGETLKYLSHNKHYIKGVVTQFFYAGLQTTVWSFTIRLVLNLNHQITDSGASTFMIYSYVAWFVGKLVANTFMSRFSITKVLTWYSLLGTLALVVTFTVPNMIAVYAAILTSFFFGPEWPTIYAHTLDAVTEKKYTETAGAIIVMALIGGAVIPAIQGLVSDATGSMQFSFVVPMLCYALITGYFFFEHRFEKAHPNEVQEH

SEQ ID NO: 70 - DNA, 2379 bp, Escherichia coli
atgtccaacaatggctcgtcaccgctggtgctttggtataaccaactcggcatgaatgatgtagacagggttgggggcaaaaatgcctccctgggtgaaatgattactaatctttccggaatgggtgtttccgttccgaatggtttcgccacaaccgccgacgcgtttaaccagtttctggaccaaagcggcgtaaaccagcgcatttatgaactgctggataaaacggatattgacgatgttactcagcttgcgaaagcgggcgcgcaaatccgccagtggattatcgacactcccttccagcctgagctggaaaacgccatccgcgaagcctatgcacagctttccgccgatgacgaaaacgcctcttttgcggtgcgctcctccgccaccgcagaagatatgccggacgcttcttttgccggtcagcaggaaaccttcctcaacgttcagggttttgacgccgttctcgtggcagtgaaacatgtatttgcttctctgtttaacgatcgcgccatctcttatcgtgtgcaccagggttacgatcaccgtggtgtggcgctctccgccggtgttcaacggatggtgcgctctgacctcgcatcatctggcgtgatgttctccattgataccgaatccggctttgaccaggtggtgtttatcacttccgcatggggccttggtgagatggtcgtgcagggtgcggttaacccggatgagttttacgtgcataaaccgacactggcggcgaatcgcccggctatcgtgcgccgcaccatggggtcgaaaaaaatccgcatggtttacgcgccgacccaggagcacggcaagcaggttaaaatcgaagacgtaccgcaggaacagcgtgacatcttctcgctgaccaacgaagaagtgcaggaactggcaaaacaggccgtacaaattgagaaacactacggtcgcccgatggatattgagtgggcgaaagatggccacaccggtaaactgttcattgtgcaggcgcgtccggaaaccgtgcgctcacgcggtcaggtcatggagcgttatacgctgcattcacagggtaagattatcgccgaaggccgtgctatcggtcatcgcatcggtgcgggtccggtgaaagtcatccatgacatcagcgaaatgaaccgcatcgaacctggcgacgtgctggttactgacatgaccgacccggactgggaaccgatcatgaagaaagcatctgccatcgtcaccaaccgtggcggtcgtacctgtcacgcggcgatcatcgctcgtgaactgggcattccggcggtagtgggctgtggagatgcaacagaacggatgaaagacggtgagaacgtcactgtttcttgtgccgaaggtgataccggttacgtctatgcggagttgctggaatttagcgtgaaaagctccagcgtagaaacgatgccggatctgccgttgaaagtgatgatgaacgtcggtaacccggaccgtgctttcgacttcgcctgcctaccgaacgaaggcgtgggccttgcgcgtctggaatttatcatcaaccgtatgattggcgtccacccacgcgcactgcttgagtttgacgatcaggaaccgcagttgcaaaacgaaatccgcgagatgatgaaaggttttgattctccgcgtgaattttacgttggtcgtctgactgaagggatcgcgacgctgggtgccgcgttttatccgaagcgcgtcattgtccgtctctctgattttaaatcgaacgaatatgccaacctggtcggtggtgagcgttacgagccagatgaagagaacccgatgctcggcttccgtggcgcgggccgctatgtttccgacagcttccgcgactgtttcgcgctggagtgtgaagcagtgaaacgtgtgcgcaacgacatgggactgaccaacgttgagatcatgatcccgttcgtgcgtaccgtagatcaggcgaaagcggtggttgaagaactggcgcgtcaggggctgaaacgtggcgagaacgggctgaaaatcatcatgatgtgtgaaatcccgtccaacgccttgctggccgagcagttcctcgaatatttcgacggcttctcaattggctcaaacgatatgacgcagctggcgctcggtctggaccgtgactccggcgtggtgtctgaattgttcgatgagcgcaacgatgcggtgaaagcactgctgtcgatggctatccgtgccgcgaagaaacagggcaaatatgtcgggatttgcggtcagggtccgtccgaccacgaagactttgccgcatggttgatggaagaggggatcgatagcctgtctctgaacccggacaccgtggtgcaaacctggttaagcctggctgaactgaagaaataa

SEQ ID NO: 71 - protein, 792 aa, Escherichia coli
MSNNGSSPLVLWYNQLGMNDVDRVGGKNASLGEMITNLSGMGVSVPNGFATTADAFNQFLDQSGVNQRIYELLDKTDIDDVTQLAKAGAQIRQWIIDTPFQPELENAIREAYAQLSADDENASFAVRSSATAEDMPDASFAGQQETFLNVQGFDAVLVAVKHVFASLFNDRAISYRVHQGYDHRGVALSAGVQRMVRSDLASSGVMFSIDTESGFDQVVFITSAWGLGEMVVQGAVNPDEFYVHKPTLAANRPAIVRRTMGSKKIRMVYAPTQEHGKQVKIEDVPQEQRDIFSLTNEEVQELAKQAVQIEKHYGRPMDIEWAKDGHTGKLFIVQARPETVRSRGQVMERYTLHSQGKIIAEGRAIGHRIGAGPVKVIHDISEMNRIEPGDVLVTDMTDPDWEPIMKKASAIVTNRGGRTCHAAIIARELGIPAVVGCGDATERMKDGENVTVSCAEGDTGYVYAELLEFSVKSSSVETMPDLPLKVMMNVGNPDRAFDFACLPNEGVGLARLEFIINRMIGVHPRALLEFDDQEPQLQNEIREMMKGFDSPREFYVGRLTEGIATLGAAFYPKRVIVRLSDFKSNEYANLVGGERYEPDEENPMLGFRGAGRYVSDSFRDCFALECEAVKRVRNDMGLTNVEIMIPFVRTVDQAKAVVEELARQGLKRGENGLKIIMMCEIPSNALLAEQFLEYFDGFSIGSNDMTQLALGLDRDSGVVSELFDERNDAVKALLSMAIRAAKKQGKYVGICGQGPSDHEDFAAWLMEEGIDSLSLNPDTVVQTWLSLAELKK

SEQ ID NO: 72 - DNA, 1623 bp, Escherichia coli
atgcgcgttaacaatggtttgaccccgcaagaactcgaggcttatggtatcagtgacgtacatgatatcgtttacaacccaagctacgacctgctgtatcaggaagagctcgatccgagcctgacaggttatgagcgcggggtgttaactaatctgggtgccgttgccgtcgataccgggatcttcaccggtcgttcaccaaaagataagtatatcgtccgtgacgataccactcgcgatactttctggtgggcagacaaaggcaaaggtaagaacgacaacaaacctctctctccggaaacctggcagcatctgaaaggcctggtgaccaggcagctttccggcaaacgtctgttcgttgtcgacgctttctgtggtgcgaacccggatactcgtctttccgtccgtttcatcaccgaagtggcctggcaggcgcattttgtcaaaaacatgtttattcgcccgagcgatgaagaactggcaggtttcaaaccagactttatcgttatgaacggcgcgaagtgcactaacccgcagtggaaagaacagggtctcaactccgaaaacttcgtggcgtttaacctgaccgagcgcatgcagctgattggcggcacctggtacggcggcgaaatgaagaaagggatgttctcgatgatgaactacctgctgccgctgaaaggtatcgcttctatgcactgctccgccaacgttggtgagaaaggcgatgttgcggtgttcttcggcctttccggcaccggtaaaaccaccctttccaccgacccgaaacgtcgcctgattggcgatgacgaacacggctgggacgatgacggcgtgtttaacttcgaaggcggctgctacgcaaaaactatcaagctgtcgaaagaagcggaacctgaaatctacaacgctatccgtcgtgatgcgttgctggaaaacgtcaccgtgcgtgaagatggcactatcgactttgatgatggttcaaaaaccgagaacacccgcgtttcttatccgatctatcacatcgataacattgttaagccggtttccaaagcgggccacgcgactaaggttatcttcctgactgctgatgctttcggcgtgttgccgccggtttctcgcctgactgccgatcaaacccagtatcacttcctctctggcttcaccgccaaactggccggtactgagcgtggcatcaccgaaccgacgccaaccttctccgcttgcttcggcgcggcattcctgtcgctgcacccgactcagtacgcagaagtgctggtgaaacgtatgcaggcggcgggcgcgcaggcttatctggttaacactggctggaacggcactggcaaacgtatctcgattaaagatacccgcgccattatcgacgccatcctcaacggttcgctggataatgcagaaaccttcactctgccgatgtttaacctggcgatcccaaccgaactgccgggcgtagacacgaagattctcgatccgcgtaacacctacgcttctccggaacagtggcaggaaaaagccgaaaccctggcgaaactgtttatcgacaacttcgataaatacaccgacacccctgcgggtgccgcgctggtagcggctggtccgaaactgtaa

SEQ ID NO: 73 - protein, 540 aa, Escherichia coli
MRVNNGLTPQELEAYGISDVHDIVYNPSYDLLYQEELDPSLTGYERGVLTNLGAVAVDTGIFTGRSPKDKYIVRDDTTRDTFWWADKGKGKNDNKPLSPETWQHLKGLVTRQLSGKRLFVVDAFCGANPDTRLSVRFITEVAWQAHFVKNMFIRPSDEELAGFKPDFIVMNGAKCTNPQWKEQGLNSENFVAFNLTERMQLIGGTWYGGEMKKGMFSMMNYLLPLKGIASMHCSANVGEKGDVAVFFGLSGTGKTTLSTDPKRRLIGDDEHGWDDDGVFNFEGGCYAKTIKLSKEAEPEIYNAIRRDALLENVTVREDGTIDFDDGSKTENTRVSYPIYHIDNIVKPVSKAGHATKVIFLTADAFGVLPPVSRLTADQTQYHFLSGFTAKLAGTERGITEPTPTFSACFGAAFLSLHPTQYAEVLVKRMQAAGAQAYLVNTGWNGTGKRISIKDTRAIIDAILNGSLDNAETFTLPMFNLAIPTELPGVDTKILDPRNTYASPEQWQEKAETLAKLFIDNFDKYTDTPAGAALVAAGPKL

SEQ ID NO: 74 - DNA, 1443 bp, Escherichia coli
atgtccagaaggcttcgcagaacaaaaatcgttaccacgttaggcccagcaacagatcgcgataataatcttgaaaaagttatcgcggcgggtgccaacgttgtacgtatgaacttttctcacggctcgcctgaagatcacaaaatgcgcgcggataaagttcgtgagattgccgcaaaactggggcgtcatgtggctattctgggtgacctccaggggcccaaaatccgtgtatccacctttaaagaaggcaaagttttcctcaatattggggataaattcctgctcgacgccaacctgggtaaaggtgaaggcgacaaagaaaaagtcggtatcgactacaaaggcctgcctgctgacgtcgtgcctggtgacatcctgctgctggacgatggtcgcgtccagttaaaagtactggaagttcagggcatgaaagtgttcaccgaagtcaccgtcggtggtcccctctccaacaataaaggtatcaacaaacttggcggcggtttgtcggctgaagcgctgaccgaaaaagacaaagcagacattaagactgcggcgttgattggcgtagattacctggctgtctccttcccacgctgtggcgaagatctgaactatgcccgtcgcctggcacgcgatgcaggatgtgatgcgaaaattgttgccaaggttgaacgtgcggaagccgtttgcagccaggatgcaatggatgacatcatcctcgcctctgacgtggtaatggttgcacgtggcgacctcggtgtggaaattggcgacccggaactggtcggcattcagaaagcgttgatccgtcgtgcgcgtcagctaaaccgagcggtaatcacggcgacccagatgatggagtcaatgattactaacccgatgccgacgcgtgcagaagtcatggacgtagcaaacgccgttctggatggtactgacgctgtgatgctgtctgcagaaactgccgctgggcagtatccgtcagaaaccgttgcagccatggcgcgcgtttgcctgggtgcggaaaaaatcccgagcatcaacgtttctaaacaccgtctggacgttcagttcgacaatgtggaagaagctattgccatgtcagcaatgtacgcagctaaccacctgaaaggcgttacggcgatcatcaccatgaccgaatcgggtcgtaccgcgctgatgacctcccgtatcagctctggtctgccaattttcgccatgtcgcgccatgaacgtacgctgaacctgactgctctctatcgtggcgttacgccggtgcactttgatagcgctaatgacggcgtagcagctgccagcgaagcggttaatctgctgcgcgataaaggttacttgatgtctggtgacctggtgattgtcacccagggcgacgtgatgagtaccgtgggttctactaataccacgcgtattttaacggtagagtaa

SEQ ID NO: 75 - protein, 480 aa, Escherichia coli
MSRRLRRTKIVTTLGPATDRDNNLEKVIAAGANVVRMNFSHGSPEDHKMRADKVREIAAKLGRHVAILGDLQGPKIRVSTFKEGKVFLNIGDKFLLDANLGKGEGDKEKVGIDYKGLPADVVPGDILLLDDGRVQLKVLEVQGMKVFTEVTVGGPLSNNKGINKLGGGLSAEALTEKDKADIKTAALIGVDYLAVSFPRCGEDLNYARRLARDAGCDAKIVAKVERAEAVCSQDAMDDIILASDVVMVARGDLGVEIGDPELVGIQKALIRRARQLNRAVITATQMMESMITNPMPTRAEVMDVANAVLDGTDAVMLSAETAAGQYPSETVAAMARVCLGAEKIPSINVSKHRLDVQFDNVEEAIAMSAMYAANHLKGVTAIITMTESGRTALMTSRISSGLPIFAMSRHERTLNLTALYRGVTPVHFDSANDGVAAASEAVNLLRDKGYLMSGDLVIVTQGDVMSTVGSTNTTRILTVE

SEQ ID NO: 76 - DNA, 1413 bp, Escherichia coli
atgaaaaagaccaaaattgtttgcaccatcggaccgaaaaccgaatctgaagagatgttagctaaaatgctggacgctggcatgaacgttatgcgtctgaacttctctcatggtgactatgcagaacacggtcagcgcattcagaatctgcgcaacgtgatgagcaaaactggtaaaaccgccgctatcctgcttgataccaaaggtccggaaatccgcaccatgaaactggaaggcggtaacgacgtttctctgaaagctggtcagacctttactttcaccactgataaatctgttatcggcaacagcgaaatggttgcggtaacgtatgaaggtttcactactgacctgtctgttggcaacaccgtactggttgacgatggtctgatcggtatggaagttaccgccattgaaggtaacaaagttatctgtaaagtgctgaacaacggtgacctgggcgaaaacaaaggtgtgaacctgcctggcgtttccattgctctgccagcactggctgaaaaagacaaacaggacctgatctttggttgcgaacaaggcgtagactttgttgctgcttcctttattcgtaagcgttctgacgttatcgaaatccgtgagcacctgaaagcgcacggcggcgaaaacatccacatcatctccaaaatcgaaaaccaggaaggcctcaacaacttcgacgaaatcctcgaagcctctgacggcatcatggttgcgcgtggcgacctgggtgtagaaatcccggtagaagaagttatcttcgcccagaagatgatgatcgaaaaatgtatccgtgcacgtaaagtcgttatcactgcgacccagatgctggattccatgatcaaaaacccacgcccgactcgcgcagaagccggtgacgttgcaaacgccatcctcgacggtactgacgcagtgatgctgtctggtgaatccgcaaaaggtaaatacccgctggaagcggtttctatcatggcgaccatctgcgaacgtaccgaccgcgtgatgaacagccgtctcgagttcaacaatgacaaccgtaaactgcgcattaccgaagcggtatgccgtggtgccgttgaaactgctgaaaaactggatgctccgctgatcgtggttgctactcagggcggtaaatctgctcgcgcagtacgtaaatacttcccggatgccaccatcctggcactgaccaccaacgaaaaaacggctcatcagttggtactgagcaaaggcgttgtgccgcagcttgttaaagagatcacttctactgatgatttctaccgtctgggtaaagaactggctctgcagagcggtctggcacacaaaggtgacgttgtagttatggtttctggtgcactggtaccgagcggcactactaacaccgcatctgttcacgtcctgtaa

SEQ ID NO: 77 - protein, 470 aa, Escherichia coli
MKKTKIVCTIGPKTESEEMLAKMLDAGMNVMRLNFSHGDYAEHGQRIQNLRNVMSKTGKTAAILLDTKGPEIRTMKLEGGNDVSLKAGQTFTFTTDKSVIGNSEMVAVTYEGFTTDLSVGNTVLVDDGLIGMEVTAIEGNKVICKVLNNGDLGENKGVNLPGVSIALPALAEKDKQDLIFGCEQGVDFVAASFIRKRSDVIEIREHLKAHGGENIHIISKIENQEGLNNFDEILEASDGIMVARGDLGVEIPVEEVIFAQKMMIEKCIRARKVVITATQMLDSMIKNPRPTRAEAGDVANAILDGTDAVMLSGESAKGKYPLEAVSIMATICERTDRVMNSRLEFNNDNRKLRITEAVCRGAVETAEKLDAPLIVVATQGGKSARAVRKYFPDATILALTTNEKTAHQLVLSKGVVPQLVKEITSTDDFYRLGKELALQSGLAHKGDVVVMVSGALVPSGTTNTASVHVL

SEQ ID NO: 78 - DNA, 1410 bp, Escherichia coli
atgtccgctgaacacgtactgacgatgctgaacgagcacgaagtgaagtttgttgatttgcgcttcaccgatactaaaggtaaagaacagcacgtcactatccctgctcatcaggtgaatgctgaattcttcgaagaaggcaaaatgtttgacggctcctcgattggcggctggaaaggcattaacgagtccgacatggtgctgatgccagacgcatccaccgcagtgattgacccgttcttcgccgactccaccctgattatccgttgcgacatccttgaacctggcaccctgcaaggctatgaccgtgacccgcgctccattgcgaagcgcgccgaagattacctgcgttccactggcattgccgacaccgtactgttcgggccagaacctgaattcttcctgttcgatgacatccgtttcggatcatctatctccggttcccacgttgctatcgacgatatcgaaggcgcatggaactcctccacccaatacgaaggtggtaacaaaggtcaccgtccggcagtgaaaggcggttacttcccggttccaccggtagactcggctcaggatattcgttctgaaatgtgtctggtgatggaacagatgggtctggtggttgaagcccatcaccacgaagtagcgactgctggtcagaacgaagtggctacccgcttcaataccatgaccaaaaaagctgacgaaattcagatctacaaatatgttgtgcacaacgtagcgcaccgcttcggtaaaaccgcgacctttatgccaaaaccgatgttcggtgataacggctccggtatgcactgccacatgtctctgtctaaaaacggcgttaacctgttcgcaggcgacaaatacgcaggtctgtctgagcaggcgctgtactacattggcggcgtaatcaaacacgctaaagcgattaacgccctggcaaacccgaccaccaactcttataagcgtctggtcccgggctatgaagcaccggtaatgctggcttactctgcgcgtaaccgttctgcgtctatccgtattccggtggtttcttctccgaaagcacgtcgtatcgaagtacgtttcccggatccggcagctaacccgtacctgtgctttgctgccctgctgatggccggtcttgatggtatcaagaacaagatccatccgggcgaagccatggacaaaaacctgtatgacctgccgccagaagaagcgaaagagatcccacaggttgcaggctctctggaagaagcactgaacgaactggatctggaccgcgagttcctgaaagccggtggcgtgttcactgacgaagcaattgatgcgtacatcgctctgcgtcgcgaagaagatgaccgcgtgcgtatgactccgcatccggtagagtttgagctgtactacagcgtctaa

SEQ ID NO: 79 - protein, 469 aa, Escherichia coli
MSAEHVLTMLNEHEVKFVDLRFTDTKGKEQHVTIPAHQVNAEFFEEGKMFDGSSIGGWKGINESDMVLMPDASTAVIDPFFADSTLIIRCDILEPGTLQGYDRDPRSIAKRAEDYLRSTGIADTVLFGPEPEFFLFDDIRFGSSISGSHVAIDDIEGAWNSSTQYEGGNKGHRPAVKGGYFPVPPVDSAQDIRSEMCLVMEQMGLVVEAHHHEVATAGQNEVATRFNTMTKKADEIQIYKYVVHNVAHRFGKTATFMPKPMFGDNGSGMHCHMSLSKNGVNLFAGDKYAGLSEQALYYIGGVIKHAKAINALANPTTNSYKRLVPGYEAPVMLAYSARNRSASIRIPVVSSPKARRIEVRFPDPAANPYLCFAALLMAGLDGIKNKIHPGEAMDKNLYDLPPEEAKEIPQVAGSLEEALNELDLDREFLKAGGVFTDEAIDAYIALRREEDDRVRMTPHPVEFELYYSV

SEQ ID NO: 80 - DNA, 4461 bp, Escherichia coli
atgttgtacgataaatcccttgagagggataactgtggtttcggcctgatcgcccacatagaaggcgaacctagccacaaggtagtgcgtactgcaatacacgcactggcccgcatgcagcaccgtggcgcgattctcgccgatggtaaaaccggcgacggttgcggcttgctgttacaaaaaccggatcgcttttttcgcatcgttgcgcaggagcgcggctggcgtttagcaaaaaactacgctgtcgggatgctcttcctgaataaagatcctgaactcgccgctgccgcacgccgcatcgttgaagaagaactgcaacgcgaaaccttgtcgattgtgggctggcgtgatgtccccactaacgaaggcgtgctgggtgaaatcgccctctcctctctgccacgcattgagcaaatttttgtgaacgccccggcaggctggcgtccacgcgatatggagcgccgtctgtttatcgcccgccgccgcattgaaaagcgtctcgaagccgacaaagacttctacgtctgtagcctgtcgaatctggtgaacatctataaaggtctgtgtatgccgacggatctgccgcgcttttatctggatcttgcggacctgcgtctggaatcggccatttgcctgttccaccagcgcttctccactaacaccgtaccgcgctggccgctggcgcaaccgttccgctatctggcgcataacggtgaaatcaacaccatcaccggtaaccgccaatgggcgcgtgcgcgtacttataaattccagacaccgcttatccctgacctgcacgacgccgcaccgttcgtcaacgaaaccggctctgactccagttcgatggataacatgctggaactgctgctggcaggcgggatggatatcatccgcgccatgcgtctattagtaccacccgcctggcagaacaacccggatatggacccggaactgcgtgccttctttgactttaactccatgcatatggagccgtgggatggcccggcgggcatcgtgatgtccgacggtcgttttgccgcctgtaacctcgaccgtaacggtctgcgtccggcgcgctacgtcatcaccaaagataagctcatcacctgcgcctctgaagtcggtatctgggattaccagcctgacgaagtggtcgaaaaaggccgcgtcgggccaggcgaactgatggttatcgacacccgcagtgggcgtattctgcactcggcagaaaccgatgacgatctgaaaagccgccatccatataaagagtggatggagaaaaacgtccgccgactggtaccgtttgaagatctgcccgatgaagaagtgggtagccgcgaactggacgacgacacgcttgccagctaccagaaacagtttaactacagcgcggaagagctggactccgtaattcgcgtactgggcgaaaacggtcaggaagcggtcggttcgatgggcgatgataccccattcgccgtgctctccagtcagccgcgcattatttacgactacttccgccagcagtttgcccaggtgactaacccgccaatcgacccgctgcgtgaagcgcatgttatgtcgctcgccaccagtatcggtcgtgaaatgaacgtcttttgcgaagcagagggccaggcgcaccgtttaagctttaaatcgccgattctgctctactccgatttcaaacagctcacgacgatgaaagaggagcactaccgcgcagatacgctggatatcacctttgacgtcactaaaaccacgctcgaagcgacagtcaaagagctgtgcgacaaagccgaaaaaatggtacgtagcggcaccgtgctgctggtgctctccgaccggaatatcgctaaagatcgcctgccggttccagccccgatggcggttggcgcgatccagacccgtctggtcgatcaaagcctgcgttgcgatgccaacatcatcgtcgaaaccgccagcgcccgcgatccgcaccacttcgccgtgttgctgggcttcggcgcgacggctatttatccataccttgcctatgaaacgctgggccgcctggtagacacccatgcgattgccaaagattatcgtaccgtgatgctcaactaccgtaacggcatcaacaaaggcttgtacaaaatcatgtccaaaatgggcatctccaccatcgcctcttaccgctgctcgaaactgtttgaagcggtcggtctacacgatgatgtagtgggcctgtgcttccagggggcggtcagccgcattggtggagcaagctttgaagacttccagcaggatctgctgaatctgtcgaaacgtgcctggctggcgcgtaagcccatcagccagggcggtctgctgaaatacgtccacggcggcgaataccacgcctacaacccggacgtggtgcgcacgctgcaacaagcggtacaaagcggcgagtacagcgactatcaggaatacgcgaagctggttaatgagcgtccggcaaccacgctgcgcgatctgctggcaattacgccgggtgaaaacgcggtcaacattgctgatgttgaaccggcaagcgaactgtttaaacgctttgataccgccgcgatgtctatcggcgcgttaagcccggaagcccacgaggcgctggcggaagcgatgaacagcatcggcggtaattcgaactccggtgaaggcggcgaagacccggcgcgctacggcaccaacaaagtgtcgcgcatcaagcaggtggcttccggtcgctttggggttactccggcgtatctggtcaatgccgacgtcattcagattaaagtcgcccagggcgcgaagccaggcgaaggcggtcagttgccgggtgataaagtcacgccttacatcgccaaactgcgctattcggtgcccggagtgacgctgatctccccgccgccgcaccacgatatctactctatcgaggacttagcgcagctcattttcgacctcaagcaggttaacccgaaagcgatgatctccgtgaagctggtttccgaaccgggagtaggcaccatcgcgactggcgtggcaaaagcttatgcggacttgatcaccatcgcaggctatgacggcggcaccggcgcaagtccgctttcatcggtgaaatacgcaggctgtccgtgggagctggggcttgttgaaacccagcaggcgctggttgctaacggcttgcgtcacaagatccgtttgcaggtcgatggcggcctgaaaacgggtgtcgatatcatcaaggcggcgattctcggcgcagaaagcttcggcttcggcactggcccgatggtggcgctcggctgtaaatatctacgtatttgccatctgaacaactgcgcaacgggtgtagcaactcaggatgacaaactgcgtaagaaccactatcacggcctgccattcaaggtgacgaattactttgagtttatcgcccgtgaaacccgcgagctgatggcacagcttggcgtaacacgtctggtggatctgattggtcgcaccgacctgctgaaagagctggacggtttcaccgccaaacagcagaagctggcgctgtcgaagctgctggagactgccgaaccgcatccaggtaaggcactctactgcaccgaaaacaacccgccgtttgataacggcctgctgaacgcgcagttgctgcaacaggcgaaaccgtttgtcgatgagcgccagagcaaaaccttctggttcgatattcgcaacaccgaccgttctgtcggcgcgtcgctttcaggctatatcgcccagacgcacggcgatcaggggctggcagccgatcctatcaaagcgtacttcaacggcaccgcaggccagagcttcggcgtgtggaacgcgggcggcgtggaactgtacctgaccggtgatgccaacgactatgtcggtaaaggcatggcgggcggcttaatcgccattcgtcctccggttggttccgccttccgcagccatgaagcaagcattatcggcaacacctgcctgtatggcgcgaccggtggtcgtctgtatgccgcaggccgcgcgggtgaacgtttcggcgtgcgtaactccggtgctatcaccgtggtagaaggcattggcgacaacggttgtgaatatatgacgggtggtatcgtctgcattctgggtaaaaccggcgttaacttcggtgcgggcatgaccggcggtttcgcttacgttctcgatgaaagcggcgatttccgcaaacgcgttaacccggaactggtcgaggtcttaagcgttgacgctctggcgatccatgaagagcatctgcgtggtcttatcaccgagcatgtgcagcataccggctctcagcgcggtgaagagattctggcgaactggtcaaccttcgccactaaatttgcgctggttaaaccgaagtccagtgatgtaaaagcactgctgggtcaccgtagtcgtagcgcagctgagttgcgcgtgcaggcgcagtaa

SEQ ID NO: 81 - protein, 1486 aa, Escherichia coli
MLYDKSLERDNCGFGLIAHIEGEPSHKVVRTAIHALARMQHRGAILADGKTGDGCGLLLQKPDRFFRIVAQERGWRLAKNYAVGMLFLNKDPELAAAARRIVEEELQRETLSIVGWRDVPTNEGVLGEIALSSLPRIEQIFVNAPAGWRPRDMERRLFIARRRIEKRLEADKDFYVCSLSNLVNIYKGLCMPTDLPRFYLDLADLRLESAICLFHQRFSTNTVPRWPLAQPFRYLAHNGEINTITGNRQWARARTYKFQTPLIPDLHDAAPFVNETGSDSSSMDNMLELLLAGGMDIIRAMRLLVPPAWQNNPDMDPELRAFFDFNSMHMEPWDGPAGIVMSDGRFAACNLDRNGLRPARYVITKDKLITCASEVGIWDYQPDEVVEKGRVGPGELMVIDTRSGRILHSAETDDDLKSRHPYKEWMEKNVRRLVPFEDLPDEEVGSRELDDDTLASYQKQFNYSAEELDSVIRVLGENGQEAVGSMGDDTPFAVLSSQPRIIYDYFRQQFAQVTNPPIDPLREAHVMSLATSIGREMNVFCEAEGQAHRLSFKSPILLYSDFKQLTTMKEEHYRADTLDITFDVTKTTLEATVKELCDKAEKMVRSGTVLLVLSDRNIAKDRLPVPAPMAVGAIQTRLVDQSLRCDANIIVETASARDPHHFAVLLGFGATAIYPYLAYETLGRLVDTHAIAKDYRTVMLNYRNGINKGLYKIMSKMGISTIASYRCSKLFEAVGLHDDVVGLCFQGAVSRIGGASFEDFQQDLLNLSKRAWLARKPISQGGLLKYVHGGEYHAYNPDVVRTLQQAVQSGEYSDYQEYAKLVNERPATTLRDLLAITPGENAVNIADVEPASELFKRFDTAAMSIGALSPEAHEALAEAMNSIGGNSNSGEGGEDPARYGTNKVSRIKQVASGRFGVTPAYLVNADVIQIKVAQGAKPGEGGQLPGDKVTPYIAKLRYSVPGVTLISPPPHHDIYSIEDLAQLIFDLKQVNPKAMISVKLVSEPGVGTIATGVAKAYADLITIAGYDGGTGASPLSSVKYAGCPWELGLVETQQALVANGLRHKIRLQVDGGLKTGVDIIKAAILGAESFGFGTGPMVALGCKYLRICHLNNCATGVATQDDKLRKNHYHGLPFKVTNYFEFIARETRELMAQLGVTRLVDLIGRTDLLKELDGFTAKQQKLALSKLLETAEPHPGKALYCTENNPPFDNGLLNAQLLQQAKPFVDERQSKTFWFDIRNTDRSVGASLSGYIAQTHGDQGLAADPIKAYFNGTAGQSFGVWNAGGVELYLTGDANDYVGKGMAGGLIAIRPPVGSAFRSHEASIIGNTCLYGATGGRLYAAGRAGERFGVRNSGAITVVEGIGDNGCEYMTGGIVCILGKTGVNFGAGMTGGFAYVLDESGDFRKRVNPELVEVLSVDALAIHEEHLRGLITEHVQHTGSQRGEEILANWSTFATKFALVKPKSSDVKALLGHRSRSAAELRVQAQ

SEQ ID NO: 82 - DNA, 1419 bp, Escherichia coli
atgagtcagaatgtttatcaatttatcgacctgcagcgcgttgatccgccaaagaaaccgctgaagatccgcaaaattgagtttgttgaaatttacgagccgttttccgaaggccaggccaaagcgcaggctgaccgctgcctgtcgtgcggcaacccatactgcgagtggaaatgcccggtacacaactacatcccgaactggctgaagctcgccaacgaggggcgtatttttgaagcggcggaactgtcgcaccagaccaacaccctgccggaagtttgcggacgagtctgcccgcaagaccgtctgtgcgaaggttcctgcactctgaacgatgagtttggcgcggtgaccatcggcaacattgagcgctatatcaacgataaagcgttcgagatgggctggcgtccggatatgtctggtgtgaaacagaccggtaaaaaagtggcgattatcggcgcaggcccggcaggtctggcgtgtgcggatgtcctgacgcgtaacggcgtaaaagccgttgtcttcgaccgtcatccagaaattggcgggctgctgaccttcggtattccggccttcaagctggaaaaagaggtaatgacgcgtcgccgtgaaatcttcaccggcatgggtattgaattcaaactcaataccgaagtgggccgcgacgtacagctggacgatctgctgagtgattacgatgccgtgttccttggcgtcgggacttatcagtcaatgcgcggcgggctggaaaacgaagacgccgatggcgtgtacgcagcgctgccgttcctcatcgccaacaccaaacagttaatgggctttggtgaaacccgcgacgaaccgttcgtcagcatggaaggcaaacgcgtggtggtccttggcggtggcgacactgcgatggactgcgtgcgtacgtccgtgcgccagggagcgaagcacgttacctgtgcctatcgtcgtgatgaagagaacatgccgggttcccgccgcgaagtgaaaaacgcgcgggaagaaggcgtagagttcaaattcaacgtccagccgctgggtattgaagtgaacggtaacggcaaagtcagcggcgtaaaaatggtgcgtaccgaaatgggcgaaccggacgccaaaggccgtcgccgcgcggagatcgttgcaggttccgaacatatcgttccggcagatgcggtgatcatggcgtttggtttccgtccacacaacatggaatggctggcaaaacacagcgtcgagctggattcacaaggccgcatcatcgccccggaaggcagcgacaacgccttccagaccagcaacccgaaaatctttgctggcggcgatatcgtccgtggttccgatctggtggtgaccgctattgccgaaggtcgtaaggcggcagacggtattatgaactggctggaagtttaa

SEQ ID NO: 83 - protein, 472 aa, Escherichia coli
MSQNVYQFIDLQRVDPPKKPLKIRKIEFVEIYEPFSEGQAKAQADRCLSCGNPYCEWKCPVHNYIPNWLKLANEGRIFEAAELSHQTNTLPEVCGRVCPQDRLCEGSCTLNDEFGAVTIGNIERYINDKAFEMGWRPDMSGVKQTGKKVAIIGAGPAGLACADVLTRNGVKAVVFDRHPEIGGLLTFGIPAFKLEKEVMTRRREIFTGMGIEFKLNTEVGRDVQLDDLLSDYDAVFLGVGTYQSMRGGLENEDADGVYAALPFLIANTKQLMGFGETRDEPFVSMEGKRVVVLGGGDTAMDCVRTSVRQGAKHVTCAYRRDEENMPGSRREVKNAREEGVEFKFNVQPLGIEVNGNGKVSGVKMVRTEMGEPDAKGRRRAEIVAGSEHIVPADAVIMAFGFRPHNMEWLAKHSVELDSQGRIIAPEGSDNAFQTSNPKIFAGGDIVRGSDLVVTAIAEGRKAADGIMNWLEV

SEQ ID NO: 84 - DNA, 1665 bp, Escherichia coli
atgtgttcaatttttggcgtattcgatatcaaaacagacgcagttgagctgcgtaagaaagccctcgagctgtcacgcctgatgcgtcatcgtggcccggactggtccggtatttatgccagcgataacgccattctcgcccacgaacgtctgtcaattgttgacgttaacgcgggggcgcaacctctctacaaccaacaaaaaacccacgtactggcggtaaacggtgaaatctacaaccaccaggcattgcgcgccgaatatggcgatcgttaccagttccagaccgggtctgactgtgaagtgatcctcgcgctgtatcaggaaaaagggccggaatttctcgacgacttgcagggcatgtttgcctttgcactgtacgacagcgaaaaagatgcctacctgattggtcgcgaccatctggggatcatcccactgtatatggggtatgacgaacacggtcagctgtatgtggcctcagaaatgaaagcgctggtgccagtttgccgcacgattaaagagttcccggcggggagctatttgtggagccaggacggcgaaatccgttcttactatcatcgcgactggttcgactacgatgcggtgaaagataacgtgaccgacaaaaacgagctgcgtcaggcactggaagattcagttaaaagccatctgatgtctgatgtgccttacggtgtgctgctttctggtggtctggattcctcaattatttccgctatcaccaagaaatacgcagcccgtcgcgtggaagatcaggaacgctctgaagcctggtggccgcagttacactcctttgctgtaggtctgccgggttcaccggatctgaaagcagcccaggaagtggcaaaccatctgggcacggtgcatcacgaaattcacttcactgtacaggaaggtctggatgccatccgcgacgtgatttaccacatcgaaacttatgatgtgaccactattcgcgcttcaacaccgatgtatttaatgtcgcgtaagatcaaggcgatgggcattaaaatggtgctgtccggtgaaggttctgatgaagtgttcggcggttatctttacttccacaaagcaccgaatgccaaagaactgcatgaagagacggtgcgtaaactgctggccctgcatatgtatgactgcgcgcgtgccaacaaagcgatgtcagcctggggcgtggaagcacgcgttccgttcctcgacaaaaaattccttgatgtggcgatgcgtattaacccacaggataaaatgtgcggtaacggcaaaatggaaaaacacatcctgcgtgaatgttttgaagcgtatctgcctgcaagcgtggcctggcggcagaaagagcagttctccgatggcgtcggttacagttggatcgacaccctgaaagaagtggctgcgcagcaggtttctgatcagcaactggaaactgcccgcttccgcttcccgtacaacacgccaacctctaaagaagcgtacttgtatcgggagatctttgaagaactattcccgcttccgagcgccgctgagtgcgtgccgggcggtccttccgtcgcttgttcttccgctaaagcgatcgaatgggatgaagcgttcaagaaaatggacgatccgtctggtcgcgcggttggtgttcaccagtcggcgtataagtaa

SEQ ID NO: 85 - protein, 554 aa, Escherichia coli
MCSIFGVFDIKTDAVELRKKALELSRLMRHRGPDWSGIYASDNAILAHERLSIVDVNAGAQPLYNQQKTHVLAVNGEIYNHQALRAEYGDRYQFQTGSDCEVILALYQEKGPEFLDDLQGMFAFALYDSEKDAYLIGRDHLGIIPLYMGYDEHGQLYVASEMKALVPVCRTIKEFPAGSYLWSQDGEIRSYYHRDWFDYDAVKDNVTDKNELRQALEDSVKSHLMSDVPYGVLLSGGLDSSIISAITKKYAARRVEDQERSEAWWPQLHSFAVGLPGSPDLKAAQEVANHLGTVHHEIHFTVQEGLDAIRDVIYHIETYDVTTIRASTPMYLMSRKIKAMGIKMVLSGEGSDEVFGGYLYFHKAPNAKELHEETVRKLLALHMYDCARANKAMSAWGVEARVPFLDKKFLDVAMRINPQDKMCGNGKMEKHILRECFEAYLPASVAWRQKEQFSDGVGYSWIDTLKEVAAQQVSDQQLETARFRFPYNTPTSKEAYLYREIFEELFPLPSAAECVPGGPSVACSSAKAIEWDEAFKKMDDPSGRAVGVHQSAYK

SEQ ID NO: 86 - DNA, 933 bp, Escherichia coli
atgttagatgcaaacaaattacagcaggcagtggatcaggcttacacccaatttcactcacttaacggcggacaaaatgccgattacattccctttctggcgaatgtaccaggtcaactggcggcagtggctatcgtgacctgcgatggcaacgtctatagtgcgggtgacagtgattaccgctttgcactggaatccatctcgaaagtctgtacgttagcccttgcgttagaagatgtcggcccgcaggcggtacaggacaaaattggcgctgacccgaccggattgccctttaactcagttatcgccttagagttgcatggcggcaaaccgctttcgccactggtaaatgctggcgctattgccaccaccagcctgattaacgctgaaaatgttgaacaacgctggcagcgaattttacatatccaacagcaactggctggcgagcaggtagcgctctctgacgaagtcaaccagtcggaacaaacaaccaacttccataaccgggccatagcctggctgctgtactccgccggatatctctattgtgatgcaatggaagcctgtgacgtgtatacccgtcagtgctccacgctcctcaatactattgaactggcaacgcttggcgcgacgctggcggcaggtggtgtgaatccgttgacgcataaacgcgttcttcaggccgacaacgtgccgtacattctggccgaaatgatgatggaagggctgtatggtcgctccggtgactgggcgtatcgtgttggtttaccgggcaaaagcggtgtaggtggcggtattctggcggtcgtccctggagtgatgggaattgccgcgttctcaccaccgctggacgaagatggcaacagtgttcgcggtcaaaaaatggtggcatcggtcgctaagcaactcggctataacgtgtttaagggctga

SEQ ID NO: 87 - protein, 310 aa, Escherichia coli
MLDANKLQQAVDQAYTQFHSLNGGQNADYIPFLANVPGQLAAVAIVTCDGNVYSAGDSDYRFALESISKVCTLALALEDVGPQAVQDKIGADPTGLPFNSVIALELHGGKPLSPLVNAGAIATTSLINAENVEQRWQRILHIQQQLAGEQVALSDEVNQSEQTTNFHNRAIAWLLYSAGYLYCDAMEACDVYTRQCSTLLNTIELATLGATLAAGGVNPLTHKRVLQADNVPYILAEMMMEGLYGRSGDWAYRVGLPGKSGVGGGILAVVPGVMGIAAFSPPLDEDGNSVRGQKMVASVAKQLGYNVFKG

SEQ ID NO: 88 - DNA, 927 bp, Escherichia coli
atggcagtcgccatggataatgcaattttagaaaacatcttgcggcaagtgcggccgctcattggtcagggtaaagtcgcggattatattccggcgctggctacagtagacggttcccgattggggattgctatctgtaccgttgacggacagctttttcaggccggagacgcgcaagaacgtttttccattcagtctatttccaaagtgctgagtctcgttgtcgccatgcgtcattactccgaagaggaaatctggcaacgcgtcggcaaagatccgtctggatcaccgttcaattccttagtgcaactggaaatggagcagggtataccgcgtaatccgttcattaatgccggtgcgctggtggtctgcgatatgttgcaagggcgattaagcgcaccacggcaacgtatgctggaagtcgtgcgcggcttaagcggtgtgtctgatatttcctacgatacggtggtagcgcgttccgaatttgaacattccgcgcgaaatgcggctatcgcctggctgatgaagtcgtttggcaatttccatcatgacgtgacaaccgttctgcaaaactactttcattactgcgctctgaaaatgagctgtgtagagctggcccggacgtttgtctttctggctaatcaggggaaagctattcatattgatgaaccagtggtgacgccaatgcaggcgcggcaaattaacgcgctgatggcgaccagtggtatgtaccagaacgcgggggagtttgcctggcgggtggggctaccggcgaaatctggcgttggtggcggtattgtggcgattgttccgcatgaaatggccatcgctgtctggagtccggaactggatgatgcaggtaactcgcttgcgggtattgccgttcttgaacaattgacgaaacagttagggcgttcggtttattaa

SEQ ID NO: 89 - protein, 927 aa, Escherichia coli
GTGGCAGTCGCCATGGATAATGCAATTTTAGAAAACATCTTGCGGCAAGTGCGGCCGCTCATTGGTCAGGGTAAAGTCGCGGATTATATTCCGGCGCTGGCTACAGTAGACGGTTCCCGATTGGGGATTGCTATCTGTACCGTTGACGGACAGCTTTTTCAGGCCGGAGACGCGCAAGAACGTTTTTCCATTCAGTCTATTTCCAAAGTGCTGAGTCTCGTTGTCGCCATGCGTCATTACTCCGAAGAGGAAATCTGGCAACGCGTCGGCAAAGATCCGTCTGGATCACCGTTCAATTCCTTAGTGCAACTGGAAATGGAGCAGGGTATACCGCGTAATCCGTTCATTAATGCCGGTGCGCTGGTGGTCTGCGATATGTTGCAAGGGCGATTAAGCGCACCACGGCAACGTATGCTGGAAGTCGTGCGCGGCTTAAGCGGTGTGTCTGATATTTCCTACGATACGGTGGTAGCGCGTTCCGAATTTGAACATTCCGCGCGAAATGCGGCTATCGCCTGGCTGATGAAGTCGTTTGGCAATTTCCATCATGACGTGACAACCGTTCTGCAAAACTACTTTCATTACTGCGCTCTGAAAATGAGCTGTGTAGAGCTGGCCCGGACGTTTGTCTTTCTGGCTAATCAGGGGAAAGCTATTCATATTGATGAACCAGTGGTGACGCCAATGCAGGCGCGGCAAATTAACGCGCTGATGGCGACCAGTGGTATGTACCAGAACGCGGGGGAGTTTGCCTGGCGGGTGGGGCTACCGGCGAAATCTGGCGTTGGTGGCGGTATTGTGGCGATTGTTCCGCATGAAATGGCCATCGCTGTCTGGAGTCCGGAACTGGATGATGCAGGTAACTCGCTTGCGGGTATTGCCGTTCTTGAACAATTGACGAAACAGTTAGGGCGTTCGGTTTATTAA

SEQ ID NO: 90 - DNA, 1344 bp, Escherichia coli
atggatcagacatattctctggagtcattcctcaaccatgtccaaaagcgcgacccgaatcaaaccgagttcgcgcaagccgttcgtgaagtaatgaccacactctggccttttcttgaacaaaatccaaaatatcgccagatgtcattactggagcgtctggttgaaccggagcgcgtgatccagtttcgcgtggtatgggttgatgatcgcaaccagatacaggtcaaccgtgcatggcgtgtgcagttcagctctgccatcggcccgtacaaaggcggtatgcgcttccatccgtcagttaacctttccattctcaaattcctcggctttgaacaaaccttcaaaaatgccctgactactctgccgatgggcggtggtaaaggcggcagcgatttcgatccgaaaggaaaaagcgaaggtgaagtgatgcgtttttgccaggcgctgatgactgaactgtatcgccacctgggcgcggataccgacgttccggcaggtgatatcggggttggtggtcgtgaagtcggctttatggcggggatgatgaaaaagctctccaacaataccgcctgcgtcttcaccggtaagggcctttcatttggcggcagtcttattcgcccggaagctaccggctacggtctggtttatttcacagaagcaatgctaaaacgccacggtatgggttttgaagggatgcgcgtttccgtttctggctccggcaacgtcgcccagtacgctatcgaaaaagcgatggaatttggtgctcgtgtgatcactgcgtcagactccagcggcactgtagttgatgaaagcggattcacgaaagagaaactggcacgtcttatcgaaatcaaagccagccgcgatggtcgagtggcagattacgccaaagaatttggtctggtctatctcgaaggccaacagccgtggtctctaccggttgatatcgccctgccttgcgccacccagaatgaactggatgttgacgccgcgcatcagcttatcgctaatggcgttaaagccgtcgccgaaggggcaaatatgccgaccaccatcgaagcgactgaactgttccagcaggcaggcgtactatttgcaccgggtaaagcggctaatgctggtggcgtcgctacatcgggcctggaaatggcacaaaacgctgcgcgcctgggctggaaagccgagaaagttgacgcacgtttgcatcacatcatgctggatatccaccatgcctgtgttgagcatggtggtgaaggtgagcaaaccaactacgtgcagggcgcgaacattgccggttttgtgaaggttgccgatgcgatgctggcgcagggtgtgatttaa

SEQ ID NO: 91 - protein, 447 aa, Escherichia coli
MDQTYSLESFLNHVQKRDPNQTEFAQAVREVMTTLWPFLEQNPKYRQMSLLERLVEPERVIQFRVVWVDDRNQIQVNRAWRVQFSSAIGPYKGGMRFHPSVNLSILKFLGFEQTFKNALTTLPMGGGKGGSDFDPKGKSEGEVMRFCQALMTELYRHLGADTDVPAGDIGVGGREVGFMAGMMKKLSNNTACVFTGKGLSFGGSLIRPEATGYGLVYFTEAMLKRHGMGFEGMRVSVSGSGNVAQYAIEKAMEFGARVITASDSSGTVVDESGFTKEKLARLIEIKASRDGRVADYAKEFGLVYLEGQQPWSLPVDIALPCATQNELDVDAAHQLIANGVKAVAEGANMPTTIEATELFQQAGVLFAPGKAANAGGVATSGLEMAQNAARLGWKAEKVDARLHHIMLDIHHACVEHGGEGEQTNYVQGANIAGFVKVADAMLAQGVI

SEQ ID NO: 92 - DNA, 1479 bp, Escherichia coli
atgagcttacgtgaaaaaaccatcagcggcgcgaagtggtcggcgattgccacggtgatcatcatcggcctcgggctggtgcagatgaccgtgctggcgcggattatcgacaaccaccagttcggcctgcttaccgtgtcgctggtgattatcgcgctggcagatacgctttctgacttcggtatcgctaactcgattattcagcgaaaagaaatcagtcaccttgaactcaccacgttgtactggctgaacgtcgggctggggatcgtggtgtgcgtggcggtgtttttgttgagtgatctcatcggcgacgtgctgaataacccggacctggcaccgttgattaaaacattatcgctggcgtttgtggtaatcccccacgggcaacagttccgcgcgttgatgcaaaaagagctggagttcaacaaaatcggcatgatcgaaaccagcgcggtgctggcgggcttcacttgtacggtggttagcgcccatttctggccgctggcgatgaccgcgatcctcggttatctggtcaatagtgcggtgagaacgctgctgtttggctactttggccgcaaaatttatcgccccggtctgcatttctcgctggcgtcggtggcaccgaacttacgctttggtgcctggctgacggcggacagcatcatcaactatctcaataccaacctttcaacgctcgtgctggcgcgtattctcggcgcgggcgtggcagggggatacaacctggcgtacaacgtggccgttgtgccaccgatgaagctgaacccaatcatcacccgcgtgttgtttccggcattcgccaaaattcaggacgataccgaaaagctgcgtgttaacttctacaagctgctgtcggtagtggggattatcaactttccggcgctgctcgggctaatggtggtgtcgaataactttgtaccgctggtctttggtgagaagtggaacagcattattccggtgctgcaattgctgtgtgtggtgggtctgctgcgctccgtaggtaacccgattggttcgctgctgatggcgaaagcgcgggtcgatatcagctttaaattcaacgtattcaaaacatttctgtttattccggcgattgttataggtgggcagatggcgggcgcgatcggcgtcacgcttggcttcctgctggtgcaaattatcaacaccattctgagttacttcgtgatgattaaaccggttcttggttccagttatcgccagtacatcctgagtttatggctgccgttttatctctcgctgccgacgctggtggtcagttatgcgctgggcattgtgctgaaagggcaactggcgctggggatgctgctggcggtgcaaatagccacgggggtgctggcgtttgtggtgatgattgtgctgtcgcgccatccgctggtggtggaagtgaagcgtcagttttgtcgcagcgaaaaaatgaaaatgcttttacgggcggggtga

SEQ ID NO: 93 - protein, 492 aa, Escherichia coli
MSLREKTISGAKWSAIATVIIIGLGLVQMTVLARIIDNHQFGLLTVSLVIIALADTLSDFGIANSIIQRKEISHLELTTLYWLNVGLGIVVCVAVFLLSDLIGDVLNNPDLAPLIKTLSLAFVVIPHGQQFRALMQKELEFNKIGMIETSAVLAGFTCTVVSAHFWPLAMTAILGYLVNSAVRTLLFGYFGRKIYRPGLHFSLASVAPNLRFGAWLTADSIINYLNTNLSTLVLARILGAGVAGGYNLAYNVAVVPPMKLNPIITRVLFPAFAKIQDDTEKLRVNFYKLLSVVGIINFPALLGLMVVSNNFVPLVFGEKWNSIIPVLQLLCVVGLLRSVGNPIGSLLMAKARVDISFKFNVFKTFLFIPAIVIGGQMAGAIGVTLGFLLVQIINTILSYFVMIKPVLGSSYRQYILSLWLPFYLSLPTLVVSYALGIVLKGQLALGMLLAVQIATGVLAFVVMIVLSRHPLVVEVKRQFCRSEKMKMLLRAG

SEQ ID NO: 94 - DNA, 1395 bp, Escherichia coli
atgacaaatctaaaaaagcgcgagcgagcgaaaaccaatgcatcgttaatctctatggtgcaacgcttttcagatatcaccatcatgtttgccggactatggctggtttgcgaagtcagcggactgtcattcctctacatgcacctgttggtggcgctgattacgctggtggtgttccagatgctgggcggcatcaccgatttttatcgctcatggcgcggtgttcgggcagcgacagaatttgccctgttgctacaaaactggaccttaagcgtgattttcagcgccggactggtggcgttcaacaatgatttcgacacgcaactgaaaatctggctggcgtggtatgcgctgaccagcatcggactggtggtttgccgttcgtgtattcgcattggggcgggctggctgcgtaatcatggctataacaagcgcatggtcgcggtggcgggggatttagccgccgggcaaatgctgatggagagcttccgtaaccagccgtggttagggtttgaagtggtgggcgtttaccacgacccgaaaccgggcggcgtttctaacgactgggcgggtaacctgcaacagctggtcgaggacgcgaaagcgggcaagattcataacgtctatatcgcgatgcaaatgtgcgacggcgcgcgagtgaaaaaactggtccatcaactggcggacaccacctgttcggtgctgctgatccccgacgtctttaccttcaacattctccattcacgcctcgaagagatgaacggcgtaccggtggtgccgctttacgacacgccgctttccggggttaaccgcctgctcaaacgtgcggaagacattgtgctggcgacgcttattctgctgctgatctccccggtgctgtgctgtattgcgctggcggtgaaactcagttcaccagggccggttattttccgccagactcgctacggcatggatggcaagccgatcaaagtgtggaagttccgttccatgaaagtgatggagaacgacaaagtggtgacccaggcgacgcagaacgatccgcgcgtcaccaaagtggggaactttctgcgccgtacctcgctggatgaattgccgcagtttatcaatgtgctgaccggggggatgtcgattgtcggtccacgtccgcacgcagtagcgcataacgaacagtatcgacagctcattgaaggctacatgctgcgccataaggtgaaaccgggcattaccggctgggcgcagattaacggctggcgcggcgaaaccgacacgctggagaaaatggaaaaacgcgtcgagttcgaccttgagtacatccgcgaatggagcgtctggttcgatatcaaaatcgttttcctgacggtgttcaaaggtttcgttaacaaagcggcatattga

SEQ ID NO: 95 - protein, 464 aa, Escherichia coli
MTNLKKRERAKTNASLISMVQRFSDITIMFAGLWLVCEVSGLSFLYMHLLVALITLVVFQMLGGITDFYRSWRGVRAATEFALLLQNWTLSVIFSAGLVAFNNDFDTQLKIWLAWYALTSIGLVVCRSCIRIGAGWLRNHGYNKRMVAVAGDLAAGQMLMESFRNQPWLGFEVVGVYHDPKPGGVSNDWAGNLQQLVEDAKAGKIHNVYIAMQMCDGARVKKLVHQLADTTCSVLLIPDVFTFNILHSRLEEMNGVPVVPLYDTPLSGVNRLLKRAEDIVLATLILLLISPVLCCIALAVKLSSPGPVIFRQTRYGMDGKPIKVWKFRSMKVMENDKVVTQATQNDPRVTKVGNFLRRTSLDELPQFINVLTGGMSIVGPRPHAVAHNEQYRQLIEGYMLRHKVKPGITGWAQINGWRGETDTLEKMEKRVEFDLEYIREWSVWFDIKIVFLTVFKGFVNKAAY

SEQ ID NO: 96 - DNA, 1119 bp, Escherichia coli
atgattaattatggcgttgttggtgttggatactttggcgctgaattagctcgttttatgaatatgcatgataatgcaaaaattacatgtgtatacgatcctgaaaatggagaaaatattgcccgtgaattgcagtgtatcaatatgtcaagcttggatgctttagtctcaagtaaattagtcgattgcgtgatcgtagccaccccaaattatctgcataaagaaccagtaattaaagcagcaaagaataagaagcatgttttttgtgaaaaaccaattgcattaagttatgaagattgtgtggatatggtcaaagcgtgtaaagaagctggtgtgacctttatggccgggcatattatgaattttttcaatggggttcaatatgcacggaagttaattaaagaaggtgttatcggcgaaatattatcatgtcatactaagagaaatggctgggaaaacaaacaagagagactttcctggaaaaagatgaaagaacaatctggtggacatctatatcatcatatacatgagttagattgtgttcagcatttacttggagaaataccagagacggttactatgattggtggaaatttggcccattctggtccaggatttggcaatgaagatgatatgttatttatgaccttggaattcccgtcaggaaaactagcaaccttagagtgggggagtgcatttaactggccggaacattatgtcatcatcaatggaactaaaggctctattaaaattgatatgcaagaaacagcagggtcacttaggattggcggtcagacaaagcattttttggtccatgaaacacaagaagaagatgatgatcgtcggaaaggcaatatgacctcagaaatggatggcgctatagcatatggtcatccaggaaaaaaaacaccattatggcttgccagtttaataagaaaggagacgttattcctccataatatcctctgtggtgcaaaacctgaagaagattatattgaccttctcaatggtgaggcggccatgtcggcgattgctactgctgatgctgccactctttcaagatcgcaggacaggaaagtgaaaatcagtgagatcattaaacatacatcagtaatgtaa

SEQ ID NO: 97 - protein, 372 aa, Escherichia coli
MINYGVVGVGYFGAELARFMNMHDNAKITCVYDPENGENIARELQCINMSSLDALVSSKLVDCVIVATPNYLHKEPVIKAAKNKKHVFCEKPIALSYEDCVDMVKACKEAGVTFMAGHIMNFFNGVQYARKLIKEGVIGEILSCHTKRNGWENKQERLSWKKMKEQSGGHLYHHIHELDCVQHLLGEIPETVTMIGGNLAHSGPGFGNEDDMLFMTLEFPSGKLATLEWGSAFNWPEHYVIINGTKGSIKIDMQETAGSLRIGGQTKHFLVHETQEEDDDRRKGNMTSEMDGAIAYGHPGKKTPLWLASLIRKETLFLHNILCGAKPEEDYIDLLNGEAAMSAIATADAATLSRSQDRKVKISEIIKHTSVM

SEQ ID NO: 98 - DNA, 1776 bp, Escherichia coli
atgaaaaaaatcagcttaccgaaaattggtatccgcccggttattgacggtcgtcgcatgggtgttcgtgagtcgcttgaagaacaaacaatgaatatggcgaaagctacggccgcactgctgaccgagaaactgcgccatgcctgcggagctgccgtcgagtgtgtcatttccgatacctgtatcgcgggtatggctgaagccgctgcttgcgaagaaaaattcagcagtcagaatgtaggcctcaccattacggtaacgccttgctggtgctatggcagtgaaaccatcgacatggatccaacccgcccgaaggccatttggggctttaacggcactgaacgccccggcgctgtttacctggcagcggctctggcagctcacagccagaaaggcatcccagcattctccatttacggtcatgacgttcaggatgccgatgacacatcgattcctgccgatgttgaagaaaaactgctgcgctttgcccgcgccggtttggccgtcgccagcatgaaaggtaaaagctatctgtcgctgggcggcgtttcgatgggtatcgccggttccattgttgatcacaacttctttgaatcctggctgggaatgaaagtccaggcggtggatatgaccgaactgcgtcgccgtatcgatcagaagatttacgacgaagccgaattggaaatggcactggcctgggctgataaaaacttccgctatggcgaagatgaaaataacaaacagtatcaacgtaatgccgagcaaagccgcgcagttctgcgcgaaagtttactgatggcgatgtgtatccgcgacatgatgcaaggcaacagcaaactggccgatattggtcgcgtggaagaatcacttggctacaacgccatcgctgcgggcttccaggggcaacgtcactggaccgatcaatatcccaatggtgacaccgccgaagcgatcctcaacagttcatttgactggaatggcgtgcgcgaaccctttgtcgtggcgaccgaaaacgacagtcttaacggcgtggcaatgctaatgggtcaccagctcaccggcaccgctcaggtatttgccgatgtgcgtacctactggtcaccagaagcaattgagcgtgtaacggggcataaactggatggactggcagaacacggcatcatccatttgatcaactccggttctgctgcgctggacggttcctgtaaacaacgcgacagcgaaggtaacccgacgatgaagccacactgggaaatctctcagcaagaggctgacgcttgcctcgccgctaccgaatggtgcccggcgatccacgaatacttccgtggcggcggttactcttcccgcttccttaccgaaggcggcgtcccgttcaccatgactcgtgtcaacatcatcaaaggcctgggaccggtactgcaaatcgcggaaggctggagcgtggaattgccgaaggatgtgcatgacatcctcaacaaacgcaccaactcaacctggccaaccacctggtttgcaccgcgcctcaccggtaaagggccgtttacggatgtgtactcggtaatggcgaactggggcgctaaccatggggttctgaccatcggccacgttggcgcagactttatcactctcgcctccatgctgcgtatcccggtatgtatgcacaacgttgaagagaccaaagtgtatcgtccttctgcctgggctgcgcacggcatggatattgaaggccaggattaccgcgcttgccagaactacggtccgttgtacaagcgttaa

SEQ ID NO: 99 - protein, 591 aa, Escherichia coli
MKKISLPKIGIRPVIDGRRMGVRESLEEQTMNMAKATAALLTEKLRHACGAAVECVISDTCIAGMAEAAACEEKFSSQNVGLTITVTPCWCYGSETIDMDPTRPKAIWGFNGTERPGAVYLAAALAAHSQKGIPAFSIYGHDVQDADDTSIPADVEEKLLRFARAGLAVASMKGKSYLSLGGVSMGIAGSIVDHNFFESWLGMKVQAVDMTELRRRIDQKIYDEAELEMALAWADKNFRYGEDENNKQYQRNAEQSRAVLRESLLMAMCIRDMMQGNSKLADIGRVEESLGYNAIAAGFQGQRHWTDQYPNGDTAEAILNSSFDWNGVREPFVVATENDSLNGVAMLMGHQLTGTAQVFADVRTYWSPEAIERVTGHKLDGLAEHGIIHLINSGSAALDGSCKQRDSEGNPTMKPHWEISQQEADACLAATEWCPAIHEYFRGGGYSSRFLTEGGVPFTMTRVNIIKGLGPVLQIAEGWSVELPKDVHDILNKRTNSTWPTTWFAPRLTGKGPFTDVYSVMANWGANHGVLTIGHVGADFITLASMLRIPVCMHNVEETKVYRPSAWAAHGMDIEGQDYRACQNYGPLYKR

SEQ ID NO: 100 - DNA, 1419 bp, Escherichia coli
atgaaacaagaagttatcctggtactcgactgtggcgcgaccaatgtcagggccatcgcggttaatcggcagggcaaaattgttgcccgcgcctcaacgcctaatgccagcgatatcgcgatggaaaacaacacctggcaccagtggtctttagacgccattttgcaacgctttgctgattgctgtcggcaaatcaatagtgaactgactgaatgccacatccgcggtatcgccgtcaccacctttggtgtggatggcgctctggtagataagcaaggcaatctgctctatccgattattagctggaaatgtccgcgaacagcagcggttatggacaatattgaacggttaatctccgcacagcggttgcaggctatttctggcgtcggagcctttagtttcaatacgttatataagttggtgtggttgaaagaaaatcatccacaactgctggaacgcgcgcacgcctggctctttatttcgtcgctgattaaccaccgtttaaccggcgaattcactactgatatcacgatggccggaaccagccagatgctggatatccagcaacgcgatttcagtccgcaaattttacaagccaccggtattccacgccgactcttccctcgtctggtggaagcgggtgaacagattggtacgctacagaacagcgccgcagcaatgctcggcttacccgttggcataccggtgatttccgcaggtcacgatacccagttcgccctttttggcgctggtgctgaacaaaatgaacccgtgctctcttccggtacatgggaaattttaatggttcgcagcgcccaggttgatacttcgctgttaagtcagtacgccggttccacctgcgaactggatagccaggcagggttgtataacccaggtatgcaatggctggcatccggcgtgctggaatgggtgagaaaactgttctggacggctgaaacaccctggcaaatgttgattgaagaagctcgtctgatcgcgcctggcgcggatggcgtaaaaatgcagtgtgatttattgtcgtgtcagaacgctggctggcaaggagtgacgcttaataccacgcgggggcatttctatcgcgcggcgctggaagggttaactgcgcaattacagcgcaatctacagatgctggaaaaaatcgggcactttaaggcctctgaattattgttagtcggtggaggaagtcgcaacacattgtggaatcagattaaagccaatatgcttgatattccggtaaaagttctcgacgacgccgaaacgaccgtcgcaggagctgcgctgttcggttggtatggcgtaggggaatttaacagcccggaagaagcccgcgcacagattcattatcagtaccgttatttctacccgcaaactgaacctgaatttatagaggaagtgtga

SEQ ID NO: 101 - protein, 472 aa, Escherichia coli
MKQEVILVLDCGATNVRAIAVNRQGKIVARASTPNASDIAMENNTWHQWSLDAILQRFADCCRQINSELTECHIRGIAVTTFGVDGALVDKQGNLLYPIISWKCPRTAAVMDNIERLISAQRLQAISGVGAFSFNTLYKLVWLKENHPQLLERAHAWLFISSLINHRLTGEFTTDITMAGTSQMLDIQQRDFSPQILQATGIPRRLFPRLVEAGEQIGTLQNSAAAMLGLPVGIPVISAGHDTQFALFGAGAEQNEPVLSSGTWEILMVRSAQVDTSLLSQYAGSTCELDSQAGLYNPGMQWLASGVLEWVRKLFWTAETPWQMLIEEARLIAPGADGVKMQCDLLSCQNAGWQGVTLNTTRGHFYRAALEGLTAQLQRNLQMLEKIGHFKASELLLVGGGSRNTLWNQIKANMLDIPVKVLDDAETTVAGAALFGWYGVGEFNSPEEARAQIHYQYRYFYPQTEPEFIEEV

SEQ ID NO: 102 - DNA, 492 bp, Escherichia coli
atgcattgctataacgggatgacaggtttacatcaccgcgaaccgggaatggttggcgcgggattaacggacaagcgcgcctggctggaactgatagccgatggtcatcatgtgcatccggcggcaatgtcgctgtgttgttgctgtgcgaaagagagaatcgtactgatcaccgacgcgatgcaggcagctgggatgccggatggtcgctatacgttatgtggtgaagaagtgcagatgcacggtggcgttgtccgtaccgcgtctggtgggctggcgggcagtacgctgtctgttgatgcggcagtgcgcaatatggtcgagttgacgggcgtaacgctgcggaagccatccatatggcgtcgctgcatccggcgcgaatgctgggtgttgatggtgttctgggatcgcttaaaccgggcaaacgcgccagagtcgttgcgctggatagcgggctacatgtgcaacaaatctggattcagggtcaattag

SEQ ID NO: 103 - protein, 167 aa, Escherichia coli
MHCYNGMTGLHHREPGMVGAGLTDKRAWLELIADGHHVHPAAMSLCCCCAKERIVLITDAMQAAGMPDGRYTLCGEEVQMHGGVVRTASGGLAGSTLSVDAAVRNMVELTGVTPAEAIHMASLHPARMLGVDGVLGSLKPGKRASVVALDSGLHVQQIWIQGQLASF